European Patent Application EP 4 282 877 A2, published November 29, 2023. Title: CHIMERIC ANTIGEN RECEPTORS TARGETING BCMA AND METHODS OF USE THEREOF. Applicant: Legend Biotech Ireland Limited. The sequence listing filed with the application follows.

SEQUENCE LISTING (399 sequences)

SEQ ID NO: 1 - protein, 6 aa, synthetic construct
DYYAIG

SEQ ID NO: 2 - protein, 5 aa, synthetic construct
TYGMA

SEQ ID NO: 3 - protein, 5 aa, synthetic construct
TFTMG

SEQ ID NO: 4 - protein, 5 aa, synthetic construct
INAMG

SEQ ID NO: 5 - protein, 5 aa, synthetic construct
SIVMG

SEQ ID NO: 6 - protein, 5 aa, synthetic construct
RAVIV

SEQ ID NO: 7 - protein, 5 aa, synthetic construct
SDVMG

SEQ ID NO: 8 - protein, 5 aa, synthetic construct
NDHMA

SEQ ID NO: 9 - protein, 5 aa, synthetic construct
KNTVA

SEQ ID NO: 10 - protein, 5 aa, synthetic construct
SHVMG

SEQ ID NO: 11 - protein, 5 aa, synthetic construct
TYFMA

SEQ ID NO: 12 - protein, 5 aa, synthetic construct
INVMA

SEQ ID NO: 13 - protein, 5 aa, synthetic construct
TFTMG

SEQ ID NO: 14 - protein, 5 aa, synthetic construct
INAMG

SEQ ID NO: 15 - protein, 5 aa, synthetic construct
KNTVA

SEQ ID NO: 16 - protein, 5 aa, synthetic construct
SIVMG

SEQ ID NO: 17 - protein, 5 aa, synthetic construct
TFTMG

SEQ ID NO: 18 - protein, 5 aa, synthetic construct
KNTVA

SEQ ID NO: 19 - protein, 5 aa, synthetic construct
INTMD

SEQ ID NO: 20 - protein, 5 aa, synthetic construct
KNTVA

SEQ ID NO: 21 - protein, 5 aa, synthetic construct
DYWMH

SEQ ID NO: 22 - protein, 5 aa, synthetic construct
SNTMA

SEQ ID NO: 23 - protein, 5 aa, synthetic construct
TFTMG

SEQ ID NO: 24 - protein, 6 aa, synthetic construct
VAAISL

SEQ ID NO: 25 - protein, 5 aa, synthetic construct
KNTVA

SEQ ID NO: 26 - protein, 5 aa, synthetic construct
TFTMG

SEQ ID NO: 27 - protein, 5 aa, synthetic construct
TFTMG

SEQ ID NO: 28 - protein, 5 aa, synthetic construct
SIVMG

SEQ ID NO: 29 - protein, 5 aa, synthetic construct
TFTMG

SEQ ID NO: 30 - protein, 5 aa, synthetic construct
TFTMG

SEQ ID NO: 31 - protein, 5 aa, synthetic construct
TFTMG

SEQ ID NO: 32 - protein, 5 aa, synthetic construct
TFTMG

SEQ ID NO: 33 - protein, 5 aa, synthetic construct
TFTMG

SEQ ID NO: 34 - protein, 5 aa, synthetic construct
NHVMG

SEQ ID NO: 35 - protein, 5 aa, synthetic construct
NYILA

SEQ ID NO: 36 - protein, 5 aa, synthetic construct
TFTMG

SEQ ID NO: 37 - protein, 5 aa, synthetic construct
TFTMG

SEQ ID NO: 38 - protein, 6 aa, synthetic construct
NNFVMG

SEQ ID NO: 39 - protein, 17 aa, synthetic construct
CISRSDGSTYYADSVKG

SEQ ID NO: 40 - protein, 19 aa, synthetic construct
SKASMNYSGRTYYADSVKG

SEQ ID NO: 41 - protein, 17 aa, synthetic construct
AISLSPTLAYYAESVKG

SEQ ID NO: 42 - protein, 16 aa, synthetic construct
SIRGLGRTNYDDSVKG

SEQ ID NO: 43 - protein, 17 aa, synthetic construct
AIMWNDGITYLQDSVKG

SEQ ID NO: 44 - protein, 17 aa, synthetic construct
FIKPSDGTIYYIDSLKG

SEQ ID NO: 45 - protein, 17 aa, synthetic construct
AIMWNDGITYLQDSVKG

SEQ ID NO: 46 - protein, 17 aa, synthetic construct
AIDWSGRTTNYADPVEG

SEQ ID NO: 47 - protein, 17 aa, synthetic construct
SITWDGRTTYYADSVKG

SEQ ID NO: 48 - protein, 17 aa, synthetic construct
VIGWRDISTSYADSVKG

SEQ ID NO: 49 - protein, 17 aa, synthetic construct
GIAWSGGSTAYADSVKG

SEQ ID NO: 50 - protein, 16 aa, synthetic construct
AVTRDGRKSCGDSVKG

SEQ ID NO: 51 - protein, 17 aa, synthetic construct
SITWDGRSAYYAESVKG

SEQ ID NO: 52 - protein, 16 aa, synthetic construct
TITRGGSTNYGPSVKG

SEQ ID NO: 53 - protein, 17 aa, synthetic construct
SITCDGRTTYYANSVNG

SEQ ID NO: 54 - protein, 17 aa, synthetic construct
AIMWNDGLTYLQGSVKG

SEQ ID NO: 55 - protein, 17 aa, synthetic construct
AISLSPTLAYYAESVKG

SEQ ID NO: 56 - protein, 17 aa, synthetic construct
SITWDGRTTYYADSVKG

SEQ ID NO: 57 - protein, 17 aa, synthetic construct
AISLSPTLAYYAESVKG

SEQ ID NO: 58 - protein, 17 aa, synthetic construct
SITCDGRTTYYANSVKG

SEQ ID NO: 59 - protein, 17 aa, synthetic construct
SIDTSGQTTYYADSLKG

SEQ ID NO: 60 - protein, 17 aa, synthetic construct
STTWNGRSTYYADSVKG

SEQ ID NO: 61 - protein, 15 aa, synthetic construct
DISGGRTNYADSVKG

SEQ ID NO: 62 - protein, 21 aa, synthetic construct
FTISRDNAKNTVVLQMNSLKP

SEQ ID NO: 63 - protein, 17 aa, synthetic construct
SITWDGRTTYYADSVKG

SEQ ID NO: 64 - protein, 17 aa, synthetic construct
AISLSPTLAYYAESVKG

SEQ ID NO: 65 - protein, 19 aa, synthetic construct
AISLSPTLAYYAESVKGKG

SEQ ID NO: 66 - protein, 17 aa, synthetic construct
AIMWNDGITYLQDSVKG

SEQ ID NO: 67 - protein, 17 aa, synthetic construct
AINLSPTLTYYAESVKG

SEQ ID NO: 68 - protein, 17 aa, synthetic construct
SITLIPTFPYYAYSVKG

SEQ ID NO: 69 - protein, 17 aa, synthetic construct
AISLSPTLAYYAESVKG

SEQ ID NO: 70 - protein, 17 aa, synthetic construct
AISLSPTLAYYAESVKG

SEQ ID NO: 71 - protein, 17 aa, synthetic construct
VIGWRDINASYADSVKG

SEQ ID NO: 72 - protein, 17 aa, synthetic construct
VIGWRDISTSYADSVKG

SEQ ID NO: 73 - protein, 17 aa, synthetic construct
HISRSGGKSGYGDSVKG

SEQ ID NO: 74 - protein, 17 aa, synthetic construct
AISLSPTLAYYAESVKG

SEQ ID NO: 75 - protein, 17 aa, synthetic construct
AISLSPTLAYYAEPVKG

SEQ ID NO: 76 - protein, 17 aa, synthetic construct
AISLSPTLAYYVESVKG

SEQ ID NO: 77 - protein, 14 aa, synthetic construct
AGADCSGYLRDYEF

SEQ ID NO: 78 - protein, 18 aa, synthetic construct
AGTGCSTYGCFDAQIIDY

SEQ ID NO: 79 - protein, 13 aa, synthetic construct
ADRKSVMSIRPDY

SEQ ID NO: 80 - protein, 13 aa, synthetic construct
VYVTLLGGVNRDY

SEQ ID NO: 81 - protein, 11 aa, synthetic construct
ASKGRYSEYEY

SEQ ID NO: 82 - protein, 17 aa, synthetic construct
ASPEDWYTDWIDWSIYR

SEQ ID NO: 83 - protein, 11 aa, synthetic construct
ASKGRYSEYEY

SEQ ID NO: 84 - protein, 12 aa, synthetic construct
VLRAWISYDNDY

SEQ ID NO: 85 - protein, 12 aa, synthetic construct
DLGKWPAGPADY

SEQ ID NO: 86 - protein, 11 aa, synthetic construct
ARRIDAADFDS

SEQ ID NO: 87 - protein, 11 aa, synthetic construct
SRGIEVEEFGA

SEQ ID NO: 88 - protein, 16 aa, synthetic construct
DGWGATTLDYTYGMDY

SEQ ID NO: 89 - protein, 12 aa, synthetic construct
DRKSVMSIRPDY

SEQ ID NO: 90 - protein, 14 aa, synthetic construct
ERLDGSGYGYEYDY

SEQ ID NO: 91 - protein, 12 aa, synthetic construct
YRKSIMSIQPDY

SEQ ID NO: 92 - protein, 12 aa, synthetic construct
DRKSVMSIRPDY

SEQ ID NO: 93 - protein, 10 aa, synthetic construct
RRIDAADFDS

SEQ ID NO: 94 - protein, 11 aa, synthetic construct
LGKWPAGPADY

SEQ ID NO: 95 - protein, 12 aa, synthetic construct
DRKSVMSIRPDY

SEQ ID NO: 96 - protein, 11 aa, synthetic construct
LGKWPAGSADY

SEQ ID NO: 97 - protein, 12 aa, synthetic construct
RYRGGTWYGMAN

SEQ ID NO: 98 - protein, 11 aa, synthetic construct
LGKWPAGPADY

SEQ ID NO: 99 - protein, 12 aa, synthetic construct
DRKSVMSIRPDY

SEQ ID NO: 100 - protein, 12 aa, synthetic construct
DRKSVMSIRPDY

SEQ ID NO: 101 - protein, 16 aa, synthetic construct
TASCHLFGLGSGAFVS

SEQ ID NO: 102 - protein, 10 aa, synthetic construct
SKDRYSEYEY

SEQ ID NO: 103 - protein, 8 aa, synthetic construct
KNGGPVDY

SEQ ID NO: 104 - protein, 10 aa, synthetic construct
SKGRYSEYEY

SEQ ID NO: 105 - protein, 12 aa, synthetic construct
ERKSVMAIPPDY

SEQ ID NO: 106 - protein, 12 aa, synthetic construct
YRKYLMSILPDY

SEQ ID NO: 107 - protein, 18 aa, synthetic construct
NRNSQRVIAALSWIGMNY

SEQ ID NO: 108 - protein, 10 aa, synthetic construct
RRIDAADFDS

SEQ ID NO: 109 - protein, 10 aa, synthetic construct
RRIDATDFDS

SEQ ID NO: 110 - protein, 10 aa, synthetic construct
RRIDAADFDS

SEQ ID NO: 111 - protein, 12 aa, synthetic construct
PLWYGSPTLIDY

SEQ ID NO: 112 - protein, 12 aa, synthetic construct
DRKSVMSIRPDY

SEQ ID NO: 113 - protein, 12 aa, synthetic construct
DRKSVMSIRPDY

SEQ ID NO: 114 - protein, 12 aa, synthetic construct
DRKSVMSIRPDY

SEQ ID NO: 115 - protein, 122 aa, synthetic construct
QVQLVESGGGLVQPGGSLRLSCEASGFTLDYYAIGWFRQAPGKEREGVICISRSDGSTYYADSVKGRFTISRDNAKKTVYLQMISLKPEDTAAYYCAAGADCSGYLRDYEFRGQGTQVTVSS

SEQ ID NO: 116 - protein, 128 aa, synthetic construct
QVKLEESGGRLVQPRGSLRLSCAGSGRTFSTYGMAWFRQAPGKEREFVASKASMNYSGRTYYADSVKGRFTIARDNAKNMVFLQMNNLKPEDTAVYYCAAGTGCSTYGCFDAQIIDYWGKGTLVTVSS

SEQ ID NO: 117 - protein, 118 aa, synthetic construct
EVQLVESGGGLVQAGGSLRLSCAASGRTFTMGWFRQAPGKEREFVAAISLSPTLAYYAESVKGRFTISRDNAKNTVVLQMNSLKPEDTALYYCAADRKSVMSIRPDYWGQGTQVTVSS

SEQ ID NO: 118 - protein, 120 aa, synthetic construct
AVQLVDSGGGLVQPGGSLRLSCVASGGIFVINAMGWYRQAPGKQRELVASIRGLGRTNYDDSVKGRFTISRDNANNTVYLQMNSLEPEDTAVYYCTVYVTLLGGVNRDYWGQGTQVTVSS

SEQ ID NO: 119 - protein, 119 aa, synthetic construct
EVQLVESGGGLVQAGGSLRLSCAASGRTFSSIVMGWFRQAPGKEREFVGAIMWNDGITYLQDSVKGRFTIFRDNAKNTVYLQMNSLKLEDTAVYYCAASKGRYSEYEYWGQGTQVTVSS

SEQ ID NO: 120 - protein, 128 aa, synthetic construct
EVQLVESGGGVVQAGGSLTVSCTASGFTFDRAVIVWFRQAPGKGREGVSFIKPSDGTIYYIDSLKGRFTISSDIAKNTVYLQMKSLESEDSAVYYCAASPEDWYTDWIDWSIYRWQHWGQGTQVTVSS

SEQ ID NO: 121 - protein, 119 aa, synthetic construct
EVQLVESGGGMVQAGDSLRLSCVQSTYTVNSDVMGWFRQAPGKEREFVGAIMWNDGITYLQDSVKGRFTIFRDNAKNTVYLQMNSLKLEDTAVYYCAASKGRYSEYEYWGQGTQVTVSS

SEQ ID NO: 122 - protein, 120 aa, synthetic construct
AVQLVESGGGLVQAGDSLRLSCTASGATLTNDHMAWFRQAPGKGREFVAAIDWSGRTTNYADPVEGRFTISRNNAKNTVYLEMNSLKLEDTAVYYCAVLRAWISYDNDYWGQGTQVTVSS

SEQ ID NO: 123 - protein, 120 aa, synthetic construct
QVQLVESGGGLVQAGGSLRLSCAASGGTLSKNTVAWFRQAPGKERGFVASITWDGRTTYYADSVKGRFTISRDNAKNTVYLQMNSLKPEDTAVYVCADLGKWPAGPADYWGQGTQVTVSS

SEQ ID NO: 124 - protein, 119 aa, synthetic construct
QVKLEESGGGLVQAGRSLRLSCAASEHTFSSHVMGWFRQAPGKERESVAVIGWRDISTSYADSVKGRFTISRDNAKKTLYLQMNSLKPEDTAVYYCAARRIDAADFDSWGQGTQVTVSS

SEQ ID NO: 125 - protein, 119 aa, synthetic construct
AVQLVESGGGLVQAGDSLRLTCTASGRAFSTYFMAWFRQAPGKEREFVAGIAWSGGSTAYADSVKGRFTISRDNAKNTVYLQMNSLKSEDTAVYYCASRGIEVEEFGAWGQGTQVTVSS

SEQ ID NO: 126 - protein, 124 aa, synthetic construct
EVQLVESGGGLVPPGGSLRLSCTASGSTVSINVMAWYRQVSGKQRELVAAVTRDGRKSCGDSVKGRFTISRDGAKNAVYLQMNSLKPEDTAVYLCGADGWGATTLDYTYGMDYWGKGTQVTVSS

SEQ ID NO: 127 - protein, 118 aa, synthetic construct
AVQLVESGGGLVQAGGSLRLSCAASGRTFTMGWFRQAPGKERGFVASITWDGRSAYYAESVKGRFTISRDNAKNTVVLQMNSLKPEDTALYYCAADRKSVMSIRPDYWGQGTQVTVSS

SEQ ID NO: 128 - protein, 122 aa, synthetic construct
QVQLVESGGGLVQPGGSLRLACEAPGSGNSINAMGWYRQTPGKRRELVATITRGGSTNYGPSVKGRFTITRDNVKNTVHLQMNSLKPDDTAVYYCNAERLDGSGYGYEYDYWGQGTQVTVSS

SEQ ID NO: 129 - protein, 121 aa, synthetic construct
QVKLEESGGGLVQAGGSLRLSCAASGGTLSKNTVAWVRQAPGKERGFVTSITCDGRTTYYANSVNGRFPINRNNAENLVVLQMNSLKPDDTALYYCAAYRKSIMSIQPDYWGQGTQVTVSS

SEQ ID NO: 130 - protein, 121 aa, synthetic construct
DVQLVESGGGLVQAGGSLRLSCAASGRTFSSIVMGWFRQAPGKEREFVGAIMWNDGLTYLQGSVKGRFTISRDNAKNTVVLQMNSLKPEDTALYYCAADRKSVMSIRPDYWGQGTQVTVSS

SEQ ID NO: 131 - protein, 116 aa, synthetic construct
QVQLVESGGGLVQAGGSLRLSCAASGRTFTMGWFRQAPGKEREFVAAISLSPTLAYYAESVKGRFTISRDNAKNTVVLQMNSLKPEDTAVYYCAARRIDAADFDSWGQGTQVTVSS

SEQ ID NO: 132 - protein, 120 aa, synthetic construct; identical to SEQ ID NO: 123

SEQ ID NO: 133 - protein, 121 aa, synthetic construct
QVQLVESGGGLVQPGGSLTLSCAASGSIDSINTMDWFRQAPGKEREFVAAISLSPTLAYYAESVKGRFTISRDNAKNTVVLQMNSLKPEDTALYYCAADRKSVMSIRPDYWGQGTQVTVSS

SEQ ID NO: 134 - protein, 120 aa, synthetic construct
DVQLVESGGGLVQAGGSLRLSCAASGGTLSKNTVAWVRQAPGKERGFVTSITCDGRTTYYANSVKGRFPISRDNAENTVYLQMNSLKPEDTAGYVCADLGKWPAGSADYWGQGTHVTVSS

SEQ ID NO: 135 - protein, 121 aa, synthetic construct
QVKLEESGGGLVQPGGSLRLSCTASEFTFSDYWMHWVRQAPGKGLEWVASIDTSGQTTYYADSLKGRFTISRDNAKSTLYLQMNSLKSEDTGVYFCAKRYRGGTWYGMANWGKGTQVTVSS

SEQ ID NO: 136 - protein, 120 aa, synthetic construct
QVQLVESGGGLVQAGGSLRLSCAASGRTLSSNTMAWFRQAPGKEREFVASTTWNGRSTYYADSVKGRFTISRDNAKNTMYLQMNSLKPEDTAVYVCADLGKWPAGPADYWGQGTQVTVSS

SEQ ID NO: 137 - protein, 116 aa, synthetic construct
QVQLVESGGGLVQAGGSLRLSCAASGRTFTMGWFRQAPGKQRELVADISGGRTNYADSVKGRFTISRDNAKNTVYLQMNSLKPEDTAVYYCAADRKSVMSIRPDYWGQGTQVTVSS

SEQ ID NO: 138 - protein, 104 aa, synthetic construct
QVQLVESGGGLVQAGASLRLSCAASGRTFTVAAISLSPTLAYYAESVKGRFTISRDNAKNTVVLQMNSLKPEDTALYYCAADRKSVMSIRPDYWGQGTQVTVSS

SEQ ID NO: 139 - protein, 125 aa, synthetic construct
DVQLVESGGGLEQAGGSLRLSCAASGGTLSKNTVAWFRQAPGKERGFVASITWDGRTTYYADSVKGRFTISRDNAKNTVYLQMNSLKPEDTAVYYCASTASCHLFGLGSGAFVSWGRGTQVTVSS

SEQ ID NO: 140 - protein, 116 aa, synthetic construct
AVQLVESGGGLVQAGGSLRLSCAASGRTFTMGWFHQAPGKEREFVAAISLSPTLAYYAESVKGRFTISRDNAKNTVVLQMNSLKPEDTALYYCAASKDRYSEYEYWGQGTQVTVSS

SEQ ID NO: 141 - protein, 114 aa, synthetic construct
QVKLEESGGGLVQAGGSLRLSCAASGRTFTMGWFRQAPGKEREFVAAISLSPTLAYYAESVKGRFTISRDNAKNTVVLQMNSLKPEDTALYYCAKKNGGPVDYWGKGTQVTVSS

SEQ ID NO: 142 - protein, 119 aa, synthetic construct
DVQLVESGGGLVQPGGSLRLSCAASGRTFSSIVMGWFRQAPGKEREFVGAIMWNDGITYLQDSVKGRFTIFRDNAKNTVYLQMNSLKLEDTAVYYCAASKGRYSEYEYWGQGTQVTVSS

SEQ ID NO: 143 - protein, 118 aa, synthetic construct
QVKLEESGGRLVQAGGSLKLSWAASGRTFTMGWFRQAPGKEREFVTAINLSPTLTYYAESVKGRFPISRNNAQNTVVLQMNSLKPEDTALYYCAAERKSVMAIPPDYWGQGTQVTVSS

SEQ ID NO: 144 - protein, 118 aa, synthetic construct
EVQLVESGGGLVQAGGSLRLSCAASGRTFTMGGFRRVPRDEREFVASITLIPTFPYYAYSVKGRFALFRDNPNNTVILLMISLKPEDPDLYYCASYRKYLMSILPDYWGQGTQGTVSS

SEQ ID NO: 145 - protein, 124 aa, synthetic construct
QVKLEESGGGLVQAGGSLRLSCAASGRTFTMGWFRQAPGKEREFVAAISLSPTLAYYAESVKGRFTISRDNAKNTVDLQMNSLKPEDTAVYFCAANRNSQRVIAALSWIGMNYWGEWTQVTVSS

SEQ ID NO: 146 - protein, 116 aa, synthetic construct
QVQLVESGGGLVQAGGSLRLSCAASGRTFTMGWFRQAPGKEREFVAAISLSPTLAYYAESVKGRFTISRDNAKKTLYLRMNSLKPEDTAVYYCAARRIDAADFDSWGQGTQVTVSS

SEQ ID NO: 147 - protein, 116 aa, synthetic construct
QVKLEESGGGLVQAGGSLRLSCAASGRTFTMGWFRRAPGKERESVAVIGWRDINASYADSVKGRFAISRDNAKKTLYLQMNSLKPEDTAVYYCAARRIDATDFDSWGQGTQVTVSS

SEQ ID NO: 148 - protein, 119 aa, synthetic construct
QVKLEESGGGLVQTGGSLRLSCAASEHTFSNHVMGWFRQAPGKERESVAVIGWRDISTSYADSVKGRFTISRDNAKKTLYLQMNSLKPEDTAVYYCAARRIDAADFDSRGQGTQVTVSS

SEQ ID NO: 149 - protein, 123 aa, synthetic construct
AVQLVDSGGGLVQAGGSLRISCAVSGRTSSNYILAWFRQAPGKERDFVAHISRSGGKSGYGDSVKGRFTISRDNAENTVRVYLQMNSLKPGDTAVYYCNRPLWYGSPTLIDYWGQGTQVTVSS

SEQ ID NO: 150 - protein, 118 aa, synthetic construct
QVQLVESGGGLVQAGGSLRLSCAASGRTFTMGWFRQAPGKEREFVAAISLSPTLAYYAESVKGRFTISRDNAKNTVVLQMNSLKPEDTALYYCAADRKSVMSIRPDYWGQGTQVTVSS

SEQ ID NO: 151 - protein, 118 aa, synthetic construct
AVQLVDSGGGLVQAGGSLRLSCAASGRTFTMGWFRQAPGKEREFVAAISLSPTLAYYAEPVKGRFTISRDNAKNTVVLQMNSLKPEDTALYYCAADRKSVMSIRPDYWGQGTQVTVSS

SEQ ID NO: 152 - protein, 121 aa, synthetic construct
DVQLVESGGGSVQTGGSLRLSCTASGRTLNNFVMGWFRQAPGKEREFVAAISLSPTLAYYVESVKGRFTISRDNAKNTVVLQMNSLKPEDTALYYCAADRKSVMSIRPDYWGQGTQVTVSS

SEQ ID NO: 153 - DNA, 366 bp, synthetic construct
  source 1..366: mol_type = other DNA
caggtgcagctggtggagtctgggggaggcttggtgcagcctgggggttctctgaggctctcctgtgaagcctctggattcactttggattattatgccataggctggttccgccaggccccagggaaggagcgcgagggggtcatatgtattagtagaagtgatggtagcacatactatgcagactccgtgaagggccgattcaccatctccagagacaacgccaagaaaacggtgtatctgcaaatgatcagcctgaaacctgaggacacggccgcttattactgtgcagcaggggccgattgttcggggtacctacgagattatgagttccgggggcaggggacccaggtcaccgtctcctca

SEQ ID NO: 154 - DNA, 384 bp, synthetic construct
  source 1..384: mol_type = other DNA
caggtaaagctggaggagtctgggggacgattggtgcagccaaggggctctctgagactctcctgtgcaggctctggacgcactttcagtacctatggtatggcctggttccgccaggctccagggaaggagcgtgagttcgtagcgtctaaagcatcgatgaattacagcggtagaacatactatgcagactccgtgaagggccgattcaccatcgccagagacaacgccaagaacatggtgtttctgcaaatgaacaacctgaagcctgaggacacggccgtttattactgtgcagcgggcactggatgctcaacatatgggtgttttgacgcccagataatagactactggggcaaagggaccctggtcaccgtctcctca

SEQ ID NO: 155 - DNA, 354 bp, synthetic construct
  source 1..354: mol_type = other DNA
gaggtgcagctggtggagtctgggggaggcttggtgcaggctggggggtctctgagactctcctgtgcagcctctggacgcaccttcaccatggggtggttccgtcaggctccagggaaggagcgtgagtttgtagcagctattagtttgagtcctactttagcatattatgcagagtccgtgaagggccgattcaccatcagccgagacaacgccaagaacacggtggttttgcaaatgaacagcctgaaacctgaggacacggccctttattactgtgcagcagaccggaaatcagtaatgtctattcggcccgactactggggccaggggacccaggtcaccgtctcctca

SEQ ID NO: 156 - DNA, 360 bp, synthetic construct
  source 1..360: mol_type = other DNA
gccgtgcagctggtggattctgggggaggcttggtgcagcctggggggtctctgagactctcctgtgtagcctctggaggtatcttcgtcatcaatgccatgggctggtaccgccaggctccaggaaagcagcgcgagttggtcgcatctattcgtggactaggcagaacaaactatgacgactccgtgaagggccgattcaccatctccagagacaacgccaacaacacggtgtatctgcagatgaacagcctggaacctgaggacacggccgtctactactgtacagtctacgttacactacttggtggggttaatagggactactggggccaggggacccaggtcaccgtctcctca

SEQ ID NO: 157 - DNA, 357 bp, synthetic construct
  source 1..357: mol_type = other DNA
gaggtgcagctggtggagtctgggggaggattggtgcaggctgggggctctctgagactctcctgtgcagcctctggacggaccttcagtagcattgtcatgggctggttccgccaggctccagggaaggagcgtgagtttgtaggagcgattatgtggaatgatggtattacatacttgcaagactccgtgaagggccgatttaccatcttcagagacaatgccaagaacacggtgtatctgcaaatgaacagcctgaaacttgaggatacggccgtttattactgtgcagcatccaagggtagatactcggaatatgagtactggggccaggggacccaggtcaccgtctcctca

SEQ ID NO: 158 - DNA, 384 bp, synthetic construct
  source 1..384: mol_type = other DNA
gaggtgcagctggtggagtctgggggaggcgtggtgcaggctggggggtctctgacagtctcctgtacagcctctggattcactttcgaccgtgctgtcatagtctggttccgccaggcccccgggaagggccgtgagggggtctcatttattaaacctagtgatggcaccatatactacattgactccctgaagggccgattcacgatctccagtgacatcgccaagaatacggtatatctgcaaatgaaaagtctggaatcggaggactcggccgtttattactgtgcggcctcgcctgaggactggtacacggattggatcgactggagtatatatcggtggcagcactggggccaggggacccaggtcactgtctcctca

SEQ ID NO: 159 - DNA, 357 bp, synthetic construct
  source 1..357: mol_type = other DNA
gaggtgcagctggtggagtctgggggaggaatggtgcaggctggggactctctgagactatcctgtgtgcagtctacttacaccgtcaatagcgatgtcatgggctggttccgccaggctccagggaaggagcgtgagtttgtaggagcgattatgtggaatgatggtattacatacttgcaagactccgtgaagggccgatttaccatcttcagagacaacgccaagaacacggtgtatctgcaaatgaacagcctgaaacttgaggatacggccgtttattactgtgcagcatccaagggtagatactcggaatatgagtactggggccaggggacccaggtcaccgtctcctca

SEQ ID NO: 160 - DNA, 360 bp, synthetic construct
  source 1..360: mol_type = other DNA
gcggtgcagctggtggagtctgggggaggattggtgcaggctggggactctctgagactctcctgtacagcctctggtgcaaccttgactaacgatcacatggcatggttccgccaggctccagggaaggggcgtgaatttgtagcagctattgactggagtggtcgtaccacaaattacgcagaccccgtagagggccgattcaccatctccagaaacaacgccaagaacacggtgtatctggaaatgaacagcctgaaacttgaggacacggccgtttattactgtgcggtcctccgcgcttggatctcatatgacaatgactactggggccaggggacccaggtcaccgtctcctca

SEQ ID NO: 161 - DNA, 360 bp, synthetic construct
  source 1..360: mol_type = other DNA
caggtgcagctggtggagtctgggggaggattggtgcaggctgggggctctctgagactctcctgtgcagcctctggaggcaccttaagtaaaaataccgtggcttggttccgccaggctccagggaaggagcgtgggtttgtagcgtctattacctgggatggtcgtacgacatactatgcagactccgtgaagggccgattcaccatctccagagacaacgccaagaacacagtgtatctgcaaatgaacagcctgaaacctgaggatacggccgtttatgtctgtgcagacttagggaaatggcctgcgggcccggcggactactggggccaggggacccaggtcaccgtctcctca

SEQ ID NO: 162 - DNA, 357 bp, synthetic construct
  source 1..357: mol_type = other DNA
caggtaaagctggaggagtctgggggaggcttggtgcaggctgggcggtctctgagactctcctgtgcagcctctgaacacaccttcagtagccatgtcatgggctggttccgccaggctccagggaaggagcgtgagtctgttgcagttattggctggagagatattagcacaagctatgcagactccgtgaagggccgattcaccatctccagagacaacgccaagaagacgctgtatctgcaaatgaatagcctgaaacctgaggacacggccgtttactactgtgcagcacgtcggatcgacgcagctgactttgattcctgggggcaggggacccaggtcaccgtctcctcg

SEQ ID NO: 163 - DNA, 357 bp, synthetic construct
  source 1..357: mol_type = other DNA
gcggtgcagctggtggagtctgggggaggattggtgcaggctggggactctctgagactcacctgtacagcctctggacgcgccttcagtacctatttcatggcctggttccgccaggctccagggaaggagcgtgagtttgtagcaggaattgcatggagtggtggtagcacggcgtatgcagactccgtgaagggccgattcaccatctccagagacaacgccaagaacacggtgtatctgcaaatgaacagcctgaaatctgaggacacggccgtttattactgtgccagcagggggattgaggtcgaagagtttggtgcctggggccaggggacccaggtcaccgtctcgtcg

SEQ ID NO: 164 - DNA, 372 bp, synthetic construct
  source 1..372: mol_type = other DNA
gaggtgcagctggtggagtctgggggaggcttggtgccgcctggggggtctctgagactctcctgtacagcctctggaagcacagtcagcatcaatgtcatggcctggtaccgccaggtttcagggaagcagcgcgagttggtcgcggccgttactagggatggtaggaaaagttgtggagactccgtgaagggccgattcaccatttccagagacggcgccaagaatgcggtatatttgcaaatgaacagtctgaaacctgaggacacagcggtctatttatgtggagccgatggttggggtgctactaccttagattatacctacggcatggactattggggcaaagggacccaggtcaccgtctcctca

SEQ ID NO: 165 - DNA, 354 bp, synthetic construct
  source 1..354: mol_type = other DNA
gcggtgcagctggtggagtctgggggaggattggtgcaggctgggggctctctgagactctcctgtgcagcctctggacgcaccttcaccatggggtggttccgtcaggctccagggaaggagcgtgggtttgtagcgtctattacctgggatggtcgttcggcatactatgcagagtccgtgaagggccgattcaccatcagccgagacaacgccaagaacacggtggttttgcaaatgaacagcctgaaacctgaggacacggccctttattactgtgcagcagaccggaaatcagtaatgtctattcggcccgactactggggccaggggacccaggtcaccgtctcctca

SEQ ID NO: 166 - DNA, 366 bp, synthetic construct
  source 1..366: mol_type = other DNA
caggtacagctggtggagtctgggggaggattggtgcagcctggggggtctctaagactcgcatgtgaagcgcctggaagcggcaatagtatcaatgccatgggctggtaccggcagactccggggaagcggcgcgagttggtcgcaactattactcggggtggtagcacgaactatggaccctccgtgaagggccgattcacgatcaccagagacaatgtcaagaatacggtgcatctgcagatgaacagcctgaaacctgacgacacggccgtctattattgcaatgcggagaggctggacggctcggggtacggatatgagtatgattactggggccaggggacccaggtcaccgtctcctca

SEQ ID NO: 167 - DNA, 363 bp, synthetic construct
  source 1..363: mol_type = other DNA
caggtaaagctggaggagtctgggggaggattggtgcaggctgggggctctctgagactctcctgtgcagcctctggaggcaccttaagtaagaataccgtggcttgggtccgccaggctccagggaaggagcgtgggtttgtaacgtctattacctgtgatggtcgtacgacatactatgcgaactccgtaaacggccgattccccatcaaccgaaacaacgccgagaatttggtggttttgcaaatgaacagcctgaaacctgacgacacggccctttattactgtgcagcataccggaagtcaataatgtctattcagcccgactactggggccaggggacccaggtcaccgtctcctca

SEQ ID NO: 168 - DNA, 363 bp, synthetic construct
  source 1..363: mol_type = other DNA
gatgtgcagctggtggagtctgggggaggattggtgcaggctgggggctctctgagactctcctgtgcagcctctggacggaccttcagtagcattgtcatgggctggttccgccaggctccagggaaggagcgtgagtttgtaggagcgattatgtggaatgatggtctgacatacttgcaagggtccgtgaagggccgattcaccatttccagagacaacgccaagaacacggtggttttgcaaatgaacagcctgaaacctgaggacacggccctttattactgtgcagcagaccggaaatcagtaatgtctattcggcccgactactggggccaggggacccaggtcaccgtctcctca

SEQ ID NO: 169 - DNA, 348 bp, synthetic construct
  source 1..348: mol_type = other DNA
caggtacagctggtggagtctgggggaggattggtgcaggctgggggctctctgagactctcctgtgcagcctctggacgcaccttcaccatggggtggttccgtcaggctccagggaaggagcgtgagtttgtagcagctattagtttgagtcctactttagcatattatgcagagtccgtgaagggccgattcaccatcagccgagacaacgccaagaacacggtggttttgcaaatgaacagcctgaaacctgaggacacggccgtttactactgtgcagcacgtcggatcgacgcagctgactttgattcctgggggcaggggacccaggtcaccgtctcctca

SEQ ID NO: 170 - DNA, 360 bp, synthetic construct
  source 1..360: mol_type = other DNA
caggtacagctggtggagtctgggggaggattggtgcaggctgggggctctctgagactctcctgtgcagcctctggaggcaccttaagtaaaaataccgtggcttggttccgccaggctccagggaaggagcgtgggtttgtagcgtctattacctgggatggtcgtacgacatactatgcagactccgtgaagggccgattcaccatctccagagacaacgccaagaacacagtgtatctgcaaatgaacagcctgaaacctgaggatacggccgtttatgtctgtgcagacttagggaaatggcctgcgggcccggcggactactggggccaggggacccaggtcaccgtctcctca

SEQ ID NO: 171 - DNA, 363 bp, synthetic construct
  source 1..363: mol_type = other DNA
caggtgcagctggtggagtctgggggaggcttggtgcagcctggggggtctctgacactctcctgtgcagcctctggaagcatcgacagtatcaataccatggactggttccgtcaggctccagggaaggagcgtgagtttgtagcagctattagtttgagtcccactttagcatattatgcagagtccgtgaagggccgattcaccatcagccgagacaacgccaagaacacggtggttttgcaaatgaacagcctgaaacctgaggacacggccctttattactgtgcagcagaccggaaatcagtaatgtctattcggcccgactactggggccaggggacccaggtcaccgtctcctca

SEQ ID NO: 172 - DNA, 360 bp, synthetic construct
  source 1..360: mol_type = other DNA
gatgtgcagctggtggagtctgggggaggattggtgcaggctgggggctctctgagactctcctgtgcagcctctggaggcaccttaagtaagaataccgtggcttgggtccgccaggctccagggaaggagcgtgggtttgtaacgtctattacctgtgatggtcgtacgacatactatgcgaactccgtgaagggccgattccccatctccagagacaacgccgagaacacagtgtatctgcaaatgaacagcctgaaacctgaggatacggccggttatgtctgtgcagacttagggaagtggcctgcgggttcggcggactactggggccaggggacccacgtcaccgtctcctcc

SEQ ID NO: 173 - DNA, 363 bp, synthetic construct
  source 1..363: mol_type = other DNA
caggtaaagctggaggagtctgggggaggcttggtgcagcctggggggtctctgagactctcctgtacagcctcggaattcacattcagtgactactggatgcattgggtccgtcaggctccggggaaggggctcgagtgggtcgcatctatagatactagtggacagaccacatactatgcagactccctgaagggccgattcaccatctccagagacaacgccaagagcacgttgtatctgcaaatgaacagtctgaaatctgaagacacgggcgtgtatttctgtgcaaaacgatataggggtggtacctggtatggcatggccaactggggcaaagggacccaggtcaccgtctcctca

SEQ ID NO: 174 - DNA, 360 bp, synthetic construct
  source 1..360: mol_type = other DNA
caggtgcagctggtggagtctgggggaggattggtgcaggctgggggctctctgagactctcctgtgcagcctctggacgcaccttaagtagtaataccatggcttggttccgccaggctccagggaaggagcgtgagtttgtagcgtctactacctggaatggtcgtagcacatactatgcagactccgtgaagggccgattcaccatctccagagacaacgccaagaacacgatgtatctgcaaatgaacagcctgaaacctgaggatacggccgtttatgtctgtgcagacttagggaaatggcctgcgggcccggcggactactggggccaggggacccaggtcaccgtctcctca

SEQ ID NO: 175 - DNA, 348 bp, synthetic construct
  source 1..348: mol_type = other DNA
caggtgcagctggtggagtctgggggaggattggtgcaggctgggggctctctgagactctcctgtgcagcctctggacgcaccttcaccatggggtggttccgtcaggctccagggaagcagcgcgaattggtcgcagatattagtggtggtcgcacaaactatgcagattccgtgaagggacgattcaccatctccagagacaacgccaagaacacggtatatctgcaaatgaacagcctgaaacctgaggacacggccgtttattactgtgcagcagaccggaaatcagtaatgtctattcggcccgactactggggccaggggacccaggtcaccgtctcctca

SEQ ID NO: 176 - DNA, 312 bp, synthetic construct
  source 1..312: mol_type = other DNA
caggtgcagctggtggagtctgggggaggcttggtgcaggctggggcctctctgagactctcctgtgcagcctctggacgcaccttcaccgtggcagctattagtttgagtcctactttagcatattatgcagagtccgtgaagggccgattcaccatcagccgagacaacgccaagaacacggtggttttgcaaatgaacagcctgaaacctgaggacacggccctttattactgtgcagcagaccggaaatcagtaatgtctattcggcccgactactggggccaggggacccaggtcaccgtctcctca

SEQ ID NO: 177 - DNA, 375 bp, synthetic construct
  source 1..375: mol_type = other DNA
gatgtgcagctggtggagtctgggggaggattggagcaggctgggggctctctgagactctcctgtgcagcctctggaggcaccttaagtaaaaataccgtggcttggttccgccaggctccagggaaggagcgtgggtttgtagcgtctattacctgggatggtcgtacgacatactatgcagactccgtgaagggccgattcaccatctccagagacaacgccaagaacacagtgtatctgcaaatgaacagcctgaaacctgaggatacggccgtttattactgtgcgtcgacggcatcgtgccacctcttcggattggggtccggggcctttgtgtcctggggccgggggacccaggtcaccgtctcctca

SEQ ID NO: 178 - DNA, 348 bp, synthetic construct
  source 1..348: mol_type = other DNA
gcggtgcagctggtggagtctgggggaggattggtgcaggctgggggctctctgagactctcctgtgcagcctctggacgcaccttcaccatggggtggttccatcaggctccagggaaggagcgtgagtttgtagcagctattagtttgagtcctactttagcatattatgcagagtccgtgaagggccgattcaccatcagccgagacaacgccaagaacacggtggttttgcaaatgaacagcctgaaacctgaggacacggccctttattactgtgcagcatccaaggatagatattcggaatatgagtactggggccaggggacccaggtcaccgtctcctca

SEQ ID NO: 179 - DNA, 342 bp, synthetic construct
  source 1..342: mol_type = other DNA
caggtaaagctggaggagtctgggggaggattggtgcaggctgggggctctctgagactctcctgtgcagcctctggacgcaccttcaccatggggtggttccgtcaggctccagggaaggagcgtgagtttgtagcagctattagtttgagtcctactttagcatattatgcagagtccgtgaagggccgattcaccatcagccgagacaacgccaagaacacggtggttttgcaaatgaacagcctgaaacctgaggacacggccctttattactgtgcaaaaaaaaacggggggcctgtggactactggggcaaagggacccaggtcaccgtctcctca

SEQ ID NO: 180 - DNA, 357 bp, synthetic construct
  source 1..357: mol_type = other DNA
gatgtgcagctggtggagtctgggggaggcttggtgcagcctggggggtctctgagactctcctgtgcagcctctggacggaccttcagtagcattgtcatgggctggttccgccaggctccagggaaggagcgtgagtttgtaggagcgattatgtggaatgatggtattacatacttgcaagactccgtgaagggccgatttaccatcttcagagacaacgccaagaacacggtgtatctgcaaatgaacagcctgaaacttgaggatacggccgtttattactgtgcagcatccaagggtagatactcggaatatgagtactggggccaggggacccaggtcaccgtctcctca

SEQ ID NO: 181 - DNA, 354 bp, synthetic construct
  source 1..354: mol_type = other DNA
caggtaaagctggaggaatctgggggaagattggtgcaggctgggggctctctgaaactctcctgggcagcctctggacgcaccttcaccatggggtggttccgtcaggctccagggaaggaacgtgagtttgtaacagctattaatttgagtcctactttaacatattatgcagaatccgtgaagggccgattccccatcagccgaaacaacgcccagaacacggtggttttgcaaatgaacagcctgaaacctgaggacacggccctttattactgtgcagcagaacggaaatcagtaatggctattccgcccgactactggggccaggggacccaggtcaccgtctcctca

SEQ ID NO: 182 - DNA, 354 bp, synthetic construct
  source 1..354: mol_type = other DNA
gaggtgcagctggtggagtctgggggaggattggtgcaggctgggggctctctgagactctcctgtgcagcctctggacgcaccttcaccatgggggggttccgtcgggttcctcgggatgagcgggagtttgtagcatctattactttgattcctacttttccttattatgcatattccgtgaagggccgattcgccctcttccgagacaaccccaacaacaccgtgattttgctgatgatcagcctgaaacctgaggacccggacctttattactgtgcttcataccggaaatacctaatgtctattctgcccgactactggggccaggggacccagggcaccgtctcctcc

SEQ ID NO: 183 - DNA, 372 bp, synthetic construct
  source 1..372: mol_type = other DNA
caggtaaagctggaggagtctgggggaggattggtgcaggctgggggctctctgagactctcctgtgcagcctctggacgcaccttcaccatggggtggttccgtcaggctccagggaaggagcgtgagtttgtagcagctattagtttgagtcctactttagcatattatgcagagtccgtgaagggccgattcaccatcagccgagacaacgccaagaacacggtggatctgcaaatgaacagcctgaaacctgaggacacggccgtctatttctgtgcagcaaatcggaactcccaacgggtaattgcggcactgtcctggattggcatgaactactggggcgaatggacccaggtcaccgtctcctcc

SEQ ID NO: 184 - DNA, 348 bp, synthetic construct
  source 1..348: mol_type = other DNA
caggtgcagctggtggagtctgggggaggattggtgcaggctgggggctctctgagactctcctgtgcagcctctggacgcaccttcaccatggggtggttccgtcaggctccagggaaggagcgtgagtttgtagcagctattagtttgagtcctactttagcatattatgcagagtccgtgaagggccgattcaccatctccagagacaacgccaagaagacgctgtatctgcgaatgaatagcctgaaacctgaggacacggccgtttactactgtgcagcacgtcggatcgacgcagctgactttgattcctgggggcaggggacccaggtcaccgtctcctca

SEQ ID NO: 185 - DNA, 348 bp, synthetic construct
  source 1..348: mol_type = other DNA
caggtaaagctggaggagtctgggggaggattggtgcaggctgggggctctctgagactctcctgtgcagcctctggacgcaccttcaccatggggtggttccgtcgggctccagggaaggagcgtgagtctgttgcagttattggctggagagatattaacgcaagctatgcagactccgtgaagggccgattcgccatctccagagacaacgccaagaagacgctgtatctgcagatgaatagcctgaaacctgaggacacggccgtttactactgtgcagcacgtcggatcgacgcaactgactttgattcctgggggcaggggacccaggtcaccgtctcctca

SEQ ID NO: 186 - DNA, 357 bp, synthetic construct
  source 1..357: mol_type = other DNA
caggtaaagctggaggagtctgggggaggattggtgcagactgggggctctctgagactctcctgtgcagcctctgaacacaccttcagtaaccatgtcatgggctggttccgccaggctccagggaaggagcgtgagtctgttgcagttattggctggagagatattagcacaagctatgcagactccgtgaagggccgattcaccatctccagagacaacgccaagaagacgctgtatctgcaaatgaatagcctgaaacctgaggacacggccgtttactactgtgcagcacgtcggatcgacgcagctgactttgattcccgggggcaggggacccaggtcaccgtctcctca

SEQ ID NO: 187 - DNA, 369 bp, synthetic construct
  source 1..369: mol_type = other DNA
gccgtgcagctggtggattctgggggaggattggtgcaggctgggggctctctgagaatttcctgtgcagtctctggacgcacctccagtaactatatattggcctggttccgtcaggctccaggaaaagagcgtgactttgtagcacatattagccggagtggtggtaagtccggctatggagactccgtgaagggccgattcaccatctccagagacaacgccgagaacacggtcagggtgtatctgcaaatgaacagtctgaaacctggggacacggccgtctattactgtaatcgccccctctggtacggaagtcccacgttgattgactactggggccaggggacccaggtcaccgtctcctca

SEQ ID NO: 188 - DNA, 354 bp, synthetic construct
  source 1..354: mol_type = other DNA
gcggtgcagctggtggagtctgggggaggcttggtgcagcctggggggtctctgagactctcctgtgcagcctctggacgcaccttcaccatggggtggttccgtcaggctccagggaaggagcgtgagtttgtagcagctattagtttgagtcctactttagcatattatgcagagtccgtgaagggccgattcaccatcagccgagacaacgccaagaacacggtggttttgcaaatgaacagcctgaaacctgaggacacggccctttattactgtgcagcagaccggaaatcagtaatgtctattcggcccgactactggggccaggggacccaggtcaccgtctcctca

SEQ ID NO: 189 - DNA, 354 bp, synthetic construct
  source 1..354: mol_type = other DNA
gcggtgcagctggtggagtctgggggaggattggtgcaggctgggggctctctgagactctcctgtgcagcctctggacgcaccttcaccatggggtggttccgtcaggctccagggaaggagcgtgagtttgtagcagctattagtttgagtcctactttagcatattatgcagagtccgtgaagggccgattcaccatcagccgagacaacgccaagaacacggtggttttgcaaatgaacagcctgaaacctgaggacacggccctttattactgtgcagcagaccggaaatcagtaatgtctattcggcccgactactggggccaggggacccaggtcaccgtctcctca

SEQ ID NO: 190 - DNA, 363 bp, synthetic construct
  source 1..363: mol_type = other DNA
gatgtgcagctggtggagtctgggggaggatcggtgcagactgggggctctctgagactctcctgtacagcctctggacgcaccctcaataactttgtcatgggctggttccgtcaggctccagggaaggagcgtgagtttgtagcagctattagtttgagtcctactttagcatattatgtagagtccgtgaagggccgattcaccatcagccgagacaacgccaagaacacggtggttttgcaaatgaacagcctgaaacctgaggacacggccctttattactgtgcagcagaccggaaatcagtaatgtctattcggcccgactactggggccaggggacccaggtcaccgtctcctca

SEQ ID NO: 191 - protein, 21 aa, synthetic construct
MALPVTALLLPLALLLHAARP

SEQ ID NO: 192 - protein, 45 aa, synthetic construct
TTTPAPRPPTPAPTIASQPLSLRPEACRPAAGGAVHTRGLDFACD

SEQ ID NO: 193 - protein, 24 aa, synthetic construct
IYIWAPLAGTCGVLLLSLVITLYC

SEQ ID NO: 194 - protein, 27 aa, synthetic construct
FWVLVVVGGVLACYSLLVTVAFIIFWV

SEQ ID NO: 195 - protein, 41 aa, synthetic construct
RSKRSRLLHSDYMNMTPRRPGPTRKHYQPYAPPRDFAAYRS

SEQ ID NO: 196 - protein, 42 aa, synthetic construct
KRGRKKLLYIFKQPFMRPVQTTQEEDGCSCRFPEEEEGGCEL

SEQ ID NO: 197 - protein, 113 aa, synthetic construct
RVKFSRSADAPAYQQGQNQLYNELNLGRREEYDVLDKRRGRDPEMGGKPQRRKNPQEGLYNELQKDKMAEAYSEIGMKGERRRGKGHDGLYQGLSTATKDTYDALHMQALPPR

SEQ ID NO: 198 - protein, 113 aa, synthetic construct
RVKFSRSADAPAYKQGQNQLYNELNLGRREEYDVLDKRRGRDPEMGGKPQRRKNPQEGLYNELQKDKMAEAYSEIGMKGERRRGKGHDGLYQGLSTATKDTYDALHMQALPPR

SEQ ID NO: 199 - DNA, 63 bp, synthetic construct
  source 1..63: mol_type = other DNA
atggccttaccagtgaccgccttgctcctgccgctggccttgctgctccacgccgccaggccg

SEQ ID NO: 200 - DNA, 63 bp, synthetic construct
  source 1..63: mol_type = other DNA
atggctctgcccgtcactgctctgctgctgcccctggctctgctgctgcacgccgcaagaccc

SEQ ID NO: 201 - DNA, 135 bp, synthetic construct
  source 1..135: mol_type = other DNA
accacgacgccagcgccgcgaccaccaacaccggcgcccaccatcgcgtcgcagcccctgtccctgcgcccagaggcgtgccggccagcggcggggggcgcagtgcacacgagggggctggacttcgcctgtgat

SEQ ID NO: 202 - DNA, 72 bp, synthetic construct
  source 1..72: mol_type = other DNA
atctacatctgggcgcccttggccgggacttgtggggtccttctcctgtcactggttatcaccctttactgc

SEQ ID NO: 203 - DNA, 81 bp, synthetic construct
  source 1..81: mol_type = other DNA
ttttgggtgctggtggtggttggtggagtcctggcttgctatagcttgctagtaacagtggcctttattattttctgggtg

SEQ ID NO: 204 - DNA, 123 bp, synthetic construct
  source 1..123: mol_type = other DNA
aggagtaagaggagcaggctcctgcacagtgactacatgaacatgactccccgccgccccgggcccacccgcaagcattaccagccctatgccccaccacgcgacttcgcagcctatcgctcc

SEQ ID NO: 205 - DNA, 126 bp, synthetic construct
  source 1..126: mol_type = other DNA
aaacggggcagaaagaaactcctgtatatattcaaacaaccatttatgagaccagtacaaactactcaagaggaagatggctgtagctgccgatttccagaagaagaagaaggaggatgtgaactg

SEQ ID NO: 206 - DNA, 336 bp, synthetic construct
  source 1..336: mol_type = other DNA
agagtgaagttcagcaggagcgcagacgcccccgcgtaccagcagggccagaaccagctctataacgagctcaatctaggacgaagagaggagtacgatgttttggacaagagacgtggccgggaccctgagatggggggaaagccgagaaggaagaaccctcaggaaggcctgtacaatgaactgcagaaagataagatggcggaggcctacagtgagattgggatgaaaggcgagcgccggaggggcaaggggcacgatggcctttaccagggtctcagtacagccaccaaggacacctacgacgcccttcacatgcaggccctgccccctcgc

SEQ ID NO: 207 - DNA, 336 bp, synthetic construct
  source 1..336: mol_type = other DNA
agagtgaagttcagcaggagcgcagacgcccccgcgtacaagcagggccagaaccagctctataacgagctcaatctaggacgaagagaggagtacgatgttttggacaagagacgtggccgggaccctgagatggggggaaagccgagaaggaagaaccctcaggaaggcctgtacaatgaactgcagaaagataagatggcggaggcctacagtgagattgggatgaaaggcgagcgccggaggggcaaggggcacgatggcctttaccagggtctcagtacagccaccaaggacacctacgacgcccttcacatgcaggccctgccccctcgc

SEQ ID NO: 208 - protein, 5 aa, synthetic construct
GGGGS

SEQ ID NO: 209 - protein, 10 aa, synthetic construct
GGGGSGGGGS

SEQ ID NO: 210 - protein, 16 aa, synthetic construct
GGGSGGGSGGGSGGGS

SEQ ID NO: 211 - protein, 24 aa, synthetic construct
GGGGSGGGGSGGGGGGSGSGGGGS

SEQ ID NO: 212 - protein, 34 aa, synthetic construct
GGGGSGGGGSGGGGGGSGSGGGGSGGGGSGGGGS

SEQ ID NO: 213 - protein, 15 aa, synthetic construct
GGGGSGGGGSGGGGS

SEQ ID NO: 214 - protein, 20 aa, synthetic construct
GGGGSGGGGSGGGGSGGGGS

SEQ ID NO: 215 - protein, 25 aa, synthetic construct
GGGGSGGGGSGGGGSGGGGSGGGGS

SEQ ID NO: 216 - protein, 420 aa, synthetic construct
MALPVTALLLPLALLLHAARPVNRTRRMHQVQLVESGGGLVQPGGSLRLSCEASGFTLDYYAIGWFRQAPGKEREGVICISRSDGSTYYADSVKGRFTISRDNAKKTVYLQMISLKPEDTAAYYCAAGADCSGYLRDYEFRGQGTQVTVSSTSTTTPAPRPPTPAPTIASQPLSLRPEACRPAAGGAVHTRGLDFACDFWVLVVVGGVLACYSLLVTVAFIIFWVRSKRSRLLHSDYMNMTPRRPGPTRKHYQPYAPPRDFAAYRSKRGRKKLLYIFKQPFMRPVQTTQEEDGCSCRFPEEEEGGCELRVKFSRSADAPAYKQGQNQLYNELNLGRREEYDVLDKRRGRDPEMGGKPRRKNPQEGLYNELQKDKMAEAYSEIGMKGERRRGKGHDGLYQGLSTATKDTYDALHMQALPPR

SEQ ID NO: 217 - protein, 426 aa, synthetic construct
MALPVTALLLPLALLLHAARPVNRTRRMHQVKLEESGGRLVQPRGSLRLSCAGSGRTFSTYGMAWFRQAPGKEREFVASKASMNYSGRTYYADSVKGRFTIARDNAKNMVFLQMNNLKPEDTAVYYCAAGTGCSTYGCFDAQIIDYWGKGTLVTVSSTSTTTPAPRPPTPAPTIASQPLSLRPEACRPAAGGAVHTRGLDFACDFWVLVVVGGVLACYSLLVTVAFIIFWVRSKRSRLLHSDYMNMTPRRPGPTRKHYQPYAPPRDFAAYRSKRGRKKLLYIFKQPFMRPVQTTQEEDGCSCRFPEEEEGGCELRVKFSRSADAPAYKQGQNQLYNELNLGRREEYDVLDKRRGRDPEMGGKPRRKNPQEGLYNELQKDKMAEAYSEIGMKGERRRGKGHDGLYQGLSTATKDTYDALHMQALPPR

SEQ ID NO: 218 - protein, 416 aa, synthetic construct
MALPVTALLLPLALLLHAARPVNRTRRMHEVQLVESGGGLVQAGGSLRLSCAASGRTFTMGWFRQAPGKEREFVAAISLSPTLAYYAESVKGRFTISRDNAKNTVVLQMNSLKPEDTALYYCAADRKSVMSIRPDYWGQGTQVTVSSTSTTTPAPRPPTPAPTIASQPLSLRPEACRPAAGGAVHTRGLDFACDFWVLVVVGGVLACYSLLVTVAFIIFWVRSKRSRLLHSDYMNMTPRRPGPTRKHYQPYAPPRDFAAYRSKRGRKKLLYIFKQPFMRPVQTTQEEDGCSCRFPEEEEGGCELRVKFSRSADAPAYKQGQNQLYNELNLGRREEYDVLDKRRGRDPEMGGKPRRKNPQEGLYNELQKDKMAEAYSEIGMKGERRRGKGHDGLYQGLSTATKDTYDALHMQALPPR

SEQ ID NO: 219 - protein, 418 aa, synthetic construct
MALPVTALLLPLALLLHAARPVNRTRRMHAVQLVDSGGGLVQPGGSLRLSCVASGGIFVINAMGWYRQAPGKQRELVASIRGLGRTNYDDSVKGRFTISRDNANNTVYLQMNSLEPEDTAVYYCTVYVTLLGGVNRDYWGQGTQVTVSSTSTTTPAPRPPTPAPTIASQPLSLRPEACRPAAGGAVHTRGLDFACDFWVLVVVGGVLACYSLLVTVAFIIFWVRSKRSRLLHSDYMNMTPRRPGPTRKHYQPYAPPRDFAAYRSKRGRKKLLYIFKQPFMRPVQTTQEEDGCSCRFPEEEEGGCELRVKFSRSADAPAYKQGQNQLYNELNLGRREEYDVLDKRRGRDPEMGGKPRRKNPQEGLYNELQKDKMAEAYSEIGMKGERRRGKGHDGLYQGLSTATKDTYDALHMQALPPR

SEQ ID NO: 220 - protein, 417 aa, synthetic construct
MALPVTALLLPLALLLHAARPVNRTRRMHEVQLVESGGGLVQAGGSLRLSCAASGRTFSSIVMGWFRQAPGKEREFVGAIMWNDGITYLQDSVKGRFTIFRDNAKNTVYLQMNSLKLEDTAVYYCAASKGRYSEYEYWGQGTQVTVSSTSTTTPAPRPPTPAPTIASQPLSLRPEACRPAAGGAVHTRGLDFACDFWVLVVVGGVLACYSLLVTVAFIIFWVRSKRSRLLHSDYMNMTPRRPGPTRKHYQPYAPPRDFAAYRSKRGRKKLLYIFKQPFMRPVQTTQEEDGCSCRFPEEEEGGCELRVKFSRSADAPAYKQGQNQLYNELNLGRREEYDVLDKRRGRDPEMGGKPRRKNPQEGLYNELQKDKMAEAYSEIGMKGERRRGKGHDGLYQGLSTATKDTYDALHMQALPPR

SEQ ID NO: 221 - protein, 426 aa, synthetic construct
MALPVTALLLPLALLLHAARPVNRTRRMHEVQLVESGGGVVQAGGSLTVSCTASGFTFDRAVIVWFRQAPGKGREGVSFIKPSDGTIYYIDSLKGRFTISSDIAKNTVYLQMKSLESEDSAVYYCAASPEDWYTDWIDWSIYRWQHWGQGTQVTVSSTSTTTPAPRPPTPAPTIASQPLSLRPEACRPAAGGAVHTRGLDFACDFWVLVVVGGVLACYSLLVTVAFIIFWVRSKRSRLLHSDYMNMTPRRPGPTRKHYQPYAPPRDFAAYRSKRGRKKLLYIFKQPFMRPVQTTQEEDGCSCRFPEEEEGGCELRVKFSRSADAPAYKQGQNQLYNELNLGRREEYDVLDKRRGRDPEMGGKPRRKNPQEGLYNELQKDKMAEAYSEIGMKGERRRGKGHDGLYQGLSTATKDTYDALHMQALPPR

SEQ ID NO: 222 - protein, 417 aa, synthetic construct
MALPVTALLLPLALLLHAARPVNRTRRMHEVQLVESGGGMVQAGDSLRLSCVQSTYTVNSDVMGWFRQAPGKEREFVGAIMWNDGITYLQDSVKGRFTIFRDNAKNTVYLQMNSLKLEDTAVYYCAASKGRYSEYEYWGQGTQVTVSSTSTTTPAPRPPTPAPTIASQPLSLRPEACRPAAGGAVHTRGLDFACDFWVLVVVGGVLACYSLLVTVAFIIFWVRSKRSRLLHSDYMNMTPRRPGPTRKHYQPYAPPRDFAAYRSKRGRKKLLYIFKQPFMRPVQTTQEEDGCSCRFPEEEEGGCELRVKFSRSADAPAYKQGQNQLYNELNLGRREEYDVLDKRRGRDPEMGGKPRRKNPQEGLYNELQKDKMAEAYSEIGMKGERRRGKGHDGLYQGLSTATKDTYDALHMQALPPR

SEQ ID NO: 223 - protein, 418 aa, synthetic construct
MALPVTALLLPLALLLHAARPVNRTRRMHAVQLVESGGGLVQAGDSLRLSCTASGATLTNDHMAWFRQAPGKGREFVAAIDWSGRTTNYADPVEGRFTISRNNAKNTVYLEMNSLKLEDTAVYYCAVLRAWISYDNDYWGQGTQVTVSSTSTTTPAPRPPTPAPTIASQPLSLRPEACRPAAGGAVHTRGLDFACDFWVLVVVGGVLACYSLLVTVAFIIFWVRSKRSRLLHSDYMNMTPRRPGPTRKHYQPYAPPRDFAAYRSKRGRKKLLYIFKQPFMRPVQTTQEEDGCSCRFPEEEEGGCELRVKFSRSADAPAYKQGQNQLYNELNLGRREEYDVLDKRRGRDPEMGGKPRRKNPQEGLYNELQKDKMAEAYSEIGMKGERRRGKGHDGLYQGLSTATKDTYDALHMQALPPR

SEQ ID NO: 224 - protein, 418 aa, synthetic construct
MALPVTALLLPLALLLHAARPVNRTRRMHQVQLVESGGGLVQAGGSLRLSCAASGGTLSKNTVAWFRQAPGKERGFVASITWDGRTTYYADSVKGRFTISRDNAKNTVYLQMNSLKPEDTAVYVCADLGKWPAGPADYWGQGTQVTVSSTSTTTPAPRPPTPAPTIASQPLSLRPEACRPAAGGAVHTRGLDFACDFWVLVVVGGVLACYSLLVTVAFIIFWVRSKRSRLLHSDYMNMTPRRPGPTRKHYQPYAPPRDFAAYRSKRGRKKLLYIFKQPFMRPVQTTQEEDGCSCRFPEEEEGGCELRVKFSRSADAPAYKQGQNQLYNELNLGRREEYDVLDKRRGRDPEMGGKPRRKNPQEGLYNELQKDKMAEAYSEIGMKGERRRGKGHDGLYQGLSTATKDTYDALHMQALPPR

SEQ ID NO: 225 - protein, 417 aa, synthetic construct
MALPVTALLLPLALLLHAARPVNRTRRMHQVKLEESGGGLVQAGRSLRLSCAASEHTFSSHVMGWFRQAPGKERESVAVIGWRDISTSYADSVKGRFTISRDNAKKTLYLQMNSLKPEDTAVYYCAARRIDAADFDSWGQGTQVTVSSTSTTTPAPRPPTPAPTIASQPLSLRPEACRPAAGGAVHTRGLDFACDFWVLVVVGGVLACYSLLVTVAFIIFWVRSKRSRLLHSDYMNMTPRRPGPTRKHYQPYAPPRDFAAYRSKRGRKKLLYIFKQPFMRPVQTTQEEDGCSCRFPEEEEGGCELRVKFSRSADAPAYKQGQNQLYNELNLGRREEYDVLDKRRGRDPEMGGKPRRKNPQEGLYNELQKDKMAEAYSEIGMKGERRRGKGHDGLYQGLSTATKDTYDALHMQALPPR

SEQ ID NO: 226 - protein, 417 aa, synthetic construct
MALPVTALLLPLALLLHAARPVNRTRRMHAVQLVESGGGLVQAGDSLRLTCTASGRAFSTYFMAWFRQAPGKEREFVAGIAWSGGSTAYADSVKGRFTISRDNAKNTVYLQMNSLKSEDTAVYYCASRGIEVEEFGAWGQGTQVTVSSTSTTTPAPRPPTPAPTIASQPLSLRPEACRPAAGGAVHTRGLDFACDFWVLVVVGGVLACYSLLVTVAFIIFWVRSKRSRLLHSDYMNMTPRRPGPTRKHYQPYAPPRDFAAYRSKRGRKKLLYIFKQPFMRPVQTTQEEDGCSCRFPEEEEGGCELRVKFSRSADAPAYKQGQNQLYNELNLGRREEYDVLDKRRGRDPEMGGKPRRKNPQEGLYNELQKDKMAEAYSEIGMKGERRRGKGHDGLYQGLSTATKDTYDALHMQALPPR

SEQ ID NO: 227 - protein, 376 aa, synthetic construct
MALPVTALLLPLALLLHAARPVNRTRRMHQVQLVESGGGLVQPGGSLRLSCEASGFTLDYYAIGWFRQAPGKEREGVICISRSDGSTYYADSVKGRFTISRDNAKKTVYLQMISLKPEDTAAYYCAAGADCSGYLRDYEFRGQGTQVTVSSTSTTTPAPRPPTPAPTIASQPLSLRPEACRPAAGGAVHTRGLDFACDIYIWAPLAGTCGVLLLSLVITLYCKRGRKKLLYIFKQPFMRPVQTTQEEDGCSCRFPEEEEGGCELRVKFSRSADAPAYQQGQNQLYNELNLGRREEYDVLDKRRGRDPEMGGKPRRKNPQEGLYNELQKDKMAEAYSEIGMKGERRRGKGHDGLYQGLSTATKDTYDALHMQALPPR

SEQ ID NO: 228 - protein, 373 aa, synthetic construct
MALPVTALLLPLALLLHAARPVNRTRRMHQVKLEESGGGLVQAGRSLRLSCAASEHTFSSHVMGWFRQAPGKERESVAVIGWRDISTSYADSVKGRFTISRDNAKKTLYLQMNSLKPEDTAVYYCAARRIDAADFDSWGQGTQVTVSSTSTTTPAPRPPTPAPTIASQPLSLRPEACRPAAGGAVHTRGLDFACDIYIWAPLAGTCGVLLLSLVITLYCKRGRKKLLYIFKQPFMRPVQTTQEEDGCSCRFPEEEEGGCELRVKFSRSADAPAYQQGQNQLYNELNLGRREEYDVLDKRRGRDPEMGGKPRRKNPQEGLYNELQKDKMAEAYSEIGMKGERRRGKGHDGLYQGLSTATKDTYDALHMQALPPR

SEQ ID NO: 229 - protein, 372 aa, synthetic construct
MALPVTALLLPLALLLHAARPVNRTRRMHEVQLVESGGGLVQAGGSLRLSCAASGRTFTMGWFRQAPGKEREFVAAISLSPTLAYYAESVKGRFTISRDNAKNTVVLQMNSLKPEDTALYYCAADRKSVMSIRPDYWGQGTQVTVSSTSTTTPAPRPPTPAPTIASQPLSLRPEACRPAAGGAVHTRGLDFACDIYIWAPLAGTCGVLLLSLVITLYCKRGRKKLLYIFKQPFMRPVQTTQEEDGCSCRFPEEEEGGCELRVKFSRSADAPAYQQGQNQLYNELNLGRREEYDVLDKRRGRDPEMGGKPRRKNPQEGLYNELQKDKMAEAYSEIGMKGERRRGKGHDGLYQGLSTATKDTYDALHMQALPPR

SEQ ID NO: 230 - protein, 372 aa, synthetic construct
MALPVTALLLPLALLLHAARPEVQLVESGGGLVPPGGSLRLSCTASGSTVSINVMAWYRQVSGKQRELVAAVTRDGRKSCGDSVKGRFTISRDGAKNAVYLQMNSLKPEDTAVYLCGADGWGATTLDYTYGMDYWGKGTQVTVSSAATSTTTPAPRPPTPAPTIASQPLSLRPEACRPAAGGAVHTRGLDFACDIYIWAPLAGTCGVLLLSLVITLYCKRGRKKLLYIFKQPFMRPVQTTQEEDGCSCRFPEEEEGGCELRVKFSRSADAPAYQQGQNQLYNELNLGRREEYDVLDKRRGRDPEMGGKPRRKNPQEGLYNELQKDKMAEAYSEIGMKGERRRGKGHDGLYQGLSTATKDTYDALHMQALPPR

SEQ ID NO: 231 - protein, 364 aa, synthetic construct
MALPVTALLLPLALLLHAARPAVQLVESGGGLVQAGGSLRLSCAASGRTFTMGWFRQAPGKERGFVASITWDGRSAYYAESVKGRFTISRDNAKNTVVLQMNSLKPEDTALYYCAADRKSVMSIRPDYWGQGTQVTVSSTSTTTPAPRPPTPAPTIASQPLSLRPEACRPAAGGAVHTRGLDFACDIYIWAPLAGTCGVLLLSLVITLYCKRGRKKLLYIFKQPFMRPVQTTQEEDGCSCRFPEEEEGGCELRVKFSRSADAPAYQQGQNQLYNELNLGRREEYDVLDKRRGRDPEMGGKPRRKNPQEGLYNELQKDKMAEAYSEIGMKGERRRGKGHDGLYQGLSTATKDTYDALHMQALPPR

SEQ ID NO: 232 - protein, 368 aa, synthetic construct
MALPVTALLLPLALLLHAARPQVQLVESGGGLVQPGGSLRLACEAPGSGNSINAMGWYRQTPGKRRELVATITRGGSTNYGPSVKGRFTITRDNVKNTVHLQMNSLKPDDTAVYYCNAERLDGSGYGYEYDYWGQGTQVTVSSTSTTTPAPRPPTPAPTIASQPLSLRPEACRPAAGGAVHTRGLDFACDIYIWAPLAGTCGVLLLSLVITLYCKRGRKKLLYIFKQPFMRPVQTTQEEDGCSCRFPEEEEGGCELRVKFSRSADAPAYQQGQNQLYNELNLGRREEYDVLDKRRGRDPEMGGKPRRKNPQEGLYNELQKDKMAEAYSEIGMKGERRRGKGHDGLYQGLSTATKDTYDALHMQALPPR

SEQ ID NO: 233 - protein, 367 aa, synthetic construct
MALPVTALLLPLALLLHAARPQVKLEESGGGLVQAGGSLRLSCAASGGTLSKNTVAWVRQAPGKERGFVTSITCDGRTTYYANSVNGRFPINRNNAENLVVLQMNSLKPDDTALYYCAAYRKSIMSIQPDYWGQGTQVTVSSTSTTTPAPRPPTPAPTIASQPLSLRPEACRPAAGGAVHTRGLDFACDIYIWAPLAGTCGVLLLSLVITLYCKRGRKKLLYIFKQPFMRPVQTTQEEDGCSCRFPEEEEGGCELRVKFSRSADAPAYQQGQNQLYNELNLGRREEYDVLDKRRGRDPEMGGKPRRKNPQEGLYNELQKDKMAEAYSEIGMKGERRRGKGHDGLYQGLSTATKDTYDALHMQALPPR

SEQ ID NO: 234 - protein, 367 aa, synthetic construct
MALPVTALLLPLALLLHAARPDVQLVESGGGLVQAGGSLRLSCAASGRTFSSIVMGWFRQAPGKEREFVGAIMWNDGLTYLQGSVKGRFTISRDNAKNTVVLQMNSLKPEDTALYYCAADRKSVMSIRPDYWGQGTQVTVSSTSTTTPAPRPPTPAPTIASQPLSLRPEACRPAAGGAVHTRGLDFACDIYIWAPLAGTCGVLLLSLVITLYCKRGRKKLLYIFKQPFMRPVQTTQEEDGCSCRFPEEEEGGCELRVKFSRSADAPAYQQGQNQLYNELNLGRREEYDVLDKRRGRDPEMGGKPRRKNPQEGLYNELQKDKMAEAYSEIGMKGERRRGKGHDGLYQGLSTATKDTYDALHMQALPPR

SEQ ID NO: 235 - protein, 362 aa, synthetic construct
MALPVTALLLPLALLLHAARPQVQLVESGGGLVQAGGSLRLSCAASGRTFTMGWFRQAPGKEREFVAAISLSPTLAYYAESVKGRFTISRDNAKNTVVLQMNSLKPEDTAVYYCAARRIDAADFDSWGQGTQVTVSSTSTTTPAPRPPTPAPTIASQPLSLRPEACRPAAGGAVHTRGLDFACDIYIWAPLAGTCGVLLLSLVITLYCKRGRKKLLYIFKQPFMRPVQTTQEEDGCSCRFPEEEEGGCELRVKFSRSADAPAYQQGQNQLYNELNLGRREEYDVLDKRRGRDPEMGGKPRRKNPQEGLYNELQKDKMAEAYSEIGMKGERRRGKGHDGLYQGLSTATKDTYDALHMQALPPR

SEQ ID NO: 236 - protein, 366 aa, synthetic construct
MALPVTALLLPLALLLHAARPQVQLVESGGGLVQAGGSLRLSCAASGGTLSKNTVAWFRQAPGKERGFVASITWDGRTTYYADSVKGRFTISRDNAKNTVYLQMNSLKPEDTAVYVCADLGKWPAGPADYWGQGTQVTVSSTSTTTPAPRPPTPAPTIASQPLSLRPEACRPAAGGAVHTRGLDFACDIYIWAPLAGTCGVLLLSLVITLYCKRGRKKLLYIFKQPFMRPVQTTQEEDGCSCRFPEEEEGGCELRVKFSRSADAPAYQQGQNQLYNELNLGRREEYDVLDKRRGRDPEMGGKPRRKNPQEGLYNELQKDKMAEAYSEIGMKGERRRGKGHDGLYQGLSTATKDTYDALHMQALPPR

SEQ ID NO: 237 - protein, 367 aa, synthetic construct
MALPVTALLLPLALLLHAARPQVQLVESGGGLVQPGGSLTLSCAASGSIDSINTMDWFRQAPGKEREFVAAISLSPTLAYYAESVKGRFTISRDNAKNTVVLQMNSLKPEDTALYYCAADRKSVMSIRPDYWGQGTQVTVSSTSTTTPAPRPPTPAPTIASQPLSLRPEACRPAAGGAVHTRGLDFACDIYIWAPLAGTCGVLLLSLVITLYCKRGRKKLLYIFKQPFMRPVQTTQEEDGCSCRFPEEEEGGCELRVKFSRSADAPAYQQGQNQLYNELNLGRREEYDVLDKRRGRDPEMGGKPRRKNPQEGLYNELQKDKMAEAYSEIGMKGERRRGKGHDGLYQGLSTATKDTYDALHMQALPPR

SEQ ID NO: 238 - protein, 366 aa, synthetic construct
MALPVTALLLPLALLLHAARPDVQLVESGGGLVQAGGSLRLSCAASGGTLSKNTVAWVRQAPGKERGFVTSITCDGRTTYYANSVKGRFPISRDNAENTVYLQMNSLKPEDTAGYVCADLGKWPAGSADYWGQGTHVTVSSTSTTTPAPRPPTPAPTIASQPLSLRPEACRPAAGGAVHTRGLDFACDIYIWAPLAGTCGVLLLSLVITLYCKRGRKKLLYIFKQPFMRPVQTTQEEDGCSCRFPEEEEGGCELRVKFSRSADAPAYQQGQNQLYNELNLGRREEYDVLDKRRGRDPEMGGKPRRKNPQEGLYNELQKDKMAEAYSEIGMKGERRRGKGHDGLYQGLSTATKDTYDALHMQALPPR

SEQ ID NO: 239 - protein, 367 aa, synthetic construct
MALPVTALLLPLALLLHAARPQVKLEESGGGLVQPGGSLRLSCTASEFTFSDYWMHWVRQAPGKGLEWVASIDTSGQTTYYADSLKGRFTISRDNAKSTLYLQMNSLKSEDTGVYFCAKRYRGGTWYGMANWGKGTQVTVSSTSTTTPAPRPPTPAPTIASQPLSLRPEACRPAAGGAVHTRGLDFACDIYIWAPLAGTCGVLLLSLVITLYCKRGRKKLLYIFKQPFMRPVQTTQEEDGCSCRFPEEEEGGCELRVKFSRSADAPAYQQGQNQLYNELNLGRREEYDVLDKRRGRDPEMGGKPRRKNPQEGLYNELQKDKMAEAYSEIGMKGERRRGKGHDGLYQGLSTATKDTYDALHMQALPPR

SEQ ID NO: 240 - protein, 366 aa, synthetic construct
MALPVTALLLPLALLLHAARPQVQLVESGGGLVQAGGSLRLSCAASGRTLSSNTMAWFRQAPGKEREFVASTTWNGRSTYYADSVKGRFTISRDNAKNTMYLQMNSLKPEDTAVYVCADLGKWPAGPADYWGQGTQVTVSSTSTTTPAPRPPTPAPTIASQPLSLRPEACRPAAGGAVHTRGLDFACDIYIWAPLAGTCGVLLLSLVITLYCKRGRKKLLYIFKQPFMRPVQTTQEEDGCSCRFPEEEEGGCELRVKFSRSADAPAYQQGQNQLYNELNLGRREEYDVLDKRRGRDPEMGGKPRRKNPQEGLYNELQKDKMAEAYSEIGMKGERRRGKGHDGLYQGLSTATKDTYDALHMQALPPR

SEQ ID NO: 241 - protein, 362 aa, synthetic construct
MALPVTALLLPLALLLHAARPQVQLVESGGGLVQAGGSLRLSCAASGRTFTMGWFRQAPGKQRELVADISGGRTNYADSVKGRFTISRDNAKNTVYLQMNSLKPEDTAVYYCAADRKSVMSIRPDYWGQGTQVTVSSTSTTTPAPRPPTPAPTIASQPLSLRPEACRPAAGGAVHTRGLDFACDIYIWAPLAGTCGVLLLSLVITLYCKRGRKKLLYIFKQPFMRPVQTTQEEDGCSCRFPEEEEGGCELRVKFSRSADAPAYQQGQNQLYNELNLGRREEYDVLDKRRGRDPEMGGKPRRKNPQEGLYNELQKDKMAEAYSEIGMKGERRRGKGHDGLYQGLSTATKDTYDALHMQALPPR

SEQ ID NO: 242 - protein, 350 aa, synthetic construct
MALPVTALLLPLALLLHAARPQVQLVESGGGLVQAGASLRLSCAASGRTFTVAAISLSPTLAYYAESVKGRFTISRDNAKNTVVLQMNSLKPEDTALYYCAADRKSVMSIRPDYWGQGTQVTVSSTSTTTPAPRPPTPAPTIASQPLSLRPEACRPAAGGAVHTRGLDFACDIYIWAPLAGTCGVLLLSLVITLYCKRGRKKLLYIFKQPFMRPVQTTQEEDGCSCRFPEEEEGGCELRVKFSRSADAPAYQQGQNQLYNELNLGRREEYDVLDKRRGRDPEMGGKPRRKNPQEGLYNELQKDKMAEAYSEIGMKGERRRGKGHDGLYQGLSTATKDTYDALHMQALPPR

SEQ ID NO: 243 - protein, 371 aa, synthetic construct
MALPVTALLLPLALLLHAARPDVQLVESGGGLEQAGGSLRLSCAASGGTLSKNTVAWFRQAPGKERGFVASITWDGRTTYYADSVKGRFTISRDNAKNTVYLQMNSLKPEDTAVYYCASTASCHLFGLGSGAFVSWGRGTQVTVSSTSTTTPAPRPPTPAPTIASQPLSLRPEACRPAAGGAVHTRGLDFACDIYIWAPLAGTCGVLLLSLVITLYCKRGRKKLLYIFKQPFMRPVQTTQEEDGCSCRFPEEEEGGCELRVKFSRSADAPAYQQGQNQLYNELNLGRREEYDVLDKRRGRDPEMGGKPRRKNPQEGLYNELQKDKMAEAYSEIGMKGERRRGKGHDGLYQGLSTATKDTYDALHMQALPPR

SEQ ID NO: 244 - protein, 362 aa, synthetic construct
MALPVTALLLPLALLLHAARPAVQLVESGGGLVQAGGSLRLSCAASGRTFTMGWFHQAPGKEREFVAAISLSPTLAYYAESVKGRFTISRDNAKNTVVLQMNSLKPEDTALYYCAASKDRYSEYEYWGQGTQVTVSSTSTTTPAPRPPTPAPTIASQPLSLRPEACRPAAGGAVHTRGLDFACDIYIWAPLAGTCGVLLLSLVITLYCKRGRKKLLYIFKQPFMRPVQTTQEEDGCSCRFPEEEEGGCELRVKFSRSADAPAYQQGQNQLYNELNLGRREEYDVLDKRRGRDPEMGGKPRRKNPQEGLYNELQKDKMAEAYSEIGMKGERRRGKGHDGLYQGLSTATKDTYDALHMQALPPR

SEQ ID NO: 245 - protein, 360 aa, synthetic construct
MALPVTALLLPLALLLHAARPQVKLEESGGGLVQAGGSLRLSCAASGRTFTMGWFRQAPGKEREFVAAISLSPTLAYYAESVKGRFTISRDNAKNTVVLQMNSLKPEDTALYYCAKKNGGPVDYWGKGTQVTVSSTSTTTPAPRPPTPAPTIASQPLSLRPEACRPAAGGAVHTRGLDFACDIYIWAPLAGTCGVLLLSLVITLYCKRGRKKLLYIFKQPFMRPVQTTQEEDGCSCRFPEEEEGGCELRVKFSRSADAPAYQQGQNQLYNELNLGRREEYDVLDKRRGRDPEMGGKPRRKNPQEGLYNELQKDKMAEAYSEIGMKGERRRGKGHDGLYQGLSTATKDTYDALHMQALPPR

SEQ ID NO: 246 - protein, 365 aa, synthetic construct
MALPVTALLLPLALLLHAARPDVQLVESGGGLVQPGGSLRLSCAASGRTFSSIVMGWFRQAPGKEREFVGAIMWNDGITYLQDSVKGRFTIFRDNAKNTVYLQMNSLKLEDTAVYYCAASKGRYSEYEYWGQGTQVTVSSTSTTTPAPRPPTPAPTIASQPLSLRPEACRPAAGGAVHTRGLDFACDIYIWAPLAGTCGVLLLSLVITLYCKRGRKKLLYIFKQPFMRPVQTTQEEDGCSCRFPEEEEGGCELRVKFSRSADAPAYQQGQNQLYNELNLGRREEYDVLDKRRGRDPEMGGKPRRKNPQEGLYNELQKDKMAEAYSEIGMKGERRRGKGHDGLYQGLSTATKDTYDALHMQALPPR

SEQ ID NO: 247 - protein, 364 aa, synthetic construct
MALPVTALLLPLALLLHAARPQVKLEESGGRLVQAGGSLKLSWAASGRTFTMGWFRQAPGKEREFVTAINLSPTLTYYAESVKGRFPISRNNAQNTVVLQMNSLKPEDTALYYCAAERKSVMAIPPDYWGQGTQVTVSSTSTTTPAPRPPTPAPTIASQPLSLRPEACRPAAGGAVHTRGLDFACDIYIWAPLAGTCGVLLLSLVITLYCKRGRKKLLYIFKQPFMRPVQTTQEEDGCSCRFPEEEEGGCELRVKFSRSADAPAYQQGQNQLYNELNLGRREEYDVLDKRRGRDPEMGGKPRRKNPQEGLYNELQKDKMAEAYSEIGMKGERRRGKGHDGLYQGLSTATKDTYDALHMQALPPR

SEQ ID NO: 248 - protein, 364 aa, synthetic construct
MALPVTALLLPLALLLHAARPEVQLVESGGGLVQAGGSLRLSCAASGRTFTMGGFRRVPRDEREFVASITLIPTFPYYAYSVKGRFALFRDNPNNTVILLMISLKPEDPDLYYCASYRKYLMSILPDYWGQGTQGTVSSTSTTTPAPRPPTPAPTIASQPLSLRPEACRPAAGGAVHTRGLDFACDIYIWAPLAGTCGVLLLSLVITLYCKRGRKKLLYIFKQPFMRPVQTTQEEDGCSCRFPEEEEGGCELRVKFSRSADAPAYQQGQNQLYNELNLGRREEYDVLDKRRGRDPEMGGKPRRKNPQEGLYNELQKDKMAEAYSEIGMKGERRRGKGHDGLYQGLSTATKDTYDALHMQALPPR

SEQ ID NO: 249 - protein, 370 aa, synthetic construct
MALPVTALLLPLALLLHAARPQVKLEESGGGLVQAGGSLRLSCAASGRTFTMGWFRQAPGKEREFVAAISLSPTLAYYAESVKGRFTISRDNAKNTVDLQMNSLKPEDTAVYFCAANRNSQRVIAALSWIGMNYWGEWTQVTVSSTSTTTPAPRPPTPAPTIASQPLSLRPEACRPAAGGAVHTRGLDFACDIYIWAPLAGTCGVLLLSLVITLYCKRGRKKLLYIFKQPFMRPVQTTQEEDGCSCRFPEEEEGGCELRVKFSRSADAPAYQQGQNQLYNELNLGRREEYDVLDKRRGRDPEMGGKPRRKNPQEGLYNELQKDKMAEAYSEIGMKGERRRGKGHDGLYQGLSTATKDTYDALHMQALPPR

SEQ ID NO: 250 - protein, 362 aa, synthetic construct
MALPVTALLLPLALLLHAARPQVQLVESGGGLVQAGGSLRLSCAASGRTFTMGWFRQAPGKEREFVAAISLSPTLAYYAESVKGRFTISRDNAKKTLYLRMNSLKPEDTAVYYCAARRIDAADFDSWGQGTQVTVSSTSTTTPAPRPPTPAPTIASQPLSLRPEACRPAAGGAVHTRGLDFACDIYIWAPLAGTCGVLLLSLVITLYCKRGRKKLLYIFKQPFMRPVQTTQEEDGCSCRFPEEEEGGCELRVKFSRSADAPAYQQGQNQLYNELNLGRREEYDVLDKRRGRDPEMGGKPRRKNPQEGLYNELQKDKMAEAYSEIGMKGERRRGKGHDGLYQGLSTATKDTYDALHMQALPPR

SEQ ID NO: 251 - protein, 362 aa, synthetic construct
MALPVTALLLPLALLLHAARPQVKLEESGGGLVQAGGSLRLSCAASGRTFTMGWFRRAPGKERESVAVIGWRDINASYADSVKGRFAISRDNAKKTLYLQMNSLKPEDTAVYYCAARRIDATDFDSWGQGTQVTVSSTSTTTPAPRPPTPAPTIASQPLSLRPEACRPAAGGAVHTRGLDFACDIYIWAPLAGTCGVLLLSLVITLYCKRGRKKLLYIFKQPFMRPVQTTQEEDGCSCRFPEEEEGGCELRVKFSRSADAPAYQQGQNQLYNELNLGRREEYDVLDKRRGRDPEMGGKPRRKNPQEGLYNELQKDKMAEAYSEIGMKGERRRGKGHDGLYQGLSTATKDTYDALHMQALPPR

SEQ ID NO: 252 - protein, 365 aa, synthetic construct
MALPVTALLLPLALLLHAARPQVKLEESGGGLVQTGGSLRLSCAASEHTFSNHVMGWFRQAPGKERESVAVIGWRDISTSYADSVKGRFTISRDNAKKTLYLQMNSLKPEDTAVYYCAARRIDAADFDSRGQGTQVTVSSTSTTTPAPRPPTPAPTIASQPLSLRPEACRPAAGGAVHTRGLDFACDIYIWAPLAGTCGVLLLSLVITLYCKRGRKKLLYIFKQPFMRPVQTTQEEDGCSCRFPEEEEGGCELRVKFSRSADAPAYQQGQNQLYNELNLGRREEYDVLDKRRGRDPEMGGKPRRKNPQEGLYNELQKDKMAEAYSEIGMKGERRRGKGHDGLYQGLSTATKDTYDALHMQALPPR

SEQ ID NO: 253 - protein, 369 aa, synthetic construct
MALPVTALLLPLALLLHAARPAVQLVDSGGGLVQAGGSLRISCAVSGRTSSNYILAWFRQAPGKERDFVAHISRSGGKSGYGDSVKGRFTISRDNAENTVRVYLQMNSLKPGDTAVYYCNRPLWYGSPTLIDYWGQGTQVTVSSTSTTTPAPRPPTPAPTIASQPLSLRPEACRPAAGGAVHTRGLDFACDIYIWAPLAGTCGVLLLSLVITLYCKRGRKKLLYIFKQPFMRPVQTTQEEDGCSCRFPEEEEGGCELRVKFSRSADAPAYQQGQNQLYNELNLGRREEYDVLDKRRGRDPEMGGKPRRKNPQEGLYNELQKDKMAEAYSEIGMKGERRRGKGHDGLYQGLSTATKDTYDALHMQALPPR

SEQ ID NO: 254 - protein, 364 aa, synthetic construct
MALPVTALLLPLALLLHAARPQVQLVESGGGLVQAGGSLRLSCAASGRTFTMGWFRQAPGKEREFVAAISLSPTLAYYAESVKGRFTISRDNAKNTVVLQMNSLKPEDTALYYCAADRKSVMSIRPDYWGQGTQVTVSSTSTTTPAPRPPTPAPTIASQPLSLRPEACRPAAGGAVHTRGLDFACDIYIWAPLAGTCGVLLLSLVITLYCKRGRKKLLYIFKQPFMRPVQTTQEEDGCSCRFPEEEEGGCELRVKFSRSADAPAYQQGQNQLYNELNLGRREEYDVLDKRRGRDPEMGGKPRRKNPQEGLYNELQKDKMAEAYSEIGMKGERRRGKGHDGLYQGLSTATKDTYDALHMQALPPR

SEQ ID NO: 255 - protein, 364 aa, synthetic construct
MALPVTALLLPLALLLHAARPAVQLVDSGGGLVQAGGSLRLSCAASGRTFTMGWFRQAPGKEREFVAAISLSPTLAYYAEPVKGRFTISRDNAKNTVVLQMNSLKPEDTALYYCAADRKSVMSIRPDYWGQGTQVTVSSTSTTTPAPRPPTPAPTIASQPLSLRPEACRPAAGGAVHTRGLDFACDIYIWAPLAGTCGVLLLSLVITLYCKRGRKKLLYIFKQPFMRPVQTTQEEDGCSCRFPEEEEGGCELRVKFSRSADAPAYQQGQNQLYNELNLGRREEYDVLDKRRGRDPEMGGKPRRKNPQEGLYNELQKDKMAEAYSEIGMKGERRRGKGHDGLYQGLSTATKDTYDALHMQALPPR

SEQ ID NO: 256 - protein, 367 aa, synthetic construct
MALPVTALLLPLALLLHAARPDVQLVESGGGSVQTGGSLRLSCTASGRTLNNFVMGWFRQAPGKEREFVAAISLSPTLAYYVESVKGRFTISRDNAKNTVVLQMNSLKPEDTALYYCAADRKSVMSIRPDYWGQGTQVTVSSTSTTTPAPRPPTPAPTIASQPLSLRPEACRPAAGGAVHTRGLDFACDIYIWAPLAGTCGVLLLSLVITLYCKRGRKKLLYIFKQPFMRPVQTTQEEDGCSCRFPEEEEGGCELRVKFSRSADAPAYQQGQNQLYNELNLGRREEYDVLDKRRGRDPEMGGKPRRKNPQEGLYNELQKDKMAEAYSEIGMKGERRRGKGHDGLYQGLSTATKDTYDALHMQALPPR

SEQ ID NO: 257 - DNA, 1263 bp, synthetic construct
  source 1..1263: mol_type = other DNA
atggccttaccagtgaccgccttgctcctgccgctggccttgctgctccacgccgccaggccggttaaccgcacgcgtcgcatgcatcaggtgcagctggtggagtctgggggaggcttggtgcagcctgggggttctctgaggctctcctgtgaagcctctggattcactttggattattatgccataggctggttccgccaggccccagggaaggagcgcgagggggtcatatgtattagtagaagtgatggtagcacatactatgcagactccgtgaagggccgattcaccatctccagagacaacgccaagaaaacggtgtatctgcaaatgatcagcctgaaacctgaggacacggccgcttattactgtgcagcaggggccgattgttcggggtacctacgagattatgagttccgggggcaggggacccaggtcaccgtctcctcaactagtaccacgacgccagcgccgcgaccaccaacaccggcgcccaccatcgcgtcgcagcccctgtccctgcgcccagaggcgtgccggccagcggcggggggcgcagtgcacacgagggggctggacttcgcctgtgatttttgggtgctggtggtggttggtggagtcctggcttgctatagcttgctagtaacagtggcctttattattttctgggtgaggagtaagaggagcaggctcctgcacagtgactacatgaacatgactccccgccgccccgggcccacccgcaagcattaccagccctatgccccaccacgcgacttcgcagcctatcgctccaaacggggcagaaagaaactcctgtatatattcaaacaaccatttatgagaccagtacaaactactcaagaggaagatggctgtagctgccgatttccagaagaagaagaaggaggatgtgaactgagagtgaagttcagcaggagcgcagacgcccccgcgtacaagcagggccagaaccagctctataacgagctcaatctaggacgaagagaggagtacgatgttttggacaagagacgtggccgggaccctgagatggggggaaagccgagaaggaagaaccctcaggaaggcctgtacaatgaactgcagaaagataagatggcggaggcctacagtgagattgggatgaaaggcgagcgccggaggggcaaggggcacgatggcctttaccagggtctcagtacagccaccaaggacacctacgacgcccttcacatgcaggccctgccccctcgctga

SEQ ID NO: 258 - DNA, 1281 bp, synthetic construct
  source 1..1281: mol_type = other DNA
atggccttaccagtgaccgccttgctcctgccgctggccttgctgctccacgccgccaggccggttaaccgcacgcgtcgcatgcatcaggtaaagctggaggagtctgggggacgattggtgcagccaaggggctctctgagactctcctgtgcaggctctggacgcactttcagtacctatggtatggcctggttccgccaggctccagggaaggagcgtgagttcgtagcgtctaaagcatcgatgaattacagcggtagaacatactatgcagactccgtgaagggccgattcaccatcgccagagacaacgccaagaacatggtgtttctgcaaatgaacaacctgaagcctgaggacacggccgtttattactgtgcagcgggcactggatgctcaacatatgggtgttttgacgcccagataatagactactggggcaaagggaccctggtcaccgtctcctcaactagtaccacgacgccagcgccgcgaccaccaacaccggcgcccaccatcgcgtcgcagcccctgtccctgcgcccagaggcgtgccggccagcggcggggggcgcagtgcacacgagggggctggacttcgcctgtgatttttgggtgctggtggtggttggtggagtcctggcttgctatagcttgctagtaacagtggcctttattattttctgggtgaggagtaagaggagcaggctcctgcacagtgactacatgaacatgactccccgccgccccgggcccacccgcaagcattaccagccctatgccccaccacgcgacttcgcagcctatcgctccaaacggggcagaaagaaactcctgtatatattcaaacaaccatttatgagaccagtacaaactactcaagaggaagatggctgtagctgccgatttccagaagaagaagaaggaggatgtgaactgagagtgaagttcagcaggagcgcagacgcccccgcgtacaagcagggccagaaccagctctataacgagctcaatctaggacgaagagaggagtacgatgttttggacaagagacgtggccgggaccctgagatggggggaaagccgagaaggaagaaccctcaggaaggcctgtacaatgaactgcagaaagataagatggcggaggcctacagtgagattgggatgaaaggcgagcgccggaggggcaaggggcacgatggcctttaccagggtctcagtacagccaccaaggacacctacgacgcccttcacatgcaggccctgccccctcgctga

SEQ ID NO: 259 - DNA, 1251 bp, synthetic construct
  source 1..1251: mol_type = other DNA
atggccttaccagtgaccgccttgctcctgccgctggccttgctgctccacgccgccaggccggttaaccgcacgcgtcgcatgcatgaggtgcagctggtggagtctgggggaggcttggtgcaggctggggggtctctgagactctcctgtgcagcctctggacgcaccttcaccatggggtggttccgtcaggctccagggaaggagcgtgagtttgtagcagctattagtttgagtcctactttagcatattatgcagagtccgtgaagggccgattcaccatcagccgagacaacgccaagaacacggtggttttgcaaatgaacagcctgaaacctgaggacacggccctttattactgtgcagcagaccggaaatcagtaatgtctattcggcccgactactggggccaggggacccaggtcaccgtctcctcaactagtaccacgacgccagcgccgcgaccaccaacaccggcgcccaccatcgcgtcgcagcccctgtccctgcgcccagaggcgtgccggccagcggcggggggcgcagtgcacacgagggggctggacttcgcctgtgatttttgggtgctggtggtggttggtggagtcctggcttgctatagcttgctagtaacagtggcctttattattttctgggtgaggagtaagaggagcaggctcctgcacagtgactacatgaacatgactccccgccgccccgggcccacccgcaagcattaccagccctatgccccaccacgcgacttcgcagcctatcgctccaaacggggcagaaagaaactcctgtatatattcaaacaaccatttatgagaccagtacaaactactcaagaggaagatggctgtagctgccgatttccagaagaagaagaaggaggatgtgaactgagagtgaagttcagcaggagcgcagacgcccccgcgtacaagcagggccagaaccagctctataacgagctcaatctaggacgaagagaggagtacgatgttttggacaagagacgtggccgggaccctgagatggggggaaagccgagaaggaagaaccctcaggaaggcctgtacaatgaactgcagaaagataagatggcggaggcctacagtgagattgggatgaaaggcgagcgccggaggggcaaggggcacgatggcctttaccagggtctcagtacagccaccaaggacacctacgacgcccttcacatgcaggccctgccccctcgctga

SEQ ID NO: 260 - DNA, 1257 bp, synthetic construct
  source 1..1257: mol_type = other DNA
atggccttaccagtgaccgccttgctcctgccgctggccttgctgctccacgccgccaggccggttaaccgcacgcgtcgcatgcatgccgtgcagctggtggattctgggggaggcttggtgcagcctggggggtctctgagactctcctgtgtagcctctggaggtatcttcgtcatcaatgccatgggctggtaccgccaggctccaggaaagcagcgcgagttggtcgcatctattcgtggactaggcagaacaaactatgacgactccgtgaagggccgattcaccatctccagagacaacgccaacaacacggtgtatctgcagatgaacagcctggaacctgaggacacggccgtctactactgtacagtctacgttacactacttggtggggttaatagggactactggggccaggggacccaggtcaccgtctcctcaactagtaccacgacgccagcgccgcgaccaccaacaccggcgcccaccatcgcgtcgcagcccctgtccctgcgcccagaggcgtgccggccagcggcggggggcgcagtgcacacgagggggctggacttcgcctgtgatttttgggtgctggtggtggttggtggagtcctggcttgctatagcttgctagtaacagtggcctttattattttctgggtgaggagtaagaggagcaggctcctgcacagtgactacatgaacatgactccccgccgccccgggcccacccgcaagcattaccagccctatgccccaccacgcgacttcgcagcctatcgctccaaacggggcagaaagaaactcctgtatatattcaaacaaccatttatgagaccagtacaaactactcaagaggaagatggctgtagctgccgatttccagaagaagaagaaggaggatgtgaactgagagtgaagttcagcaggagcgcagacgcccccgcgtacaagcagggccagaaccagctctataacgagctcaatctaggacgaagagaggagtacgatgttttggacaagagacgtggccgggaccctgagatggggggaaagccgagaaggaagaaccctcaggaaggcctgtacaatgaactgcagaaagataagatggcggaggcctacagtgagattgggatgaaaggcgagcgccggaggggcaaggggcacgatggcctttaccagggtctcagtacagccaccaaggacacctacgacgcccttcacatgcaggccctgccccctcgctga

SEQ ID NO: 261 - DNA, 1254 bp, synthetic construct
  source 1..1254: mol_type = other DNA
atggccttaccagtgaccgccttgctcctgccgctggccttgctgctccacgccgccaggccggttaaccgcacgcgtcgcatgcatgaggtgcagctggtggagtctgggggaggattggtgcaggctgggggctctctgagactctcctgtgcagcctctggacggaccttcagtagcattgtcatgggctggttccgccaggctccagggaaggagcgtgagtttgtaggagcgattatgtggaatgatggtattacatacttgcaagactccgtgaagggccgatttaccatcttcagagacaatgccaagaacacggtgtatctgcaaatgaacagcctgaaacttgaggatacggccgtttattactgtgcagcatccaagggtagatactcggaatatgagtactggggccaggggacccaggtcaccgtctcctcaactagtaccacgacgccagcgccgcgaccaccaacaccggcgcccaccatcgcgtcgcagcccctgtccctgcgcccagaggcgtgccggccagcggcggggggcgcagtgcacacgagggggctggacttcgcctgtgatttttgggtgctggtggtggttggtggagtcctggcttgctatagcttgctagtaacagtggcctttattattttctgggtgaggagtaagaggagcaggctcctgcacagtgactacatgaacatgactccccgccgccccgggcccacccgcaagcattaccagccctatgccccaccacgcgacttcgcagcctatcgctccaaacggggcagaaagaaactcctgtatatattcaaacaaccatttatgagaccagtacaaactactcaagaggaagatggctgtagctgccgatttccagaagaagaagaaggaggatgtgaactgagagtgaagttcagcaggagcgcagacgcccccgcgtacaagcagggccagaaccagctctataacgagctcaatctaggacgaagagaggagtacgatgttttggacaagagacgtggccgggaccctgagatggggggaaagccgagaaggaagaaccctcaggaaggcctgtacaatgaactgcagaaagataagatggcggaggcctacagtgagattgggatgaaaggcgagcgccggaggggcaaggggcacgatggcctttaccagggtctcagtacagccaccaaggacacctacgacgcccttcacatgcaggccctgccccctcgctga

SEQ ID NO: 262 - DNA, 1281 bp, synthetic construct
  source 1..1281: mol_type = other DNA
atggccttaccagtgaccgccttgctcctgccgctggccttgctgctccacgccgccaggccggttaaccgcacgcgtcgcatgcatgaggtgcagctggtggagtctgggggaggcgtggtgcaggctggggggtctctgacagtctcctgtacagcctctggattcactttcgaccgtgctgtcatagtctggttccgccaggcccccgggaagggccgtgagggggtctcatttattaaacctagtgatggcaccatatactacattgactccctgaagggccgattcacgatctccagtgacatcgccaagaatacggtatatctgcaaatgaaaagtctggaatcggaggactcggccgtttattactgtgcggcctcgcctgaggactggtacacggattggatcgactggagtatatatcggtggcagcactggggccaggggacccaggtcactgtctcctcaactagtaccacgacgccagcgccgcgaccaccaacaccggcgcccaccatcgcgtcgcagcccctgtccctgcgcccagaggcgtgccggccagcggcggggggcgcagtgcacacgagggggctggacttcgcctgtgatttttgggtgctggtggtggttggtggagtcctggcttgctatagcttgctagtaacagtggcctttattattttctgggtgaggagtaagaggagcaggctcctgcacagtgactacatgaacatgactccccgccgccccgggcccacccgcaagcattaccagccctatgccccaccacgcgacttcgcagcctatcgctccaaacggggcagaaagaaactcctgtatatattcaaacaaccatttatgagaccagtacaaactactcaagaggaagatggctgtagctgccgatttccagaagaagaagaaggaggatgtgaactgagagtgaagttcagcaggagcgcagacgcccccgcgtacaagcagggccagaaccagctctataacgagctcaatctaggacgaagagaggagtacgatgttttggacaagagacgtggccgggaccctgagatggggggaaagccgagaaggaagaaccctcaggaaggcctgtacaatgaactgcagaaagataagatggcggaggcctacagtgagattgggatgaaaggcgagcgccggaggggcaaggggcacgatggcctttaccagggtctcagtacagccaccaaggacacctacgacgcccttcacatgcaggccctgccccctcgctga

SEQ ID NO: 263 - DNA, 1254 bp, synthetic construct
  source 1..1254: mol_type = other DNA
atggccttaccagtgaccgccttgctcctgccgctggccttgctgctccacgccgccaggccggttaaccgcacgcgtcgcatgcatgaggtgcagctggtggagtctgggggaggaatggtgcaggctggggactctctgagactatcctgtgtgcagtctacttacaccgtcaatagcgatgtcatgggctggttccgccaggctccagggaaggagcgtgagtttgtaggagcgattatgtggaatgatggtattacatacttgcaagactccgtgaagggccgatttaccatcttcagagacaacgccaagaacacggtgtatctgcaaatgaacagcctgaaacttgaggatacggccgtttattactgtgcagcatccaagggtagatactcggaatatgagtactggggccaggggacccaggtcaccgtctcctcaactagtaccacgacgccagcgccgcgaccaccaacaccggcgcccaccatcgcgtcgcagcccctgtccctgcgcccagaggcgtgccggccagcggcggggggcgcagtgcacacgagggggctggacttcgcctgtgatttttgggtgctggtggtggttggtggagtcctggcttgctatagcttgctagtaacagtggcctttattattttctgggtgaggagtaagaggagcaggctcctgcacagtgactacatgaacatgactccccgccgccccgggcccacccgcaagcattaccagccctatgccccaccacgcgacttcgcagcctatcgctccaaacggggcagaaagaaactcctgtatatattcaaacaaccatttatgagaccagtacaaactactcaagaggaagatggctgtagctgccgatttccagaagaagaagaaggaggatgtgaactgagagtgaagttcagcaggagcgcagacgcccccgcgtacaagcagggccagaaccagctctataacgagctcaatctaggacgaagagaggagtacgatgttttggacaagagacgtggccgggaccctgagatggggggaaagccgagaaggaagaaccctcaggaaggcctgtacaatgaactgcagaaagataagatggcggaggcctacagtgagattgggatgaaaggcgagcgccggaggggcaaggggcacgatggcctttaccagggtctcagtacagccaccaaggacacctacgacgcccttcacatgcaggccctgccccctcgctga

SEQ ID NO: 264 - DNA, 1257 bp, synthetic construct
  source 1..1257: mol_type = other DNA
atggccttaccagtgaccgccttgctcctgccgctggccttgctgctccacgccgccaggccggttaaccgcacgcgtcgcatgcatgcggtgcagctggtggagtctgggggaggattggtgcaggctggggactctctgagactctcctgtacagcctctggtgcaaccttgactaacgatcacatggcatggttccgccaggctccagggaaggggcgtgaatttgtagcagctattgactggagtggtcgtaccacaaattacgcagaccccgtagagggccgattcaccatctccagaaacaacgccaagaacacggtgtatctggaaatgaacagcctgaaacttgaggacacggccgtttattactgtgcggtcctccgcgcttggatctcatatgacaatgactactggggccaggggacccaggtcaccgtctcctcaactagtaccacgacgccagcgccgcgaccaccaacaccggcgcccaccatcgcgtcgcagcccctgtccctgcgcccagaggcgtgccggccagcggcggggggcgcagtgcacacgagggggctggacttcgcctgtgatttttgggtgctggtggtggttggtggagtcctggcttgctatagcttgctagtaacagtggcctttattattttctgggtgaggagtaagaggagcaggctcctgcacagtgactacatgaacatgactccccgccgccccgggcccacccgcaagcattaccagccctatgccccaccacgcgacttcgcagcctatcgctccaaacggggcagaaagaaactcctgtatatattcaaacaaccatttatgagaccagtacaaactactcaagaggaagatggctgtagctgccgatttccagaagaagaagaaggaggatgtgaactgagagtgaagttcagcaggagcgcagacgcccccgcgtacaagcagggccagaaccagctctataacgagctcaatctaggacgaagagaggagtacgatgttttggacaagagacgtggccgggaccctgagatggggggaaagccgagaaggaagaaccctcaggaaggcctgtacaatgaactgcagaaagataagatggcggaggcctacagtgagattgggatgaaaggcgagcgccggaggggcaaggggcacgatggcctttaccagggtctcagtacagccaccaaggacacctacgacgcccttcacatgcaggccctgccccctcgctga

SEQ ID NO: 265 - DNA, 1257 bp, synthetic construct
  source 1..1257: mol_type = other DNA
atggccttaccagtgaccgccttgctcctgccgctggccttgctgctccacgccgccaggccggttaaccgcacgcgtcgcatgcatcaggtgcagctggtggagtctgggggaggattggtgcaggctgggggctctctgagactctcctgtgcagcctctggaggcaccttaagtaaaaataccgtggcttggttccgccaggctccagggaaggagcgtgggtttgtagcgtctattacctgggatggtcgtacgacatactatgcagactccgtgaagggccgattcaccatctccagagacaacgccaagaacacagtgtatctgcaaatgaacagcctgaaacctgaggatacggccgtttatgtctgtgcagacttagggaaatggcctgcgggcccggcggactactggggccaggggacccaggtcaccgtctcctcaactagtaccacgacgccagcgccgcgaccaccaacaccggcgcccaccatcgcgtcgcagcccctgtccctgcgcccagaggcgtgccggccagcggcggggggcgcagtgcacacgagggggctggacttcgcctgtgatttttgggtgctggtggtggttggtggagtcctggcttgctatagcttgctagtaacagtggcctttattattttctgggtgaggagtaagaggagcaggctcctgcacagtgactacatgaacatgactccccgccgccccgggcccacccgcaagcattaccagccctatgccccaccacgcgacttcgcagcctatcgctccaaacggggcagaaagaaactcctgtatatattcaaacaaccatttatgagaccagtacaaactactcaagaggaagatggctgtagctgccgatttccagaagaagaagaaggaggatgtgaactgagagtgaagttcagcaggagcgcagacgcccccgcgtacaagcagggccagaaccagctctataacgagctcaatctaggacgaagagaggagtacgatgttttggacaagagacgtggccgggaccctgagatggggggaaagccgagaaggaagaaccctcaggaaggcctgtacaatgaactgcagaaagataagatggcggaggcctacagtgagattgggatgaaaggcgagcgccggaggggcaaggggcacgatggcctttaccagggtctcagtacagccaccaaggacacctacgacgcccttcacatgcaggccctgccccctcgctga

SEQ ID NO: 266 - DNA, 1254 bp, synthetic construct
  source 1..1254: mol_type = other DNA
atggccttaccagtgaccgccttgctcctgccgctggccttgctgctccacgccgccaggccggttaaccgcacgcgtcgcatgcatcaggtaaagctggaggagtctgggggaggcttggtgcaggctgggcggtctctgagactctcctgtgcagcctctgaacacaccttcagtagccatgtcatgggctggttccgccaggctccagggaaggagcgtgagtctgttgcagttattggctggagagatattagcacaagctatgcagactccgtgaagggccgattcaccatctccagagacaacgccaagaagacgctgtatctgcaaatgaatagcctgaaacctgaggacacggccgtttactactgtgcagcacgtcggatcgacgcagctgactttgattcctgggggcaggggacccaggtcaccgtctcctcgactagtaccacgacgccagcgccgcgaccaccaacaccggcgcccaccatcgcgtcgcagcccctgtccctgcgcccagaggcgtgccggccagcggcggggggcgcagtgcacacgagggggctggacttcgcctgtgatttttgggtgctggtggtggttggtggagtcctggcttgctatagcttgctagtaacagtggcctttattattttctgggtgaggagtaagaggagcaggctcctgcacagtgactacatgaacatgactccccgccgccccgggcccacccgcaagcattaccagccctatgccccaccacgcgacttcgcagcctatcgctccaaacggggcagaaagaaactcctgtatatattcaaacaaccatttatgagaccagtacaaactactcaagaggaagatggctgtagctgccgatttccagaagaagaagaaggaggatgtgaactgagagtgaagttcagcaggagcgcagacgcccccgcgtacaagcagggccagaaccagctctataacgagctcaatctaggacgaagagaggagtacgatgttttggacaagagacgtggccgggaccctgagatggggggaaagccgagaaggaagaaccctcaggaaggcctgtacaatgaactgcagaaagataagatggcggaggcctacagtgagattgggatgaaaggcgagcgccggaggggcaaggggcacgatggcctttaccagggtctcagtacagccaccaaggacacctacgacgcccttcacatgcaggccctgccccctcgctga

SEQ ID NO: 267 - DNA, 1254 bp, synthetic construct
  source 1..1254: mol_type = other DNA
atggccttaccagtgaccgccttgctcctgccgctggccttgctgctccacgccgccaggccggttaaccgcacgcgtcgcatgcatgcggtgcagctggtggagtctgggggaggattggtgcaggctggggactctctgagactcacctgtacagcctctggacgcgccttcagtacctatttcatggcctggttccgccaggctccagggaaggagcgtgagtttgtagcaggaattgcatggagtggtggtagcacggcgtatgcagactccgtgaagggccgattcaccatctccagagacaacgccaagaacacggtgtatctgcaaatgaacagcctgaaatctgaggacacggccgtttattactgtgccagcagggggattgaggtcgaagagtttggtgcctggggccaggggacccaggtcaccgtctcgtcgactagtaccacgacgccagcgccgcgaccaccaacaccggcgcccaccatcgcgtcgcagcccctgtccctgcgcccagaggcgtgccggccagcggcggggggcgcagtgcacacgagggggctggacttcgcctgtgatttttgggtgctggtggtggttggtggagtcctggcttgctatagcttgctagtaacagtggcctttattattttctgggtgaggagtaagaggagcaggctcctgcacagtgactacatgaacatgactccccgccgccccgggcccacccgcaagcattaccagccctatgccccaccacgcgacttcgcagcctatcgctccaaacggggcagaaagaaactcctgtatatattcaaacaaccatttatgagaccagtacaaactactcaagaggaagatggctgtagctgccgatttccagaagaagaagaaggaggatgtgaactgagagtgaagttcagcaggagcgcagacgcccccgcgtacaagcagggccagaaccagctctataacgagctcaatctaggacgaagagaggagtacgatgttttggacaagagacgtggccgggaccctgagatggggggaaagccgagaaggaagaaccctcaggaaggcctgtacaatgaactgcagaaagataagatggcggaggcctacagtgagattgggatgaaaggcgagcgccggaggggcaaggggcacgatggcctttaccagggtctcagtacagccaccaaggacacctacgacgcccttcacatgcaggccctgccccctcgctga

SEQ ID NO: 268 - DNA, 1131 bp, synthetic construct
  source 1..1131: mol_type = other DNA
atggccttaccagtgaccgccttgctcctgccgctggccttgctgctccacgccgccaggccggttaaccgcacgcgtcgcatgcatcaggtgcagctggtggagtctgggggaggcttggtgcagcctgggggttctctgaggctctcctgtgaagcctctggattcactttggattattatgccataggctggttccgccaggccccagggaaggagcgcgagggggtcatatgtattagtagaagtgatggtagcacatactatgcagactccgtgaagggccgattcaccatctccagagacaacgccaagaaaacggtgtatctgcaaatgatcagcctgaaacctgaggacacggccgcttattactgtgcagcaggggccgattgttcggggtacctacgagattatgagttccgggggcaggggacccaggtcaccgtctcctcaactagtaccacgacgccagcgccgcgaccaccaacaccggcgcccaccatcgcgtcgcagcccctgtccctgcgcccagaggcgtgccggccagcggcggggggcgcagtgcacacgagggggctggacttcgcctgtgatatctacatctgggcgcccttggccgggacttgtggggtccttctcctgtcactggttatcaccctttactgcaaacggggcagaaagaaactcctgtatatattcaaacaaccatttatgagaccagtacaaactactcaagaggaagatggctgtagctgccgatttccagaagaagaagaaggaggatgtgaactgagagtgaagttcagcaggagcgcagacgcccccgcgtaccagcagggccagaaccagctctataacgagctcaatctaggacgaagagaggagtacgatgttttggacaagagacgtggccgggaccctgagatggggggaaagccgagaaggaagaaccctcaggaaggcctgtacaatgaactgcagaaagataagatggcggaggcctacagtgagattgggatgaaaggcgagcgccggaggggcaaggggcacgatggcctttaccagggtctcagtacagccaccaaggacacctacgacgcccttcacatgcaggccctgccccctcgctaa

SEQ ID NO: 269 - DNA, 1122 bp, synthetic construct
  source 1..1122: mol_type = other DNA
atggccttaccagtgaccgccttgctcctgccgctggccttgctgctccacgccgccaggccggttaaccgcacgcgtcgcatgcatcaggtaaagctggaggagtctgggggaggcttggtgcaggctgggcggtctctgagactctcctgtgcagcctctgaacacaccttcagtagccatgtcatgggctggttccgccaggctccagggaaggagcgtgagtctgttgcagttattggctggagagatattagcacaagctatgcagactccgtgaagggccgattcaccatctccagagacaacgccaagaagacgctgtatctgcaaatgaatagcctgaaacctgaggacacggccgtttactactgtgcagcacgtcggatcgacgcagctgactttgattcctgggggcaggggacccaggtcaccgtctcctcgactagtaccacgacgccagcgccgcgaccaccaacaccggcgcccaccatcgcgtcgcagcccctgtccctgcgcccagaggcgtgccggccagcggcggggggcgcagtgcacacgagggggctggacttcgcctgtgatatctacatctgggcgcccttggccgggacttgtggggtccttctcctgtcactggttatcaccctttactgcaaacggggcagaaagaaactcctgtatatattcaaacaaccatttatgagaccagtacaaactactcaagaggaagatggctgtagctgccgatttccagaagaagaagaaggaggatgtgaactgagagtgaagttcagcaggagcgcagacgcccccgcgtaccagcagggccagaaccagctctataacgagctcaatctaggacgaagagaggagtacgatgttttggacaagagacgtggccgggaccctgagatggggggaaagccgagaaggaagaaccctcaggaaggcctgtacaatgaactgcagaaagataagatggcggaggcctacagtgagattgggatgaaaggcgagcgccggaggggcaaggggcacgatggcctttaccagggtctcagtacagccaccaaggacacctacgacgcccttcacatgcaggccctgccccctcgctaa

SEQ ID NO: 270 - DNA, 1119 bp, synthetic construct
  source 1..1119: mol_type = other DNA
atggccttaccagtgaccgccttgctcctgccgctggccttgctgctccacgccgccaggccggttaaccgcacgcgtcgcatgcatgaggtgcagctggtggagtctgggggaggcttggtgcaggctggggggtctctgagactctcctgtgcagcctctggacgcaccttcaccatggggtggttccgtcaggctccagggaaggagcgtgagtttgtagcagctattagtttgagtcctactttagcatattatgcagagtccgtgaagggccgattcaccatcagccgagacaacgccaagaacacggtggttttgcaaatgaacagcctgaaacctgaggacacggccctttattactgtgcagcagaccggaaatcagtaatgtctattcggcccgactactggggccaggggacccaggtcaccgtctcctcaactagtaccacgacgccagcgccgcgaccaccaacaccggcgcccaccatcgcgtcgcagcccctgtccctgcgcccagaggcgtgccggccagcggcggggggcgcagtgcacacgagggggctggacttcgcctgtgatatctacatctgggcgcccttggccgggacttgtggggtccttctcctgtcactggttatcaccctttactgcaaacggggcagaaagaaactcctgtatatattcaaacaaccatttatgagaccagtacaaactactcaagaggaagatggctgtagctgccgatttccagaagaagaagaaggaggatgtgaactgagagtgaagttcagcaggagcgcagacgcccccgcgtaccagcagggccagaaccagctctataacgagctcaatctaggacgaagagaggagtacgatgttttggacaagagacgtggccgggaccctgagatggggggaaagccgagaaggaagaaccctcaggaaggcctgtacaatgaactgcagaaagataagatggcggaggcctacagtgagattgggatgaaaggcgagcgccggaggggcaaggggcacgatggcctttaccagggtctcagtacagccaccaaggacacctacgacgcccttcacatgcaggccctgccccctcgctaa

SEQ ID NO: 271 - DNA, 1113 bp, synthetic construct
  source 1..1113: mol_type = other DNA
atggctctgcccgtcaccgctctgctgctgcctctggctctgctgctgcacgctgctcgccctgaggtgcagctggtggagtctgggggaggcttggtgccgcctggggggtctctgagactctcctgtacagcctctggaagcacagtcagcatcaatgtcatggcctggtaccgccaggtttcagggaagcagcgcgagttggtcgcggccgttactagggatggtaggaaaagttgtggagactccgtgaagggccgattcaccatttccagagacggcgccaagaatgcggtatatttgcaaatgaacagtctgaaacctgaggacacagcggtctatttatgtggagccgatggttggggtgctactaccttagattatacctacggcatggactattggggcaaagggacccaggtcaccgtctcctcaactagtaccacgacgccagcgccgcgaccaccaacaccggcgcccaccatcgcgtcgcagcccctgtccctgcgcccagaggcgtgccggccagcggcggggggcgcagtgcacacgagggggctggacttcgcctgtgatatctacatctgggcgcccttggccgggacttgtggggtccttctcctgtcactggttatcaccctttactgcaaacggggcagaaagaaactcctgtatatattcaaacaaccatttatgagaccagtacaaactactcaagaggaagatggctgtagctgccgatttccagaagaagaagaaggaggatgtgaactgagagtgaagttcagcaggagcgcagacgcccccgcgtaccagcagggccagaaccagctctataacgagctcaatctaggacgaagagaggagtacgatgttttggacaagagacgtggccgggaccctgagatggggggaaagccgagaaggaagaaccctcaggaaggcctgtacaatgaactgcagaaagataagatggcggaggcctacagtgagattgggatgaaaggcgagcgccggaggggcaaggggcacgatggcctttaccagggtctcagtacagccaccaaggacacctacgacgcccttcacatgcaggccctgccccctcgctaa

SEQ ID NO: 272 - DNA, 1095 bp, synthetic construct
  source 1..1095: mol_type = other DNA
atggctctgcccgtcaccgctctgctgctgcctctggctctgctgctgcacgctgctcgccctgcggtgcagctggtggagtctgggggaggattggtgcaggctgggggctctctgagactctcctgtgcagcctctggacgcaccttcaccatggggtggttccgtcaggctccagggaaggagcgtgggtttgtagcgtctattacctgggatggtcgttcggcatactatgcagagtccgtgaagggccgattcaccatcagccgagacaacgccaagaacacggtggttttgcaaatgaacagcctgaaacctgaggacacggccctttattactgtgcagcagaccggaaatcagtaatgtctattcggcccgactactggggccaggggacccaggtcaccgtctcctcaactagtaccacgacgccagcgccgcgaccaccaacaccggcgcccaccatcgcgtcgcagcccctgtccctgcgcccagaggcgtgccggccagcggcggggggcgcagtgcacacgagggggctggacttcgcctgtgatatctacatctgggcgcccttggccgggacttgtggggtccttctcctgtcactggttatcaccctttactgcaaacggggcagaaagaaactcctgtatatattcaaacaaccatttatgagaccagtacaaactactcaagaggaagatggctgtagctgccgatttccagaagaagaagaaggaggatgtgaactgagagtgaagttcagcaggagcgcagacgcccccgcgtaccagcagggccagaaccagctctataacgagctcaatctaggacgaagagaggagtacgatgttttggacaagagacgtggccgggaccctgagatggggggaaagccgagaaggaagaaccctcaggaaggcctgtacaatgaactgcagaaagataagatggcggaggcctacagtgagattgggatgaaaggcgagcgccggaggggcaaggggcacgatggcctttaccagggtctcagtacagccaccaaggacacctacgacgcccttcacatgcaggccctgccccctcgctaa

SEQ ID NO: 273 - DNA, 1107 bp, synthetic construct
  source 1..1107: mol_type = other DNA
atggctctgcccgtcaccgctctgctgctgcctctggctctgctgctgcacgctgctcgccctcaggtacagctggtggagtctgggggaggattggtgcagcctggggggtctctaagactcgcatgtgaagcgcctggaagcggcaatagtatcaatgccatgggctggtaccggcagactccggggaagcggcgcgagttggtcgcaactattactcggggtggtagcacgaactatggaccctccgtgaagggccgattcacgatcaccagagacaatgtcaagaatacggtgcatctgcagatgaacagcctgaaacctgacgacacggccgtctattattgcaatgcggagaggctggacggctcggggtacggatatgagtatgattactggggccaggggacccaggtcaccgtctcctcaactagtaccacgacgccagcgccgcgaccaccaacaccggcgcccaccatcgcgtcgcagcccctgtccctgcgcccagaggcgtgccggccagcggcggggggcgcagtgcacacgagggggctggacttcgcctgtgatatctacatctgggcgcccttggccgggacttgtggggtccttctcctgtcactggttatcaccctttactgcaaacggggcagaaagaaactcctgtatatattcaaacaaccatttatgagaccagtacaaactactcaagaggaagatggctgtagctgccgatttccagaagaagaagaaggaggatgtgaactgagagtgaagttcagcaggagcgcagacgcccccgcgtaccagcagggccagaaccagctctataacgagctcaatctaggacgaagagaggagtacgatgttttggacaagagacgtggccgggaccctgagatggggggaaagccgagaaggaagaaccctcaggaaggcctgtacaatgaactgcagaaagataagatggcggaggcctacagtgagattgggatgaaaggcgagcgccggaggggcaaggggcacgatggcctttaccagggtctcagtacagccaccaaggacacctacgacgcccttcacatgcaggccctgccccctcgctaa

SEQ ID NO: 274 - DNA, 1104 bp, synthetic construct
  source 1..1104: mol_type = other DNA
atggctctgcccgtcaccgctctgctgctgcctctggctctgctgctgcacgctgctcgccctcaggtaaagctggaggagtctgggggaggattggtgcaggctgggggctctctgagactctcctgtgcagcctctggaggcaccttaagtaagaataccgtggcttgggtccgccaggctccagggaaggagcgtgggtttgtaacgtctattacctgtgatggtcgtacgacatactatgcgaactccgtaaacggccgattccccatcaaccgaaacaacgccgagaatttggtggttttgcaaatgaacagcctgaaacctgacgacacggccctttattactgtgcagcataccggaagtcaataatgtctattcagcccgactactggggccaggggacccaggtcaccgtctcctcaactagtaccacgacgccagcgccgcgaccaccaacaccggcgcccaccatcgcgtcgcagcccctgtccctgcgcccagaggcgtgccggccagcggcggggggcgcagtgcacacgagggggctggacttcgcctgtgatatctacatctgggcgcccttggccgggacttgtggggtccttctcctgtcactggttatcaccctttactgcaaacggggcagaaagaaactcctgtatatattcaaacaaccatttatgagaccagtacaaactactcaagaggaagatggctgtagctgccgatttccagaagaagaagaaggaggatgtgaactgagagtgaagttcagcaggagcgcagacgcccccgcgtaccagcagggccagaaccagctctataacgagctcaatctaggacgaagagaggagtacgatgttttggacaagagacgtggccgggaccctgagatggggggaaagccgagaaggaagaaccctcaggaaggcctgtacaatgaactgcagaaagataagatggcggaggcctacagtgagattgggatgaaaggcgagcgccggaggggcaaggggcacgatggcctttaccagggtctcagtacagccaccaaggacacctacgacgcccttcacatgcaggccctgccccctcgctaa

SEQ ID NO: 275 - DNA, 1104 bp, synthetic construct
  source 1..1104: mol_type = other DNA
atggctctgcccgtcaccgctctgctgctgcctctggctctgctgctgcacgctgctcgccctgatgtgcagctggtggagtctgggggaggattggtgcaggctgggggctctctgagactctcctgtgcagcctctggacggaccttcagtagcattgtcatgggctggttccgccaggctccagggaaggagcgtgagtttgtaggagcgattatgtggaatgatggtctgacatacttgcaagggtccgtgaagggccgattcaccatttccagagacaacgccaagaacacggtggttttgcaaatgaacagcctgaaacctgaggacacggccctttattactgtgcagcagaccggaaatcagtaatgtctattcggcccgactactggggccaggggacccaggtcaccgtctcctcaactagtaccacgacgccagcgccgcgaccaccaacaccggcgcccaccatcgcgtcgcagcccctgtccctgcgcccagaggcgtgccggccagcggcggggggcgcagtgcacacgagggggctggacttcgcctgtgatatctacatctgggcgcccttggccgggacttgtggggtccttctcctgtcactggttatcaccctttactgcaaacggggcagaaagaaactcctgtatatattcaaacaaccatttatgagaccagtacaaactactcaagaggaagatggctgtagctgccgatttccagaagaagaagaaggaggatgtgaactgagagtgaagttcagcaggagcgcagacgcccccgcgtaccagcagggccagaaccagctctataacgagctcaatctaggacgaagagaggagtacgatgttttggacaagagacgtggccgggaccctgagatggggggaaagccgagaaggaagaaccctcaggaaggcctgtacaatgaactgcagaaagataagatggcggaggcctacagtgagattgggatgaaaggcgagcgccggaggggcaaggggcacgatggcctttaccagggtctcagtacagccaccaaggacacctacgacgcccttcacatgcaggccctgccccctcgctaa

SEQ ID NO: 276 - DNA, 1089 bp, synthetic construct
  source 1..1089: mol_type = other DNA
atggctctgcccgtcaccgctctgctgctgcctctggctctgctgctgcacgctgctcgccctcaggtacagctggtggagtctgggggaggattggtgcaggctgggggctctctgagactctcctgtgcagcctctggacgcaccttcaccatggggtggttccgtcaggctccagggaaggagcgtgagtttgtagcagctattagtttgagtcctactttagcatattatgcagagtccgtgaagggccgattcaccatcagccgagacaacgccaagaacacggtggttttgcaaatgaacagcctgaaacctgaggacacggccgtttactactgtgcagcacgtcggatcgacgcagctgactttgattcctgggggcaggggacccaggtcaccgtctcctcaactagtaccacgacgccagcgccgcgaccaccaacaccggcgcccaccatcgcgtcgcagcccctgtccctgcgcccagaggcgtgccggccagcggcggggggcgcagtgcacacgagggggctggacttcgcctgtgatatctacatctgggcgcccttggccgggacttgtggggtccttctcctgtcactggttatcaccctttactgcaaacggggcagaaagaaactcctgtatatattcaaacaaccatttatgagaccagtacaaactactcaagaggaagatggctgtagctgccgatttccagaagaagaagaaggaggatgtgaactgagagtgaagttcagcaggagcgcagacgcccccgcgtaccagcagggccagaaccagctctataacgagctcaatctaggacgaagagaggagtacgatgttttggacaagagacgtggccgggaccctgagatggggggaaagccgagaaggaagaaccctcaggaaggcctgtacaatgaactgcagaaagataagatggcggaggcctacagtgagattgggatgaaaggcgagcgccggaggggcaaggggcacgatggcctttaccagggtctcagtacagccaccaaggacacctacgacgcccttcacatgcaggccctgccccctcgctaa

SEQ ID NO: 277 - DNA, 1101 bp, synthetic construct
  source 1..1101: mol_type = other DNA
atggctctgcccgtcaccgctctgctgctgcctctggctctgctgctgcacgctgctcgccctcaggtacagctggtggagtctgggggaggattggtgcaggctgggggctctctgagactctcctgtgcagcctctggaggcaccttaagtaaaaataccgtggcttggttccgccaggctccagggaaggagcgtgggtttgtagcgtctattacctgggatggtcgtacgacatactatgcagactccgtgaagggccgattcaccatctccagagacaacgccaagaacacagtgtatctgcaaatgaacagcctgaaacctgaggatacggccgtttatgtctgtgcagacttagggaaatggcctgcgggcccggcggactactggggccaggggacccaggtcaccgtctcctcaactagtaccacgacgccagcgccgcgaccaccaacaccggcgcccaccatcgcgtcgcagcccctgtccctgcgcccagaggcgtgccggccagcggcggggggcgcagtgcacacgagggggctggacttcgcctgtgatatctacatctgggcgcccttggccgggacttgtggggtccttctcctgtcactggttatcaccctttactgcaaacggggcagaaagaaactcctgtatatattcaaacaaccatttatgagaccagtacaaactactcaagaggaagatggctgtagctgccgatttccagaagaagaagaaggaggatgtgaactgagagtgaagttcagcaggagcgcagacgcccccgcgtaccagcagggccagaaccagctctataacgagctcaatctaggacgaagagaggagtacgatgttttggacaagagacgtggccgggaccctgagatggggggaaagccgagaaggaagaaccctcaggaaggcctgtacaatgaactgcagaaagataagatggcggaggcctacagtgagattgggatgaaaggcgagcgccggaggggcaaggggcacgatggcctttaccagggtctcagtacagccaccaaggacacctacgacgcccttcacatgcaggccctgccccctcgctaa

SEQ ID NO: 278 - DNA, 1104 bp, synthetic construct
  source 1..1104: mol_type = other DNA
atggctctgcccgtcaccgctctgctgctgcctctggctctgctgctgcacgctgctcgccctcaggtgcagctggtggagtctgggggaggcttggtgcagcctggggggtctctgacactctcctgtgcagcctctggaagcatcgacagtatcaataccatggactggttccgtcaggctccagggaaggagcgtgagtttgtagcagctattagtttgagtcccactttagcatattatgcagagtccgtgaagggccgattcaccatcagccgagacaacgccaagaacacggtggttttgcaaatgaacagcctgaaacctgaggacacggccctttattactgtgcagcagaccggaaatcagtaatgtctattcggcccgactactggggccaggggacccaggtcaccgtctcctcaactagtaccacgacgccagcgccgcgaccaccaacaccggcgcccaccatcgcgtcgcagcccctgtccctgcgcccagaggcgtgccggccagcggcggggggcgcagtgcacacgagggggctggacttcgcctgtgatatctacatctgggcgcccttggccgggacttgtggggtccttctcctgtcactggttatcaccctttactgcaaacggggcagaaagaaactcctgtatatattcaaacaaccatttatgagaccagtacaaactactcaagaggaagatggctgtagctgccgatttccagaagaagaagaaggaggatgtgaactgagagtgaagttcagcaggagcgcagacgcccccgcgtaccagcagggccagaaccagctctataacgagctcaatctaggacgaagagaggagtacgatgttttggacaagagacgtggccgggaccctgagatggggggaaagccgagaaggaagaaccctcaggaaggcctgtacaatgaactgcagaaagataagatggcggaggcctacagtgagattgggatgaaaggcgagcgccggaggggcaaggggcacgatggcctttaccagggtctcagtacagccaccaaggacacctacgacgcccttcacatgcaggccctgccccctcgctaa

SEQ ID NO: 279 - DNA, 1101 bp, synthetic construct
  source 1..1101: mol_type = other DNA
atggctctgcccgtcaccgctctgctgctgcctctggctctgctgctgcacgctgctcgccctgatgtgcagctggtggagtctgggggaggattggtgcaggctgggggctctctgagactctcctgtgcagcctctggaggcaccttaagtaagaataccgtggcttgggtccgccaggctccagggaaggagcgtgggtttgtaacgtctattacctgtgatggtcgtacgacatactatgcgaactccgtgaagggccgattccccatctccagagacaacgccgagaacacagtgtatctgcaaatgaacagcctgaaacctgaggatacggccggttatgtctgtgcagacttagggaagtggcctgcgggttcggcggactactggggccaggggacccacgtcaccgtctcctccactagtaccacgacgccagcgccgcgaccaccaacaccggcgcccaccatcgcgtcgcagcccctgtccctgcgcccagaggcgtgccggccagcggcggggggcgcagtgcacacgagggggctggacttcgcctgtgatatctacatctgggcgcccttggccgggacttgtggggtccttctcctgtcactggttatcaccctttactgcaaacggggcagaaagaaactcctgtatatattcaaacaaccatttatgagaccagtacaaactactcaagaggaagatggctgtagctgccgatttccagaagaagaagaaggaggatgtgaactgagagtgaagttcagcaggagcgcagacgcccccgcgtaccagcagggccagaaccagctctataacgagctcaatctaggacgaagagaggagtacgatgttttggacaagagacgtggccgggaccctgagatggggggaaagccgagaaggaagaaccctcaggaaggcctgtacaatgaactgcagaaagataagatggcggaggcctacagtgagattgggatgaaaggcgagcgccggaggggcaaggggcacgatggcctttaccagggtctcagtacagccaccaaggacacctacgacgcccttcacatgcaggccctgccccctcgctaa

SEQ ID NO: 280 - DNA, 1104 bp, synthetic construct
  source 1..1104: mol_type = other DNA
atggctctgcccgtcaccgctctgctgctgcctctggctctgctgctgcacgctgctcgccctcaggtaaagctggaggagtctgggggaggcttggtgcagcctggggggtctctgagactctcctgtacagcctcggaattcacattcagtgactactggatgcattgggtccgtcaggctccggggaaggggctcgagtgggtcgcatctatagatactagtggacagaccacatactatgcagactccctgaagggccgattcaccatctccagagacaacgccaagagcacgttgtatctgcaaatgaacagtctgaaatctgaagacacgggcgtgtatttctgtgcaaaacgatataggggtggtacctggtatggcatggccaactggggcaaagggacccaggtcaccgtctcctcaactagtaccacgacgccagcgccgcgaccaccaacaccggcgcccaccatcgcgtcgcagcccctgtccctgcgcccagaggcgtgccggccagcggcggggggcgcagtgcacacgagggggctggacttcgcctgtgatatctacatctgggcgcccttggccgggacttgtggggtccttctcctgtcactggttatcaccctttactgcaaacggggcagaaagaaactcctgtatatattcaaacaaccatttatgagaccagtacaaactactcaagaggaagatggctgtagctgccgatttccagaagaagaagaaggaggatgtgaactgagagtgaagttcagcaggagcgcagacgcccccgcgtaccagcagggccagaaccagctctataacgagctcaatctaggacgaagagaggagtacgatgttttggacaagagacgtggccgggaccctgagatggggggaaagccgagaaggaagaaccctcaggaaggcctgtacaatgaactgcagaaagataagatggcggaggcctacagtgagattgggatgaaaggcgagcgccggaggggcaaggggcacgatggcctttaccagggtctcagtacagccaccaaggacacctacgacgcccttcacatgcaggccctgccccctcgctaa

SEQ ID NO: 281 - DNA, 1101 bp, synthetic construct
  source 1..1101: mol_type = other DNA
atggctctgcccgtcaccgctctgctgctgcctctggctctgctgctgcacgctgctcgccctcaggtgcagctggtggagtctgggggaggattggtgcaggctgggggctctctgagactctcctgtgcagcctctggacgcaccttaagtagtaataccatggcttggttccgccaggctccagggaaggagcgtgagtttgtagcgtctactacctggaatggtcgtagcacatactatgcagactccgtgaagggccgattcaccatctccagagacaacgccaagaacacgatgtatctgcaaatgaacagcctgaaacctgaggatacggccgtttatgtctgtgcagacttagggaaatggcctgcgggcccggcggactactggggccaggggacccaggtcaccgtctcctcaactagtaccacgacgccagcgccgcgaccaccaacaccggcgcccaccatcgcgtcgcagcccctgtccctgcgcccagaggcgtgccggccagcggcggggggcgcagtgcacacgagggggctggacttcgcctgtgatatctacatctgggcgcccttggccgggacttgtggggtccttctcctgtcactggttatcaccctttactgcaaacggggcagaaagaaactcctgtatatattcaaacaaccatttatgagaccagtacaaactactcaagaggaagatggctgtagctgccgatttccagaagaagaagaaggaggatgtgaactgagagtgaagttcagcaggagcgcagacgcccccgcgtaccagcagggccagaaccagctctataacgagctcaatctaggacgaagagaggagtacgatgttttggacaagagacgtggccgggaccctgagatggggggaaagccgagaaggaagaaccctcaggaaggcctgtacaatgaactgcagaaagataagatggcggaggcctacagtgagattgggatgaaaggcgagcgccggaggggcaaggggcacgatggcctttaccagggtctcagtacagccaccaaggacacctacgacgcccttcacatgcaggccctgccccctcgctaa

SEQ ID NO: 282 - DNA, 1089 bp, synthetic construct
  source 1..1089: mol_type = other DNA
atggctctgcccgtcaccgctctgctgctgcctctggctctgctgctgcacgctgctcgccctcaggtgcagctggtggagtctgggggaggattggtgcaggctgggggctctctgagactctcctgtgcagcctctggacgcaccttcaccatggggtggttccgtcaggctccagggaagcagcgcgaattggtcgcagatattagtggtggtcgcacaaactatgcagattccgtgaagggacgattcaccatctccagagacaacgccaagaacacggtatatctgcaaatgaacagcctgaaacctgaggacacggccgtttattactgtgcagcagaccggaaatcagtaatgtctattcggcccgactactggggccaggggacccaggtcaccgtctcctcaactagtaccacgacgccagcgccgcgaccaccaacaccggcgcccaccatcgcgtcgcagcccctgtccctgcgcccagaggcgtgccggccagcggcggggggcgcagtgcacacgagggggctggacttcgcctgtgatatctacatctgggcgcccttggccgggacttgtggggtccttctcctgtcactggttatcaccctttactgcaaacggggcagaaagaaactcctgtatatattcaaacaaccatttatgagaccagtacaaactactcaagaggaagatggctgtagctgccgatttccagaagaagaagaaggaggatgtgaactgagagtgaagttcagcaggagcgcagacgcccccgcgtaccagcagggccagaaccagctctataacgagctcaatctaggacgaagagaggagtacgatgttttggacaagagacgtggccgggaccctgagatggggggaaagccgagaaggaagaaccctcaggaaggcctgtacaatgaactgcagaaagataagatggcggaggcctacagtgagattgggatgaaaggcgagcgccggaggggcaaggggcacgatggcctttaccagggtctcagtacagccaccaaggacacctacgacgcccttcacatgcaggccctgccccctcgctaa

SEQ ID NO: 283 - DNA, 1053 bp, synthetic construct
  source 1..1053: mol_type = other DNA
atggctctgcccgtcaccgctctgctgctgcctctggctctgctgctgcacgctgctcgccctcaggtgcagctggtggagtctgggggaggcttggtgcaggctggggcctctctgagactctcctgtgcagcctctggacgcaccttcaccgtggcagctattagtttgagtcctactttagcatattatgcagagtccgtgaagggccgattcaccatcagccgagacaacgccaagaacacggtggttttgcaaatgaacagcctgaaacctgaggacacggccctttattactgtgcagcagaccggaaatcagtaatgtctattcggcccgactactggggccaggggacccaggtcaccgtctcctcaactagtaccacgacgccagcgccgcgaccaccaacaccggcgcccaccatcgcgtcgcagcccctgtccctgcgcccagaggcgtgccggccagcggcggggggcgcagtgcacacgagggggctggacttcgcctgtgatatctacatctgggcgcccttggccgggacttgtggggtccttctcctgtcactggttatcaccctttactgcaaacggggcagaaagaaactcctgtatatattcaaacaaccatttatgagaccagtacaaactactcaagaggaagatggctgtagctgccgatttccagaagaagaagaaggaggatgtgaactgagagtgaagttcagcaggagcgcagacgcccccgcgtaccagcagggccagaaccagctctataacgagctcaatctaggacgaagagaggagtacgatgttttggacaagagacgtggccgggaccctgagatggggggaaagccgagaaggaagaaccctcaggaaggcctgtacaatgaactgcagaaagataagatggcggaggcctacagtgagattgggatgaaaggcgagcgccggaggggcaaggggcacgatggcctttaccagggtctcagtacagccaccaaggacacctacgacgcccttcacatgcaggccctgccccctcgctaa

SEQ ID NO: 284 - DNA, 1116 bp, synthetic construct
  source 1..1116: mol_type = other DNA
atggctctgcccgtcaccgctctgctgctgcctctggctctgctgctgcacgctgctcgccctgatgtgcagctggtggagtctgggggaggattggagcaggctgggggctctctgagactctcctgtgcagcctctggaggcaccttaagtaaaaataccgtggcttggttccgccaggctccagggaaggagcgtgggtttgtagcgtctattacctgggatggtcgtacgacatactatgcagactccgtgaagggccgattcaccatctccagagacaacgccaagaacacagtgtatctgcaaatgaacagcctgaaacctgaggatacggccgtttattactgtgcgtcgacggcatcgtgccacctcttcggattggggtccggggcctttgtgtcctggggccgggggacccaggtcaccgtctcctcaactagtaccacgacgccagcgccgcgaccaccaacaccggcgcccaccatcgcgtcgcagcccctgtccctgcgcccagaggcgtgccggccagcggcggggggcgcagtgcacacgagggggctggacttcgcctgtgatatctacatctgggcgcccttggccgggacttgtggggtccttctcctgtcactggttatcaccctttactgcaaacggggcagaaagaaactcctgtatatattcaaacaaccatttatgagaccagtacaaactactcaagaggaagatggctgtagctgccgatttccagaagaagaagaaggaggatgtgaactgagagtgaagttcagcaggagcgcagacgcccccgcgtaccagcagggccagaaccagctctataacgagctcaatctaggacgaagagaggagtacgatgttttggacaagagacgtggccgggaccctgagatggggggaaagccgagaaggaagaaccctcaggaaggcctgtacaatgaactgcagaaagataagatggcggaggcctacagtgagattgggatgaaaggcgagcgccggaggggcaaggggcacgatggcctttaccagggtctcagtacagccaccaaggacacctacgacgcccttcacatgcaggccctgccccctcgctaa

SEQ ID NO: 285 - DNA, 1089 bp, synthetic construct
  source 1..1089: mol_type = other DNA
atggctctgcccgtcaccgctctgctgctgcctctggctctgctgctgcacgctgctcgccctgcggtgcagctggtggagtctgggggaggattggtgcaggctgggggctctctgagactctcctgtgcagcctctggacgcaccttcaccatggggtggttccatcaggctccagggaaggagcgtgagtttgtagcagctattagtttgagtcctactttagcatattatgcagagtccgtgaagggccgattcaccatcagccgagacaacgccaagaacacggtggttttgcaaatgaacagcctgaaacctgaggacacggccctttattactgtgcagcatccaaggatagatattcggaatatgagtactggggccaggggacccaggtcaccgtctcctcaactagtaccacgacgccagcgccgcgaccaccaacaccggcgcccaccatcgcgtcgcagcccctgtccctgcgcccagaggcgtgccggccagcggcggggggcgcagtgcacacgagggggctggacttcgcctgtgatatctacatctgggcgcccttggccgggacttgtggggtccttctcctgtcactggttatcaccctttactgcaaacggggcagaaagaaactcctgtatatattcaaacaaccatttatgagaccagtacaaactactcaagaggaagatggctgtagctgccgatttccagaagaagaagaaggaggatgtgaactgagagtgaagttcagcaggagcgcagacgcccccgcgtaccagcagggccagaaccagctctataacgagctcaatctaggacgaagagaggagtacgatgttttggacaagagacgtggccgggaccctgagatggggggaaagccgagaaggaagaaccctcaggaaggcctgtacaatgaactgcagaaagataagatggcggaggcctacagtgagattgggatgaaaggcgagcgccggaggggcaaggggcacgatggcctttaccagggtctcagtacagccaccaaggacacctacgacgcccttcacatgcaggccctgccccctcgctaa

SEQ ID NO: 286 - DNA, 1083 bp, synthetic construct
  source 1..1083: mol_type = other DNA
atggctctgcccgtcaccgctctgctgctgcctctggctctgctgctgcacgctgctcgccctcaggtaaagctggaggagtctgggggaggattggtgcaggctgggggctctctgagactctcctgtgcagcctctggacgcaccttcaccatggggtggttccgtcaggctccagggaaggagcgtgagtttgtagcagctattagtttgagtcctactttagcatattatgcagagtccgtgaagggccgattcaccatcagccgagacaacgccaagaacacggtggttttgcaaatgaacagcctgaaacctgaggacacggccctttattactgtgcaaaaaaaaacggggggcctgtggactactggggcaaagggacccaggtcaccgtctcctcaactagtaccacgacgccagcgccgcgaccaccaacaccggcgcccaccatcgcgtcgcagcccctgtccctgcgcccagaggcgtgccggccagcggcggggggcgcagtgcacacgagggggctggacttcgcctgtgatatctacatctgggcgcccttggccgggacttgtggggtccttctcctgtcactggttatcaccctttactgcaaacggggcagaaagaaactcctgtatatattcaaacaaccatttatgagaccagtacaaactactcaagaggaagatggctgtagctgccgatttccagaagaagaagaaggaggatgtgaactgagagtgaagttcagcaggagcgcagacgcccccgcgtaccagcagggccagaaccagctctataacgagctcaatctaggacgaagagaggagtacgatgttttggacaagagacgtggccgggaccctgagatggggggaaagccgagaaggaagaaccctcaggaaggcctgtacaatgaactgcagaaagataagatggcggaggcctacagtgagattgggatgaaaggcgagcgccggaggggcaaggggcacgatggcctttaccagggtctcagtacagccaccaaggacacctacgacgcccttcacatgcaggccctgccccctcgctaa

SEQ ID NO: 287 - DNA, 1098 bp, synthetic construct
  source 1..1098: mol_type = other DNA
atggctctgcccgtcaccgctctgctgctgcctctggctctgctgctgcacgctgctcgccctgatgtgcagctggtggagtctgggggaggcttggtgcagcctggggggtctctgagactctcctgtgcagcctctggacggaccttcagtagcattgtcatgggctggttccgccaggctccagggaaggagcgtgagtttgtaggagcgattatgtggaatgatggtattacatacttgcaagactccgtgaagggccgatttaccatcttcagagacaacgccaagaacacggtgtatctgcaaatgaacagcctgaaacttgaggatacggccgtttattactgtgcagcatccaagggtagatactcggaatatgagtactggggccaggggacccaggtcaccgtctcctcaactagtaccacgacgccagcgccgcgaccaccaacaccggcgcccaccatcgcgtcgcagcccctgtccctgcgcccagaggcgtgccggccagcggcggggggcgcagtgcacacgagggggctggacttcgcctgtgatatctacatctgggcgcccttggccgggacttgtggggtccttctcctgtcactggttatcaccctttactgcaaacggggcagaaagaaactcctgtatatattcaaacaaccatttatgagaccagtacaaactactcaagaggaagatggctgtagctgccgatttccagaagaagaagaaggaggatgtgaactgagagtgaagttcagcaggagcgcagacgcccccgcgtaccagcagggccagaaccagctctataacgagctcaatctaggacgaagagaggagtacgatgttttggacaagagacgtggccgggaccctgagatggggggaaagccgagaaggaagaaccctcaggaaggcctgtacaatgaactgcagaaagataagatggcggaggcctacagtgagattgggatgaaaggcgagcgccggaggggcaaggggcacgatggcctttaccagggtctcagtacagccaccaaggacacctacgacgcccttcacatgcaggccctgccccctcgctaa

SEQ ID NO: 288 - DNA, 1095 bp, synthetic construct
  source 1..1095: mol_type = other DNA
atggctctgcccgtcaccgctctgctgctgcctctggctctgctgctgcacgctgctcgccctcaggtaaagctggaggaatctgggggaagattggtgcaggctgggggctctctgaaactctcctgggcagcctctggacgcaccttcaccatggggtggttccgtcaggctccagggaaggaacgtgagtttgtaacagctattaatttgagtcctactttaacatattatgcagaatccgtgaagggccgattccccatcagccgaaacaacgcccagaacacggtggttttgcaaatgaacagcctgaaacctgaggacacggccctttattactgtgcagcagaacggaaatcagtaatggctattccgcccgactactggggccaggggacccaggtcaccgtctcctcaactagtaccacgacgccagcgccgcgaccaccaacaccggcgcccaccatcgcgtcgcagcccctgtccctgcgcccagaggcgtgccggccagcggcggggggcgcagtgcacacgagggggctggacttcgcctgtgatatctacatctgggcgcccttggccgggacttgtggggtccttctcctgtcactggttatcaccctttactgcaaacggggcagaaagaaactcctgtatatattcaaacaaccatttatgagaccagtacaaactactcaagaggaagatggctgtagctgccgatttccagaagaagaagaaggaggatgtgaactgagagtgaagttcagcaggagcgcagacgcccccgcgtaccagcagggccagaaccagctctataacgagctcaatctaggacgaagagaggagtacgatgttttggacaagagacgtggccgggaccctgagatggggggaaagccgagaaggaagaaccctcaggaaggcctgtacaatgaactgcagaaagataagatggcggaggcctacagtgagattgggatgaaaggcgagcgccggaggggcaaggggcacgatggcctttaccagggtctcagtacagccaccaaggacacctacgacgcccttcacatgcaggccctgccccctcgctaa

SEQ ID NO: 289 - DNA, 1095 bp, synthetic construct
  source 1..1095: mol_type = other DNA
atggctctgcccgtcaccgctctgctgctgcctctggctctgctgctgcacgctgctcgccctgaggtgcagctggtggagtctgggggaggattggtgcaggctgggggctctctgagactctcctgtgcagcctctggacgcaccttcaccatgggggggttccgtcgggttcctcgggatgagcgggagtttgtagcatctattactttgattcctacttttccttattatgcatattccgtgaagggccgattcgccctcttccgagacaaccccaacaacaccgtgattttgctgatgatcagcctgaaacctgaggacccggacctttattactgtgcttcataccggaaatacctaatgtctattctgcccgactactggggccaggggacccagggcaccgtctcctccactagtaccacgacgccagcgccgcgaccaccaacaccggcgcccaccatcgcgtcgcagcccctgtccctgcgcccagaggcgtgccggccagcggcggggggcgcagtgcacacgagggggctggacttcgcctgtgatatctacatctgggcgcccttggccgggacttgtggggtccttctcctgtcactggttatcaccctttactgcaaacggggcagaaagaaactcctgtatatattcaaacaaccatttatgagaccagtacaaactactcaagaggaagatggctgtagctgccgatttccagaagaagaagaaggaggatgtgaactgagagtgaagttcagcaggagcgcagacgcccccgcgtaccagcagggccagaaccagctctataacgagctcaatctaggacgaagagaggagtacgatgttttggacaagagacgtggccgggaccctgagatggggggaaagccgagaaggaagaaccctcaggaaggcctgtacaatgaactgcagaaagataagatggcggaggcctacagtgagattgggatgaaaggcgagcgccggaggggcaaggggcacgatggcctttaccagggtctcagtacagccaccaaggacacctacgacgcccttcacatgcaggccctgccccctcgctaa

SEQ ID NO: 290 - DNA, 1113 bp, synthetic construct
  source 1..1113: mol_type = other DNA
atggctctgcccgtcaccgctctgctgctgcctctggctctgctgctgcacgctgctcgccctcaggtaaagctggaggagtctgggggaggattggtgcaggctgggggctctctgagactctcctgtgcagcctctggacgcaccttcaccatggggtggttccgtcaggctccagggaaggagcgtgagtttgtagcagctattagtttgagtcctactttagcatattatgcagagtccgtgaagggccgattcaccatcagccgagacaacgccaagaacacggtggatctgcaaatgaacagcctgaaacctgaggacacggccgtctatttctgtgcagcaaatcggaactcccaacgggtaattgcggcactgtcctggattggcatgaactactggggcgaatggacccaggtcaccgtctcctccactagtaccacgacgccagcgccgcgaccaccaacaccggcgcccaccatcgcgtcgcagcccctgtccctgcgcccagaggcgtgccggccagcggcggggggcgcagtgcacacgagggggctggacttcgcctgtgatatctacatctgggcgcccttggccgggacttgtggggtccttctcctgtcactggttatcaccctttactgcaaacggggcagaaagaaactcctgtatatattcaaacaaccatttatgagaccagtacaaactactcaagaggaagatggctgtagctgccgatttccagaagaagaagaaggaggatgtgaactgagagtgaagttcagcaggagcgcagacgcccccgcgtaccagcagggccagaaccagctctataacgagctcaatctaggacgaagagaggagtacgatgttttggacaagagacgtggccgggaccctgagatggggggaaagccgagaaggaagaaccctcaggaaggcctgtacaatgaactgcagaaagataagatggcggaggcctacagtgagattgggatgaaaggcgagcgccggaggggcaaggggcacgatggcctttaccagggtctcagtacagccaccaaggacacctacgacgcccttcacatgcaggccctgccccctcgctaa

SEQ ID NO: 291 - DNA, 1089 bp, synthetic construct
  source 1..1089: mol_type = other DNA
atggctctgcccgtcaccgctctgctgctgcctctggctctgctgctgcacgctgctcgccctcaggtgcagctggtggagtctgggggaggattggtgcaggctgggggctctctgagactctcctgtgcagcctctggacgcaccttcaccatggggtggttccgtcaggctccagggaaggagcgtgagtttgtagcagctattagtttgagtcctactttagcatattatgcagagtccgtgaagggccgattcaccatctccagagacaacgccaagaagacgctgtatctgcgaatgaatagcctgaaacctgaggacacggccgtttactactgtgcagcacgtcggatcgacgcagctgactttgattcctgggggcaggggacccaggtcaccgtctcctcaactagtaccacgacgccagcgccgcgaccaccaacaccggcgcccaccatcgcgtcgcagcccctgtccctgcgcccagaggcgtgccggccagcggcggggggcgcagtgcacacgagggggctggacttcgcctgtgatatctacatctgggcgcccttggccgggacttgtggggtccttctcctgtcactggttatcaccctttactgcaaacggggcagaaagaaactcctgtatatattcaaacaaccatttatgagaccagtacaaactactcaagaggaagatggctgtagctgccgatttccagaagaagaagaaggaggatgtgaactgagagtgaagttcagcaggagcgcagacgcccccgcgtaccagcagggccagaaccagctctataacgagctcaatctaggacgaagagaggagtacgatgttttggacaagagacgtggccgggaccctgagatggggggaaagccgagaaggaagaaccctcaggaaggcctgtacaatgaactgcagaaagataagatggcggaggcctacagtgagattgggatgaaaggcgagcgccggaggggcaaggggcacgatggcctttaccagggtctcagtacagccaccaaggacacctacgacgcccttcacatgcaggccctgccccctcgctaa

SEQ ID NO: 292 - DNA, 1089 bp, synthetic construct
  source 1..1089: mol_type = other DNA
atggctctgcccgtcaccgctctgctgctgcctctggctctgctgctgcacgctgctcgccctcaggtaaagctggaggagtctgggggaggattggtgcaggctgggggctctctgagactctcctgtgcagcctctggacgcaccttcaccatggggtggttccgtcgggctccagggaaggagcgtgagtctgttgcagttattggctggagagatattaacgcaagctatgcagactccgtgaagggccgattcgccatctccagagacaacgccaagaagacgctgtatctgcagatgaatagcctgaaacctgaggacacggccgtttactactgtgcagcacgtcggatcgacgcaactgactttgattcctgggggcaggggacccaggtcaccgtctcctcaactagtaccacgacgccagcgccgcgaccaccaacaccggcgcccaccatcgcgtcgcagcccctgtccctgcgcccagaggcgtgccggccagcggcggggggcgcagtgcacacgagggggctggacttcgcctgtgatatctacatctgggcgcccttggccgggacttgtggggtccttctcctgtcactggttatcaccctttactgcaaacggggcagaaagaaactcctgtatatattcaaacaaccatttatgagaccagtacaaactactcaagaggaagatggctgtagctgccgatttccagaagaagaagaaggaggatgtgaactgagagtgaagttcagcaggagcgcagacgcccccgcgtaccagcagggccagaaccagctctataacgagctcaatctaggacgaagagaggagtacgatgttttggacaagagacgtggccgggaccctgagatggggggaaagccgagaaggaagaaccctcaggaaggcctgtacaatgaactgcagaaagataagatggcggaggcctacagtgagattgggatgaaaggcgagcgccggaggggcaaggggcacgatggcctttaccagggtctcagtacagccaccaaggacacctacgacgcccttcacatgcaggccctgccccctcgctaa

SEQ ID NO: 293 - DNA, 1098 bp, synthetic construct
  source 1..1098: mol_type = other DNA
atggctctgcccgtcaccgctctgctgctgcctctggctctgctgctgcacgctgctcgccctcaggtaaagctggaggagtctgggggaggattggtgcagactgggggctctctgagactctcctgtgcagcctctgaacacaccttcagtaaccatgtcatgggctggttccgccaggctccagggaaggagcgtgagtctgttgcagttattggctggagagatattagcacaagctatgcagactccgtgaagggccgattcaccatctccagagacaacgccaagaagacgctgtatctgcaaatgaatagcctgaaacctgaggacacggccgtttactactgtgcagcacgtcggatcgacgcagctgactttgattcccgggggcaggggacccaggtcaccgtctcctcaactagtaccacgacgccagcgccgcgaccaccaacaccggcgcccaccatcgcgtcgcagcccctgtccctgcgcccagaggcgtgccggccagcggcggggggcgcagtgcacacgagggggctggacttcgcctgtgatatctacatctgggcgcccttggccgggacttgtggggtccttctcctgtcactggttatcaccctttactgcaaacggggcagaaagaaactcctgtatatattcaaacaaccatttatgagaccagtacaaactactcaagaggaagatggctgtagctgccgatttccagaagaagaagaaggaggatgtgaactgagagtgaagttcagcaggagcgcagacgcccccgcgtaccagcagggccagaaccagctctataacgagctcaatctaggacgaagagaggagtacgatgttttggacaagagacgtggccgggaccctgagatggggggaaagccgagaaggaagaaccctcaggaaggcctgtacaatgaactgcagaaagataagatggcggaggcctacagtgagattgggatgaaaggcgagcgccggaggggcaaggggcacgatggcctttaccagggtctcagtacagccaccaaggacacctacgacgcccttcacatgcaggccctgccccctcgctaa

SEQ ID NO: 294 - DNA, 1110 bp, synthetic construct
  source 1..1110: mol_type = other DNA
atggctctgcccgtcaccgctctgctgctgcctctggctctgctgctgcacgctgctcgccctgccgtgcagctggtggattctgggggaggattggtgcaggctgggggctctctgagaatttcctgtgcagtctctggacgcacctccagtaactatatattggcctggttccgtcaggctccaggaaaagagcgtgactttgtagcacatattagccggagtggtggtaagtccggctatggagactccgtgaagggccgattcaccatctccagagacaacgccgagaacacggtcagggtgtatctgcaaatgaacagtctgaaacctggggacacggccgtctattactgtaatcgccccctctggtacggaagtcccacgttgattgactactggggccaggggacccaggtcaccgtctcctcaactagtaccacgacgccagcgccgcgaccaccaacaccggcgcccaccatcgcgtcgcagcccctgtccctgcgcccagaggcgtgccggccagcggcggggggcgcagtgcacacgagggggctggacttcgcctgtgatatctacatctgggcgcccttggccgggacttgtggggtccttctcctgtcactggttatcaccctttactgcaaacggggcagaaagaaactcctgtatatattcaaacaaccatttatgagaccagtacaaactactcaagaggaagatggctgtagctgccgatttccagaagaagaagaaggaggatgtgaactgagagtgaagttcagcaggagcgcagacgcccccgcgtaccagcagggccagaaccagctctataacgagctcaatctaggacgaagagaggagtacgatgttttggacaagagacgtggccgggaccctgagatggggggaaagccgagaaggaagaaccctcaggaaggcctgtacaatgaactgcagaaagataagatggcggaggcctacagtgagattgggatgaaaggcgagcgccggaggggcaaggggcacgatggcctttaccagggtctcagtacagccaccaaggacacctacgacgcccttcacatgcaggccctgccccctcgctaa

SEQ ID NO: 295 - DNA, 1095 bp, synthetic construct
  source 1..1095: mol_type = other DNA
atggctctgcccgtcaccgctctgctgctgcctctggctctgctgctgcacgctgctcgccctgcggtgcagctggtggagtctgggggaggcttggtgcagcctggggggtctctgagactctcctgtgcagcctctggacgcaccttcaccatggggtggttccgtcaggctccagggaaggagcgtgagtttgtagcagctattagtttgagtcctactttagcatattatgcagagtccgtgaagggccgattcaccatcagccgagacaacgccaagaacacggtggttttgcaaatgaacagcctgaaacctgaggacacggccctttattactgtgcagcagaccggaaatcagtaatgtctattcggcccgactactggggccaggggacccaggtcaccgtctcctcaactagtaccacgacgccagcgccgcgaccaccaacaccggcgcccaccatcgcgtcgcagcccctgtccctgcgcccagaggcgtgccggccagcggcggggggcgcagtgcacacgagggggctggacttcgcctgtgatatctacatctgggcgcccttggccgggacttgtggggtccttctcctgtcactggttatcaccctttactgcaaacggggcagaaagaaactcctgtatatattcaaacaaccatttatgagaccagtacaaactactcaagaggaagatggctgtagctgccgatttccagaagaagaagaaggaggatgtgaactgagagtgaagttcagcaggagcgcagacgcccccgcgtaccagcagggccagaaccagctctataacgagctcaatctaggacgaagagaggagtacgatgttttggacaagagacgtggccgggaccctgagatggggggaaagccgagaaggaagaaccctcaggaaggcctgtacaatgaactgcagaaagataagatggcggaggcctacagtgagattgggatgaaaggcgagcgccggaggggcaaggggcacgatggcctttaccagggtctcagtacagccaccaaggacacctacgacgcccttcacatgcaggccctgccccctcgctaa

SEQ ID NO: 296 - DNA, 1095 bp, synthetic construct
  source 1..1095: mol_type = other DNA
atggctctgcccgtcaccgctctgctgctgcctctggctctgctgctgcacgctgctcgccctgcggtgcagctggtggagtctgggggaggattggtgcaggctgggggctctctgagactctcctgtgcagcctctggacgcaccttcaccatggggtggttccgtcaggctccagggaaggagcgtgagtttgtagcagctattagtttgagtcctactttagcatattatgcagagtccgtgaagggccgattcaccatcagccgagacaacgccaagaacacggtggttttgcaaatgaacagcctgaaacctgaggacacggccctttattactgtgcagcagaccggaaatcagtaatgtctattcggcccgactactggggccaggggacccaggtcaccgtctcctcaactagtaccacgacgccagcgccgcgaccaccaacaccggcgcccaccatcgcgtcgcagcccctgtccctgcgcccagaggcgtgccggccagcggcggggggcgcagtgcacacgagggggctggacttcgcctgtgatatctacatctgggcgcccttggccgggacttgtggggtccttctcctgtcactggttatcaccctttactgcaaacggggcagaaagaaactcctgtatatattcaaacaaccatttatgagaccagtacaaactactcaagaggaagatggctgtagctgccgatttccagaagaagaagaaggaggatgtgaactgagagtgaagttcagcaggagcgcagacgcccccgcgtaccagcagggccagaaccagctctataacgagctcaatctaggacgaagagaggagtacgatgttttggacaagagacgtggccgggaccctgagatggggggaaagccgagaaggaagaaccctcaggaaggcctgtacaatgaactgcagaaagataagatggcggaggcctacagtgagattgggatgaaaggcgagcgccggaggggcaaggggcacgatggcctttaccagggtctcagtacagccaccaaggacacctacgacgcccttcacatgcaggccctgccccctcgctaa

SEQ ID NO: 297 - DNA, 1104 bp, synthetic construct
  source 1..1104: mol_type = other DNA
atggctctgcccgtcaccgctctgctgctgcctctggctctgctgctgcacgctgctcgccctgatgtgcagctggtggagtctgggggaggatcggtgcagactgggggctctctgagactctcctgtacagcctctggacgcaccctcaataactttgtcatgggctggttccgtcaggctccagggaaggagcgtgagtttgtagcagctattagtttgagtcctactttagcatattatgtagagtccgtgaagggccgattcaccatcagccgagacaacgccaagaacacggtggttttgcaaatgaacagcctgaaacctgaggacacggccctttattactgtgcagcagaccggaaatcagtaatgtctattcggcccgactactggggccaggggacccaggtcaccgtctcctcaactagtaccacgacgccagcgccgcgaccaccaacaccggcgcccaccatcgcgtcgcagcccctgtccctgcgcccagaggcgtgccggccagcggcggggggcgcagtgcacacgagggggctggacttcgcctgtgatatctacatctgggcgcccttggccgggacttgtggggtccttctcctgtcactggttatcaccctttactgcaaacggggcagaaagaaactcctgtatatattcaaacaaccatttatgagaccagtacaaactactcaagaggaagatggctgtagctgccgatttccagaagaagaagaaggaggatgtgaactgagagtgaagttcagcaggagcgcagacgcccccgcgtaccagcagggccagaaccagctctataacgagctcaatctaggacgaagagaggagtacgatgttttggacaagagacgtggccgggaccctgagatggggggaaagccgagaaggaagaaccctcaggaaggcctgtacaatgaactgcagaaagataagatggcggaggcctacagtgagattgggatgaaaggcgagcgccggaggggcaaggggcacgatggcctttaccagggtctcagtacagccaccaaggacacctacgacgcccttcacatgcaggccctgccccctcgctaa

SEQ ID NO: 298 - protein, 495 aa, synthetic construct
MALPVTALLLPLALLLHAARPQVQLVESGGGLVQPGGSLRLSCEASGFTLDYYAIGWFRQAPGKEREGVICISRSDGSTYYADSVKGRFTISRDNAKKTVYLQMISLKPEDTAAYYCAAGADCSGYLRDYEFRGQGTQVTVSSGGGGSQVQLVESGGGLVQPGGSLRLSCEASGFTLDYYAIGWFRQAPGKEREGVICISRSDGSTYYADSVKGRFTISRDNAKKTVYLQMISLKPEDTAAYYCAAGADCSGYLRDYEFRGQGTQVTVSSTSTTTPAPRPPTPAPTIASQPLSLRPEACRPAAGGAVHTRGLDFACDIYIWAPLAGTCGVLLLSLVITLYCKRGRKKLLYIFKQPFMRPVQTTQEEDGCSCRFPEEEEGGCELRVKFSRSADAPAYQQGQNQLYNELNLGRREEYDVLDKRRGRDPEMGGKPRRKNPQEGLYNELQKDKMAEAYSEIGMKGERRRGKGHDGLYQGLSTATKDTYDALHMQALPPR

SEQ ID NO: 299 - protein, 622 aa, synthetic construct
MALPVTALLLPLALLLHAARPQVQLVESGGGLVQPGGSLRLSCEASGFTLDYYAIGWFRQAPGKEREGVICISRSDGSTYYADSVKGRFTISRDNAKKTVYLQMISLKPEDTAAYYCAAGADCSGYLRDYEFRGQGTQVTVSSGGGGSQVQLVESGGGLVQPGGSLRLSCEASGFTLDYYAIGWFRQAPGKEREGVICISRSDGSTYYADSVKGRFTISRDNAKKTVYLQMISLKPEDTAAYYCAAGADCSGYLRDYEFRGQGTQVTVSSGGGGSQVQLVESGGGLVQPGGSLRLSCEASGFTLDYYAIGWFRQAPGKEREGVICISRSDGSTYYADSVKGRFTISRDNAKKTVYLQMISLKPEDTAAYYCAAGADCSGYLRDYEFRGQGTQVTVSSTSTTTPAPRPPTPAPTIASQPLSLRPEACRPAAGGAVHTRGLDFACDIYIWAPLAGTCGVLLLSLVITLYCKRGRKKLLYIFKQPFMRPVQTTQEEDGCSCRFPEEEEGGCELRVKFSRSADAPAYQQGQNQLYNELNLGRREEYDVLDKRRGRDPEMGGKPRRKNPQEGLYNELQKDKMAEAYSEIGMKGERRRGKGHDGLYQGLSTATKDTYDALHMQALPPR

SEQ ID NO: 300 - protein, 488 aa, synthetic construct
MALPVTALLLPLALLLHAARPQVKLEESGGGLVQAGRSLRLSCAASEHTFSSHVMGWFRQAPGKERESVAVIGWRDISTSYADSVKGRFTISRDNAKKTLYLQMNSLKPEDTAVYYCAARRIDAADFDSWGQGTQVTVSSGGGGSEVQLVESGGGLVQAGGSLRLSCAASGRTFTMGWFRQAPGKEREFVAAISLSPTLAYYAESVKGRFTISRDNAKNTVVLQMNSLKPEDTALYYCAADRKSVMSIRPDYWGQGTQVTVSSTSTTTPAPRPPTPAPTIASQPLSLRPEACRPAAGGAVHTRGLDFACDIYIWAPLAGTCGVLLLSLVITLYCKRGRKKLLYIFKQPFMRPVQTTQEEDGCSCRFPEEEEGGCELRVKFSRSADAPAYQQGQNQLYNELNLGRREEYDVLDKRRGRDPEMGGKPRRKNPQEGLYNELQKDKMAEAYSEIGMKGERRRGKGHDGLYQGLSTATKDTYDALHMQALPPR

SEQ ID NO: 301 - protein, 498 aa, synthetic construct
MALPVTALLLPLALLLHAARPQVKLEESGGGLVQAGRSLRLSCAASEHTFSSHVMGWFRQAPGKERESVAVIGWRDISTSYADSVKGRFTISRDNAKKTLYLQMNSLKPEDTAVYYCAARRIDAADFDSWGQGTQVTVSSGGGGSGGGGSGGGGSEVQLVESGGGLVQAGGSLRLSCAASGRTFTMGWFRQAPGKEREFVAAISLSPTLAYYAESVKGRFTISRDNAKNTVVLQMNSLKPEDTALYYCAADRKSVMSIRPDYWGQGTQVTVSSTSTTTPAPRPPTPAPTIASQPLSLRPEACRPAAGGAVHTRGLDFACDIYIWAPLAGTCGVLLLSLVITLYCKRGRKKLLYIFKQPFMRPVQTTQEEDGCSCRFPEEEEGGCELRVKFSRSADAPAYQQGQNQLYNELNLGRREEYDVLDKRRGRDPEMGGKPRRKNPQEGLYNELQKDKMAEAYSEIGMKGERRRGKGHDGLYQGLSTATKDTYDALHMQALPPR

SEQ ID NO: 302 - protein, 508 aa, synthetic construct
MALPVTALLLPLALLLHAARPQVKLEESGGGLVQAGRSLRLSCAASEHTFSSHVMGWFRQAPGKERESVAVIGWRDISTSYADSVKGRFTISRDNAKKTLYLQMNSLKPEDTAVYYCAARRIDAADFDSWGQGTQVTVSSGGGGSGGGGSGGGGSGGGGSGGGGSEVQLVESGGGLVQAGGSLRLSCAASGRTFTMGWFRQAPGKEREFVAAISLSPTLAYYAESVKGRFTISRDNAKNTVVLQMNSLKPEDTALYYCAADRKSVMSIRPDYWGQGTQVTVSSTSTTTPAPRPPTPAPTIASQPLSLRPEACRPAAGGAVHTRGLDFACDIYIWAPLAGTCGVLLLSLVITLYCKRGRKKLLYIFKQPFMRPVQTTQEEDGCSCRFPEEEEGGCELRVKFSRSADAPAYQQGQNQLYNELNLGRREEYDVLDKRRGRDPEMGGKPRRKNPQEGLYNELQKDKMAEAYSEIGMKGERRRGKGHDGLYQGLSTATKDTYDALHMQALPPR

SEQ ID NO: 303 - protein, 493 aa, synthetic construct
MALPVTALLLPLALLLHAARPEVQLVESGGGLVQAGGSLRLSCAASGRTFTMGWFRQAPGKEREFVAAISLSPTLAYYAESVKGRFTISRDNAKNTVVLQMNSLKPEDTALYYCAADRKSVMSIRPDYWGQGTQVTVSSGGGGSGGGGSQVKLEESGGGLVQAGRSLRLSCAASEHTFSSHVMGWFRQAPGKERESVAVIGWRDISTSYADSVKGRFTISRDNAKKTLYLQMNSLKPEDTAVYYCAARRIDAADFDSWGQGTQVTVSSTSTTTPAPRPPTPAPTIASQPLSLRPEACRPAAGGAVHTRGLDFACDIYIWAPLAGTCGVLLLSLVITLYCKRGRKKLLYIFKQPFMRPVQTTQEEDGCSCRFPEEEEGGCELRVKFSRSADAPAYQQGQNQLYNELNLGRREEYDVLDKRRGRDPEMGGKPRRKNPQEGLYNELQKDKMAEAYSEIGMKGERRRGKGHDGLYQGLSTATKDTYDALHMQALPPR

SEQ ID NO: 304 - protein, 498 aa, synthetic construct
MALPVTALLLPLALLLHAARPEVQLVESGGGLVQAGGSLRLSCAASGRTFTMGWFRQAPGKEREFVAAISLSPTLAYYAESVKGRFTISRDNAKNTVVLQMNSLKPEDTALYYCAADRKSVMSIRPDYWGQGTQVTVSSGGGGSGGGGSGGGGSQVKLEESGGGLVQAGRSLRLSCAASEHTFSSHVMGWFRQAPGKERESVAVIGWRDISTSYADSVKGRFTISRDNAKKTLYLQMNSLKPEDTAVYYCAARRIDAADFDSWGQGTQVTVSSTSTTTPAPRPPTPAPTIASQPLSLRPEACRPAAGGAVHTRGLDFACDIYIWAPLAGTCGVLLLSLVITLYCKRGRKKLLYIFKQPFMRPVQTTQEEDGCSCRFPEEEEGGCELRVKFSRSADAPAYQQGQNQLYNELNLGRREEYDVLDKRRGRDPEMGGKPRRKNPQEGLYNELQKDKMAEAYSEIGMKGERRRGKGHDGLYQGLSTATKDTYDALHMQALPPR

SEQ ID NO: 305 - protein, 503 aa, synthetic construct
MALPVTALLLPLALLLHAARPEVQLVESGGGLVQAGGSLRLSCAASGRTFTMGWFRQAPGKEREFVAAISLSPTLAYYAESVKGRFTISRDNAKNTVVLQMNSLKPEDTALYYCAADRKSVMSIRPDYWGQGTQVTVSSGGGGSGGGGSGGGGSGGGGSQVKLEESGGGLVQAGRSLRLSCAASEHTFSSHVMGWFRQAPGKERESVAVIGWRDISTSYADSVKGRFTISRDNAKKTLYLQMNSLKPEDTAVYYCAARRIDAADFDSWGQGTQVTVSSTSTTTPAPRPPTPAPTIASQPLSLRPEACRPAAGGAVHTRGLDFACDIYIWAPLAGTCGVLLLSLVITLYCKRGRKKLLYIFKQPFMRPVQTTQEEDGCSCRFPEEEEGGCELRVKFSRSADAPAYQQGQNQLYNELNLGRREEYDVLDKRRGRDPEMGGKPRRKNPQEGLYNELQKDKMAEAYSEIGMKGERRRGKGHDGLYQGLSTATKDTYDALHMQALPPR

SEQ ID NO: 306 - protein, 489 aa, synthetic construct
MALPVTALLLPLALLLHAARPQVKLEESGGGLVQAGRSLRLSCAASEHTFSSHVMGWFRQAPGKERESVAVIGWRDISTSYADSVKGRFTISRDNAKKTLYLQMNSLKPEDTAVYYCAARRIDAADFDSWGQGTQVTVSSGGGGSAVQLVESGGGLVQAGDSLRLTCTASGRAFSTYFMAWFRQAPGKEREFVAGIAWSGGSTAYADSVKGRFTISRDNAKNTVYLQMNSLKSEDTAVYYCASRGIEVEEFGAWGQGTQVTVSSTSTTTPAPRPPTPAPTIASQPLSLRPEACRPAAGGAVHTRGLDFACDIYIWAPLAGTCGVLLLSLVITLYCKRGRKKLLYIFKQPFMRPVQTTQEEDGCSCRFPEEEEGGCELRVKFSRSADAPAYQQGQNQLYNELNLGRREEYDVLDKRRGRDPEMGGKPRRKNPQEGLYNELQKDKMAEAYSEIGMKGERRRGKGHDGLYQGLSTATKDTYDALHMQALPPR

SEQ ID NO: 307 - protein, 499 aa, synthetic construct
MALPVTALLLPLALLLHAARPQVKLEESGGGLVQAGRSLRLSCAASEHTFSSHVMGWFRQAPGKERESVAVIGWRDISTSYADSVKGRFTISRDNAKKTLYLQMNSLKPEDTAVYYCAARRIDAADFDSWGQGTQVTVSSGGGGSGGGGSGGGGSAVQLVESGGGLVQAGDSLRLTCTASGRAFSTYFMAWFRQAPGKEREFVAGIAWSGGSTAYADSVKGRFTISRDNAKNTVYLQMNSLKSEDTAVYYCASRGIEVEEFGAWGQGTQVTVSSTSTTTPAPRPPTPAPTIASQPLSLRPEACRPAAGGAVHTRGLDFACDIYIWAPLAGTCGVLLLSLVITLYCKRGRKKLLYIFKQPFMRPVQTTQEEDGCSCRFPEEEEGGCELRVKFSRSADAPAYQQGQNQLYNELNLGRREEYDVLDKRRGRDPEMGGKPRRKNPQEGLYNELQKDKMAEAYSEIGMKGERRRGKGHDGLYQGLSTATKDTYDALHMQALPPR

SEQ ID NO: 308 - protein, 509 aa, synthetic construct
MALPVTALLLPLALLLHAARPQVKLEESGGGLVQAGRSLRLSCAASEHTFSSHVMGWFRQAPGKERESVAVIGWRDISTSYADSVKGRFTISRDNAKKTLYLQMNSLKPEDTAVYYCAARRIDAADFDSWGQGTQVTVSSGGGGSGGGGSGGGGSGGGGSGGGGSAVQLVESGGGLVQAGDSLRLTCTASGRAFSTYFMAWFRQAPGKEREFVAGIAWSGGSTAYADSVKGRFTISRDNAKNTVYLQMNSLKSEDTAVYYCASRGIEVEEFGAWGQGTQVTVSSTSTTTPAPRPPTPAPTIASQPLSLRPEACRPAAGGAVHTRGLDFACDIYIWAPLAGTCGVLLLSLVITLYCKRGRKKLLYIFKQPFMRPVQTTQEEDGCSCRFPEEEEGGCELRVKFSRSADAPAYQQGQNQLYNELNLGRREEYDVLDKRRGRDPEMGGKPRRKNPQEGLYNELQKDKMAEAYSEIGMKGERRRGKGHDGLYQGLSTATKDTYDALHMQALPPR

SEQ ID NO: 309 - protein, 494 aa, synthetic construct
MALPVTALLLPLALLLHAARPAVQLVESGGGLVQAGDSLRLTCTASGRAFSTYFMAWFRQAPGKEREFVAGIAWSGGSTAYADSVKGRFTISRDNAKNTVYLQMNSLKSEDTAVYYCASRGIEVEEFGAWGQGTQVTVSSGGGGSGGGGSQVKLEESGGGLVQAGRSLRLSCAASEHTFSSHVMGWFRQAPGKERESVAVIGWRDISTSYADSVKGRFTISRDNAKKTLYLQMNSLKPEDTAVYYCAARRIDAADFDSWGQGTQVTVSSTSTTTPAPRPPTPAPTIASQPLSLRPEACRPAAGGAVHTRGLDFACDIYIWAPLAGTCGVLLLSLVITLYCKRGRKKLLYIFKQPFMRPVQTTQEEDGCSCRFPEEEEGGCELRVKFSRSADAPAYQQGQNQLYNELNLGRREEYDVLDKRRGRDPEMGGKPRRKNPQEGLYNELQKDKMAEAYSEIGMKGERRRGKGHDGLYQGLSTATKDTYDALHMQALPPR

SEQ ID NO: 310 - protein, 499 aa, synthetic construct
MALPVTALLLPLALLLHAARPAVQLVESGGGLVQAGDSLRLTCTASGRAFSTYFMAWFRQAPGKEREFVAGIAWSGGSTAYADSVKGRFTISRDNAKNTVYLQMNSLKSEDTAVYYCASRGIEVEEFGAWGQGTQVTVSSGGGGSGGGGSGGGGSQVKLEESGGGLVQAGRSLRLSCAASEHTFSSHVMGWFRQAPGKERESVAVIGWRDISTSYADSVKGRFTISRDNAKKTLYLQMNSLKPEDTAVYYCAARRIDAADFDSWGQGTQVTVSSTSTTTPAPRPPTPAPTIASQPLSLRPEACRPAAGGAVHTRGLDFACDIYIWAPLAGTCGVLLLSLVITLYCKRGRKKLLYIFKQPFMRPVQTTQEEDGCSCRFPEEEEGGCELRVKFSRSADAPAYQQGQNQLYNELNLGRREEYDVLDKRRGRDPEMGGKPRRKNPQEGLYNELQKDKMAEAYSEIGMKGERRRGKGHDGLYQGLSTATKDTYDALHMQALPPR

SEQ ID NO: 311 - protein, 504 aa, synthetic construct
MALPVTALLLPLALLLHAARPAVQLVESGGGLVQAGDSLRLTCTASGRAFSTYFMAWFRQAPGKEREFVAGIAWSGGSTAYADSVKGRFTISRDNAKNTVYLQMNSLKSEDTAVYYCASRGIEVEEFGAWGQGTQVTVSSGGGGSGGGGSGGGGSGGGGSQVKLEESGGGLVQAGRSLRLSCAASEHTFSSHVMGWFRQAPGKERESVAVIGWRDISTSYADSVKGRFTISRDNAKKTLYLQMNSLKPEDTAVYYCAARRIDAADFDSWGQGTQVTVSSTSTTTPAPRPPTPAPTIASQPLSLRPEACRPAAGGAVHTRGLDFACDIYIWAPLAGTCGVLLLSLVITLYCKRGRKKLLYIFKQPFMRPVQTTQEEDGCSCRFPEEEEGGCELRVKFSRSADAPAYQQGQNQLYNELNLGRREEYDVLDKRRGRDPEMGGKPRRKNPQEGLYNELQKDKMAEAYSEIGMKGERRRGKGHDGLYQGLSTATKDTYDALHMQALPPR

SEQ ID NO: 312 - protein, 498 aa, synthetic construct
MALPVTALLLPLALLLHAARPEVQLVESGGGMVQAGDSLRLSCVQSTYTVNSDVMGWFRQAPGKEREFVGAIMWNDGITYLQDSVKGRFTIFRDNAKNTVYLQMNSLKLEDTAVYYCAASKGRYSEYEYWGQGTQVTVSSGGGGSQVKLEESGGRLVQPRGSLRLSCAGSGRTFSTYGMAWFRQAPGKEREFVASKASMNYSGRTYYADSVKGRFTIARDNAKNMVFLQMNNLKPEDTAVYYCAAGTGCSTYGCFDAQIIDYWGKGTLVTVSSTSTTTPAPRPPTPAPTIASQPLSLRPEACRPAAGGAVHTRGLDFACDIYIWAPLAGTCGVLLLSLVITLYCKRGRKKLLYIFKQPFMRPVQTTQEEDGCSCRFPEEEEGGCELRVKFSRSADAPAYQQGQNQLYNELNLGRREEYDVLDKRRGRDPEMGGKPRRKNPQEGLYNELQKDKMAEAYSEIGMKGERRRGKGHDGLYQGLSTATKDTYDALHMQALPPR

SEQ ID NO: 313 - protein, 508 aa, synthetic construct
MALPVTALLLPLALLLHAARPEVQLVESGGGMVQAGDSLRLSCVQSTYTVNSDVMGWFRQAPGKEREFVGAIMWNDGITYLQDSVKGRFTIFRDNAKNTVYLQMNSLKLEDTAVYYCAASKGRYSEYEYWGQGTQVTVSSGGGGSGGGGSGGGGSQVKLEESGGRLVQPRGSLRLSCAGSGRTFSTYGMAWFRQAPGKEREFVASKASMNYSGRTYYADSVKGRFTIARDNAKNMVFLQMNNLKPEDTAVYYCAAGTGCSTYGCFDAQIIDYWGKGTLVTVSSTSTTTPAPRPPTPAPTIASQPLSLRPEACRPAAGGAVHTRGLDFACDIYIWAPLAGTCGVLLLSLVITLYCKRGRKKLLYIFKQPFMRPVQTTQEEDGCSCRFPEEEEGGCELRVKFSRSADAPAYQQGQNQLYNELNLGRREEYDVLDKRRGRDPEMGGKPRRKNPQEGLYNELQKDKMAEAYSEIGMKGERRRGKGHDGLYQGLSTATKDTYDALHMQALPPR

SEQ ID NO: 314 - protein, 518 aa, synthetic construct
MALPVTALLLPLALLLHAARPEVQLVESGGGMVQAGDSLRLSCVQSTYTVNSDVMGWFRQAPGKEREFVGAIMWNDGITYLQDSVKGRFTIFRDNAKNTVYLQMNSLKLEDTAVYYCAASKGRYSEYEYWGQGTQVTVSSGGGGSGGGGSGGGGSGGGGSGGGGSQVKLEESGGRLVQPRGSLRLSCAGSGRTFSTYGMAWFRQAPGKEREFVASKASMNYSGRTYYADSVKGRFTIARDNAKNMVFLQMNNLKPEDTAVYYCAAGTGCSTYGCFDAQIIDYWGKGTLVTVSSTSTTTPAPRPPTPAPTIASQPLSLRPEACRPAAGGAVHTRGLDFACDIYIWAPLAGTCGVLLLSLVITLYCKRGRKKLLYIFKQPFMRPVQTTQEEDGCSCRFPEEEEGGCELRVKFSRSADAPAYQQGQNQLYNELNLGRREEYDVLDKRRGRDPEMGGKPRRKNPQEGLYNELQKDKMAEAYSEIGMKGERRRGKGHDGLYQGLSTATKDTYDALHMQALPPR

SEQ ID NO: 315 - protein, 503 aa, synthetic construct
MALPVTALLLPLALLLHAARPEVQLVESGGGMVQAGDSLRLSCVQSTYTVNSDVMGWFRQAPGKEREFVGAIMWNDGITYLQDSVKGRFTIFRDNAKNTVYLQMNSLKLEDTAVYYCAASKGRYSEYEYWGQGTQVTVSSGGGGSGGGGSQVKLEESGGRLVQPRGSLRLSCAGSGRTFSTYGMAWFRQAPGKEREFVASKASMNYSGRTYYADSVKGRFTIARDNAKNMVFLQMNNLKPEDTAVYYCAAGTGCSTYGCFDAQIIDYWGKGTLVTVSSTSTTTPAPRPPTPAPTIASQPLSLRPEACRPAAGGAVHTRGLDFACDIYIWAPLAGTCGVLLLSLVITLYCKRGRKKLLYIFKQPFMRPVQTTQEEDGCSCRFPEEEEGGCELRVKFSRSADAPAYQQGQNQLYNELNLGRREEYDVLDKRRGRDPEMGGKPRRKNPQEGLYNELQKDKMAEAYSEIGMKGERRRGKGHDGLYQGLSTATKDTYDALHMQALPPR

SEQ ID NO: 316 - protein, 508 aa, synthetic construct; identical to SEQ ID NO: 313

SEQ ID NO: 317 - protein, 513 aa, synthetic construct
MALPVTALLLPLALLLHAARPEVQLVESGGGMVQAGDSLRLSCVQSTYTVNSDVMGWFRQAPGKEREFVGAIMWNDGITYLQDSVKGRFTIFRDNAKNTVYLQMNSLKLEDTAVYYCAASKGRYSEYEYWGQGTQVTVSSGGGGSGGGGSGGGGSGGGGSQVKLEESGGRLVQPRGSLRLSCAGSGRTFSTYGMAWFRQAPGKEREFVASKASMNYSGRTYYADSVKGRFTIARDNAKNMVFLQMNNLKPEDTAVYYCAAGTGCSTYGCFDAQIIDYWGKGTLVTVSSTSTTTPAPRPPTPAPTIASQPLSLRPEACRPAAGGAVHTRGLDFACDIYIWAPLAGTCGVLLLSLVITLYCKRGRKKLLYIFKQPFMRPVQTTQEEDGCSCRFPEEEEGGCELRVKFSRSADAPAYQQGQNQLYNELNLGRREEYDVLDKRRGRDPEMGGKPRRKNPQEGLYNELQKDKMAEAYSEIGMKGERRRGKGHDGLYQGLSTATKDTYDALHMQALPPR

SEQ ID NO: 318 - protein, 500 aa, synthetic construct
MALPVTALLLPLALLLHAARPQVKLEESGGRLVQPRGSLRLSCAGSGRTFSTYGMAWFRQAPGKEREFVASKASMNYSGRTYYADSVKGRFTIARDNAKNMVFLQMNNLKPEDTAVYYCAAGTGCSTYGCFDAQIIDYWGKGTLVTVSSGGGGSQVKLEESGGGLVQAGGSLRLSCAASGGTLSKNTVAWVRQAPGKERGFVTSITCDGRTTYYANSVNGRFPINRNNAENLVVLQMNSLKPDDTALYYCAAYRKSIMSIQPDYWGQGTQVTVSSTSTTTPAPRPPTPAPTIASQPLSLRPEACRPAAGGAVHTRGLDFACDIYIWAPLAGTCGVLLLSLVITLYCKRGRKKLLYIFKQPFMRPVQTTQEEDGCSCRFPEEEEGGCELRVKFSRSADAPAYQQGQNQLYNELNLGRREEYDVLDKRRGRDPEMGGKPRRKNPQEGLYNELQKDKMAEAYSEIGMKGERRRGKGHDGLYQGLSTATKDTYDALHMQALPPR

SEQ ID NO: 319 - protein, 510 aa, synthetic construct
MALPVTALLLPLALLLHAARPQVKLEESGGRLVQPRGSLRLSCAGSGRTFSTYGMAWFRQAPGKEREFVASKASMNYSGRTYYADSVKGRFTIARDNAKNMVFLQMNNLKPEDTAVYYCAAGTGCSTYGCFDAQIIDYWGKGTLVTVSSGGGGSGGGGSGGGGSQVKLEESGGGLVQAGGSLRLSCAASGGTLSKNTVAWVRQAPGKERGFVTSITCDGRTTYYANSVNGRFPINRNNAENLVVLQMNSLKPDDTALYYCAAYRKSIMSIQPDYWGQGTQVTVSSTSTTTPAPRPPTPAPTIASQPLSLRPEACRPAAGGAVHTRGLDFACDIYIWAPLAGTCGVLLLSLVITLYCKRGRKKLLYIFKQPFMRPVQTTQEEDGCSCRFPEEEEGGCELRVKFSRSADAPAYQQGQNQLYNELNLGRREEYDVLDKRRGRDPEMGGKPRRKNPQEGLYNELQKDKMAEAYSEIGMKGERRRGKGHDGLYQGLSTATKDTYDALHMQALPPR

SEQ ID NO: 320 - protein, 520 aa, synthetic construct
MALPVTALLLPLALLLHAARPQVKLEESGGRLVQPRGSLRLSCAGSGRTFSTYGMAWFRQAPGKEREFVASKASMNYSGRTYYADSVKGRFTIARDNAKNMVFLQMNNLKPEDTAVYYCAAGTGCSTYGCFDAQIIDYWGKGTLVTVSSGGGGSGGGGSGGGGSGGGGSGGGGSQVKLEESGGGLVQAGGSLRLSCAASGGTLSKNTVAWVRQAPGKERGFVTSITCDGRTTYYANSVNGRFPINRNNAENLVVLQMNSLKPDDTALYYCAAYRKSIMSIQPDYWGQGTQVTVSSTSTTTPAPRPPTPAPTIASQPLSLRPEACRPAAGGAVHTRGLDFACDIYIWAPLAGTCGVLLLSLVITLYCKRGRKKLLYIFKQPFMRPVQTTQEEDGCSCRFPEEEEGGCELRVKFSRSADAPAYQQGQNQLYNELNLGRREEYDVLDKRRGRDPEMGGKPRRKNPQEGLYNELQKDKMAEAYSEIGMKGERRRGKGHDGLYQGLSTATKDTYDALHMQALPPR

SEQ ID NO: 321 - protein, 505 aa, synthetic construct
MALPVTALLLPLALLLHAARPQVKLEESGGRLVQPRGSLRLSCAGSGRTFSTYGMAWFRQAPGKEREFVASKASMNYSGRTYYADSVKGRFTIARDNAKNMVFLQMNNLKPEDTAVYYCAAGTGCSTYGCFDAQIIDYWGKGTLVTVSSGGGGSGGGGSQVKLEESGGGLVQAGGSLRLSCAASGGTLSKNTVAWVRQAPGKERGFVTSITCDGRTTYYANSVNGRFPINRNNAENLVVLQMNSLKPDDTALYYCAAYRKSIMSIQPDYWGQGTQVTVSSTSTTTPAPRPPTPAPTIASQPLSLRPEACRPAAGGAVHTRGLDFACDIYIWAPLAGTCGVLLLSLVITLYCKRGRKKLLYIFKQPFMRPVQTTQEEDGCSCRFPEEEEGGCELRVKFSRSADAPAYQQGQNQLYNELNLGRREEYDVLDKRRGRDPEMGGKPRRKNPQEGLYNELQKDKMAEAYSEIGMKGERRRGKGHDGLYQGLSTATKDTYDALHMQALPPR

SEQ ID NO: 322 - protein, 510 aa, synthetic construct; identical to SEQ ID NO: 319

SEQ ID NO: 323 - protein, 515 aa, synthetic construct
MALPVTALLLPLALLLHAARPQVKLEESGGRLVQPRGSLRLSCAGSGRTFSTYGMAWFRQAPGKEREFVASKASMNYSGRTYYADSVKGRFTIARDNAKNMVFLQMNNLKPEDTAVYYCAAGTGCSTYGCFDAQIIDYWGKGTLVTVSSGGGGSGGGGSGGGGSGGGGSQVKLEESGGGLVQAGGSLRLSCAASGGTLSKNTVAWVRQAPGKERGFVTSITCDGRTTYYANSVNGRFPINRNNAENLVVLQMNSLKPDDTALYYCAAYRKSIMSIQPDYWGQGTQVTVSSTSTTTPAPRPPTPAPTIASQPLSLRPEACRPAAGGAVHTRGLDFACDIYIWAPLAGTCGVLLLSLVITLYCKRGRKKLLYIFKQPFMRPVQTTQEEDGCSCRFPEEEEGGCELRVKFSRSADAPAYQQGQNQLYNELNLGRREEYDVLDKRRGRDPEMGGKPRRKNPQEGLYNELQKDKMAEAYSEIGMKGERRRGKGHDGLYQGLSTATKDTYDALHMQALPPR

SEQ ID NO: 324 - protein, 492 aa, synthetic construct
MALPVTALLLPLALLLHAARPQVKLEESGGGLVQAGGSLRLSCAASGGTLSKNTVAWVRQAPGKERGFVTSITCDGRTTYYANSVNGRFPINRNNAENLVVLQMNSLKPDDTALYYCAAYRKSIMSIQPDYWGQGTQVTVSSGGGGSQVQLVESGGGLVQAGGSLRLSCAASGGTLSKNTVAWFRQAPGKERGFVASITWDGRTTYYADSVKGRFTISRDNAKNTVYLQMNSLKPEDTAVYVCADLGKWPAGPADYWGQGTQVTVSSTSTTTPAPRPPTPAPTIASQPLSLRPEACRPAAGGAVHTRGLDFACDIYIWAPLAGTCGVLLLSLVITLYCKRGRKKLLYIFKQPFMRPVQTTQEEDGCSCRFPEEEEGGCELRVKFSRSADAPAYQQGQNQLYNELNLGRREEYDVLDKRRGRDPEMGGKPRRKNPQEGLYNELQKDKMAEAYSEIGMKGERRRGKGHDGLYQGLSTATKDTYDALHMQALPPR

SEQ ID NO: 325 - protein, 502 aa, synthetic construct
MALPVTALLLPLALLLHAARPQVKLEESGGGLVQAGGSLRLSCAASGGTLSKNTVAWVRQAPGKERGFVTSITCDGRTTYYANSVNGRFPINRNNAENLVVLQMNSLKPDDTALYYCAAYRKSIMSIQPDYWGQGTQVTVSSGGGGSGGGGSGGGGSQVQLVESGGGLVQAGGSLRLSCAASGGTLSKNTVAWFRQAPGKERGFVASITWDGRTTYYADSVKGRFTISRDNAKNTVYLQMNSLKPEDTAVYVCADLGKWPAGPADYWGQGTQVTVSSTSTTTPAPRPPTPAPTIASQPLSLRPEACRPAAGGAVHTRGLDFACDIYIWAPLAGTCGVLLLSLVITLYCKRGRKKLLYIFKQPFMRPVQTTQEEDGCSCRFPEEEEGGCELRVKFSRSADAPAYQQGQNQLYNELNLGRREEYDVLDKRRGRDPEMGGKPRRKNPQEGLYNELQKDKMAEAYSEIGMKGERRRGKGHDGLYQGLSTATKDTYDALHMQALPPR

SEQ ID NO: 326 - protein, 512 aa, synthetic construct
MALPVTALLLPLALLLHAARPQVKLEESGGGLVQAGGSLRLSCAASGGTLSKNTVAWVRQAPGKERGFVTSITCDGRTTYYANSVNGRFPINRNNAENLVVLQMNSLKPDDTALYYCAAYRKSIMSIQPDYWGQGTQVTVSSGGGGSGGGGSGGGGSGGGGSGGGGSQVQLVESGGGLVQAGGSLRLSCAASGGTLSKNTVAWFRQAPGKERGFVASITWDGRTTYYADSVKGRFTISRDNAKNTVYLQMNSLKPEDTAVYVCADLGKWPAGPADYWGQGTQVTVSSTSTTTPAPRPPTPAPTIASQPLSLRPEACRPAAGGAVHTRGLDFACDIYIWAPLAGTCGVLLLSLVITLYCKRGRKKLLYIFKQPFMRPVQTTQEEDGCSCRFPEEEEGGCELRVKFSRSADAPAYQQGQNQLYNELNLGRREEYDVLDKRRGRDPEMGGKPRRKNPQEGLYNELQKDKMAEAYSEIGMKGERRRGKGHDGLYQGLSTATKDTYDALHMQALPPR

SEQ ID NO: 327 - protein, 497 aa, synthetic construct
MALPVTALLLPLALLLHAARPQVKLEESGGGLVQAGGSLRLSCAASGGTLSKNTVAWVRQAPGKERGFVTSITCDGRTTYYANSVNGRFPINRNNAENLVVLQMNSLKPDDTALYYCAAYRKSIMSIQPDYWGQGTQVTVSSGGGGSGGGGSQVQLVESGGGLVQAGGSLRLSCAASGGTLSKNTVAWFRQAPGKERGFVASITWDGRTTYYADSVKGRFTISRDNAKNTVYLQMNSLKPEDTAVYVCADLGKWPAGPADYWGQGTQVTVSSTSTTTPAPRPPTPAPTIASQPLSLRPEACRPAAGGAVHTRGLDFACDIYIWAPLAGTCGVLLLSLVITLYCKRGRKKLLYIFKQPFMRPVQTTQEEDGCSCRFPEEEEGGCELRVKFSRSADAPAYQQGQNQLYNELNLGRREEYDVLDKRRGRDPEMGGKPRRKNPQEGLYNELQKDKMAEAYSEIGMKGERRRGKGHDGLYQGLSTATKDTYDALHMQALPPR

SEQ ID NO: 328 - protein, 502 aa, synthetic construct; identical to SEQ ID NO: 325

SEQ ID NO: 329 - protein, 507 aa, synthetic construct
MALPVTALLLPLALLLHAARPQVKLEESGGGLVQAGGSLRLSCAASGGTLSKNTVAWVRQAPGKERGFVTSITCDGRTTYYANSVNGRFPINRNNAENLVVLQMNSLKPDDTALYYCAAYRKSIMSIQPDYWGQGTQVTVSSGGGGSGGGGSGGGGSGGGGSQVQLVESGGGLVQAGGSLRLSCAASGGTLSKNTVAWFRQAPGKERGFVASITWDGRTTYYADSVKGRFTISRDNAKNTVYLQMNSLKPEDTAVYVCADLGKWPAGPADYWGQGTQVTVSSTSTTTPAPRPPTPAPTIASQPLSLRPEACRPAAGGAVHTRGLDFACDIYIWAPLAGTCGVLLLSLVITLYCKRGRKKLLYIFKQPFMRPVQTTQEEDGCSCRFPEEEEGGCELRVKFSRSADAPAYQQGQNQLYNELNLGRREEYDVLDKRRGRDPEMGGKPRRKNPQEGLYNELQKDKMAEAYSEIGMKGERRRGKGHDGLYQGLSTATKDTYDALHMQALPPR

SEQ ID NO: 330 - protein, 491 aa, synthetic construct
MALPVTALLLPLALLLHAARPQVQLVESGGGLVQAGGSLRLSCAASGGTLSKNTVAWFRQAPGKERGFVASITWDGRTTYYADSVKGRFTISRDNAKNTVYLQMNSLKPEDTAVYVCADLGKWPAGPADYWGQGTQVTVSSGGGGSDVQLVESGGGLVQAGGSLRLSCAASGGTLSKNTVAWVRQAPGKERGFVTSITCDGRTTYYANSVKGRFPISRDNAENTVYLQMNSLKPEDTAGYVCADLGKWPAGSADYWGQGTHVTVSSTSTTTPAPRPPTPAPTIASQPLSLRPEACRPAAGGAVHTRGLDFACDIYIWAPLAGTCGVLLLSLVITLYCKRGRKKLLYIFKQPFMRPVQTTQEEDGCSCRFPEEEEGGCELRVKFSRSADAPAYQQGQNQLYNELNLGRREEYDVLDKRRGRDPEMGGKPRRKNPQEGLYNELQKDKMAEAYSEIGMKGERRRGKGHDGLYQGLSTATKDTYDALHMQALPPR

SEQ ID NO: 331 - protein, 501 aa, synthetic construct
MALPVTALLLPLALLLHAARPQVQLVESGGGLVQAGGSLRLSCAASGGTLSKNTVAWFRQAPGKERGFVASITWDGRTTYYADSVKGRFTISRDNAKNTVYLQMNSLKPEDTAVYVCADLGKWPAGPADYWGQGTQVTVSSGGGGSGGGGSGGGGSDVQLVESGGGLVQAGGSLRLSCAASGGTLSKNTVAWVRQAPGKERGFVTSITCDGRTTYYANSVKGRFPISRDNAENTVYLQMNSLKPEDTAGYVCADLGKWPAGSADYWGQGTHVTVSSTSTTTPAPRPPTPAPTIASQPLSLRPEACRPAAGGAVHTRGLDFACDIYIWAPLAGTCGVLLLSLVITLYCKRGRKKLLYIFKQPFMRPVQTTQEEDGCSCRFPEEEEGGCELRVKFSRSADAPAYQQGQNQLYNELNLGRREEYDVLDKRRGRDPEMGGKPRRKNPQEGLYNELQKDKMAEAYSEIGMKGERRRGKGHDGLYQGLSTATKDTYDALHMQALPPR

SEQ ID NO: 332 - protein, 511 aa, synthetic construct
MALPVTALLLPLALLLHAARPQVQLVESGGGLVQAGGSLRLSCAASGGTLSKNTVAWFRQAPGKERGFVASITWDGRTTYYADSVKGRFTISRDNAKNTVYLQMNSLKPEDTAVYVCADLGKWPAGPADYWGQGTQVTVSSGGGGSGGGGSGGGGSGGGGSGGGGSDVQLVESGGGLVQAGGSLRLSCAASGGTLSKNTVAWVRQAPGKERGFVTSITCDGRTTYYANSVKGRFPISRDNAENTVYLQMNSLKPEDTAGYVCADLGKWPAGSADYWGQGTHVTVSSTSTTTPAPRPPTPAPTIASQPLSLRPEACRPAAGGAVHTRGLDFACDIYIWAPLAGTCGVLLLSLVITLYCKRGRKKLLYIFKQPFMRPVQTTQEEDGCSCRFPEEEEGGCELRVKFSRSADAPAYQQGQNQLYNELNLGRREEYDVLDKRRGRDPEMGGKPRRKNPQEGLYNELQKDKMAEAYSEIGMKGERRRGKGHDGLYQGLSTATKDTYDALHMQALPPR

SEQ ID NO: 333 - protein, 496 aa, synthetic construct
MALPVTALLLPLALLLHAARPQVQLVESGGGLVQAGGSLRLSCAASGGTLSKNTVAWFRQAPGKERGFVASITWDGRTTYYADSVKGRFTISRDNAKNTVYLQMNSLKPEDTAVYVCADLGKWPAGPADYWGQGTQVTVSSGGGGSGGGGSDVQLVESGGGLVQAGGSLRLSCAASGGTLSKNTVAWVRQAPGKERGFVTSITCDGRTTYYANSVKGRFPISRDNAENTVYLQMNSLKPEDTAGYVCADLGKWPAGSADYWGQGTHVTVSSTSTTTPAPRPPTPAPTIASQPLSLRPEACRPAAGGAVHTRGLDFACDIYIWAPLAGTCGVLLLSLVITLYCKRGRKKLLYIFKQPFMRPVQTTQEEDGCSCRFPEEEEGGCELRVKFSRSADAPAYQQGQNQLYNELNLGRREEYDVLDKRRGRDPEMGGKPRRKNPQEGLYNELQKDKMAEAYSEIGMKGERRRGKGHDGLYQGLSTATKDTYDALHMQALPPR

SEQ ID NO: 334 - protein, 501 aa, synthetic construct; identical to SEQ ID NO: 331

SEQ ID NO: 335 - protein, 506 aa, synthetic construct
MALPVTALLLPLALLLHAARPQVQLVESGGGLVQAGGSLRLSCAASGGTLSKNTVAWFRQAPGKERGFVASITWDGRTTYYADSVKGRFTISRDNAKNTVYLQMNSLKPEDTAVYVCADLGKWPAGPADYWGQGTQVTVSSGGGGSGGGGSGGGGSGGGGSDVQLVESGGGLVQAGGSLRLSCAASGGTLSKNTVAWVRQAPGKERGFVTSITCDGRTTYYANSVKGRFPISRDNAENTVYLQMNSLKPEDTAGYVCADLGKWPAGSADYWGQGTHVTVSSTSTTTPAPRPPTPAPTIASQPLSLRPEACRPAAGGAVHTRGLDFACDIYIWAPLAGTCGVLLLSLVITLYCKRGRKKLLYIFKQPFMRPVQTTQEEDGCSCRFPEEEEGGCELRVKFSRSADAPAYQQGQNQLYNELNLGRREEYDVLDKRRGRDPEMGGKPRRKNPQEGLYNELQKDKMAEAYSEIGMKGERRRGKGHDGLYQGLSTATKDTYDALHMQALPPR

SEQ ID NO: 336 - DNA, 1488 bp, synthetic construct
  source 1..1488: mol_type = other DNA
atggctctgcccgtcactgctctgctgctgcccctggctctgctgctgcacgctgctcgccctcaggtccagctggtggaaagcggaggaggcctggtgcagccaggaggcagcctgaggctgtcctgcgaggcctctggcttcaccctggactactatgccatcggctggtttaggcaggcacctggaaaggagagggagggagtgatctgtatctctcgcagcgacggcagcacatactatgccgattccgtgaagggccggttcaccatcagcagagacaacgccaagaagacagtgtacctgcagatgatctccctgaagcctgaggataccgcagcatactattgcgcagcaggagcagactgtagcggatacctgagggattatgagtttaggggacagggaacccaggtgacagtgagctccggaggaggaggctcccaggtgcagctggtggagtctggaggcggcctggtgcagcctggaggcagcctgagactgagctgtgaagcttccggatttaccctggactactatgcaatcggatggtttaggcaggcaccaggaaaggagagagaaggcgtgatctgtatctccagatctgacggctctacatactatgccgatagtgtcaaaggacggttcaccatctctagagataatgccaagaagacagtctatctgcagatgattagcctgaagcccgaggacacagccgcctattactgcgcagcaggagcagattgtagtgggtatctgagggactatgagtttcgggggcaggggacacaggtgacagtgagttctactagtaccacgacgccagcgccgcgaccaccaacaccggcgcccaccatcgcgtcgcagcccctgtccctgcgcccagaggcgtgccggccagcggcggggggcgcagtgcacacgagggggctggacttcgcctgtgatatctacatctgggcgcccttggccgggacttgtggggtccttctcctgtcactggttatcaccctttactgcaaacggggcagaaagaaactcctgtatatattcaaacaaccatttatgagaccagtacaaactactcaagaggaagatggctgtagctgccgatttccagaagaagaagaaggaggatgtgaactgagagtgaagttcagcaggagcgcagacgcccccgcgtaccagcagggccagaaccagctctataacgagctcaatctaggacgaagagaggagtacgatgttttggacaagagacgtggccgggaccctgagatggggggaaagccgagaaggaagaaccctcaggaaggcctgtacaatgaactgcagaaagataagatggcggaggcctacagtgagattgggatgaaaggcgagcgccggaggggcaaggggcacgatggcctttaccagggtctcagtacagccaccaaggacacctacgacgcccttcacatgcaggccctgccccctcgctaa

SEQ ID NO: 337 - DNA, 1869 bp, synthetic construct
  source 1..1869: mol_type = other DNA
atggctctgcccgtcactgctctgctgctgcctctggccctgctgctgcacgccgcacgccctcaggtccagctggtcgagtcaggaggaggcctggtgcagccaggaggctccctgcggctgtcttgcgaggccagcggcttcaccctggactactatgccatcggctggtttaggcaggcacctggaaaggagagggagggagtgatctgtatctccagatctgacggctccacatactatgccgattctgtgaagggccggttcaccatctctagagacaacgccaagaagacagtgtacctgcagatgatcagcctgaagcccgaggataccgcagcatactattgcgcagcaggagcagactgttccggatacctgagggattatgagtttaggggacagggaacccaggtgacagtgagctccggaggaggaggctcccaggtgcagctggtggagtctggaggcggcctggtgcagcctggaggctccctgaggctgtcttgcgaggcaagcggcttcaccctggattactatgcaatcggatggtttaggcaggcaccaggaaaggagagagaaggcgtgatctgtatcagccgctccgacggcagtacctactatgccgattccgtcaaaggccggttcaccatctccagagacaatgccaagaagacagtctatctgcagatgatctctctgaagcctgaggatacagccgcctattactgtgccgcaggagcagactgtagtggctatctgagagattatgagtttcgcggccagggcacccaggtgacagtgtctagcggaggaggaggcagccaggtccagctggtggaatccggcggaggcctggtgcagcccggcggctccctgagactgtcctgtgaagcctccggatttactctggattattacgctattggatggttcagacaggcccctggcaaagaaagagaaggggtgatctgtatctctcggagcgacggctctacatactatgccgatagcgtcaagggaagatttaccatctccagagataatgccaagaagacagtgtatctgcagatgatttccctgaagcccgaggacactgccgcctattactgtgcagcaggagcagattgtagcgggtatctgcgggattatgaatttagaggacagggcactcaggtgacagtctcaagcactagtaccacgacgccagcgccgcgaccaccaacaccggcgcccaccatcgcgtcgcagcccctgtccctgcgcccagaggcgtgccggccagcggcggggggcgcagtgcacacgagggggctggacttcgcctgtgatatctacatctgggcgcccttggccgggacttgtggggtccttctcctgtcactggttatcaccctttactgcaaacggggcagaaagaaactcctgtatatattcaaacaaccatttatgagaccagtacaaactactcaagaggaagatggctgtagctgccgatttccagaagaagaagaaggaggatgtgaactgagagtgaagttcagcaggagcgcagacgcccccgcgtaccagcagggccagaaccagctctataacgagctcaatctaggacgaagagaggagtacgatgttttggacaagagacgtggccgggaccctgagatggggggaaagccgagaaggaagaaccctcaggaaggcctgtacaatgaactgcagaaagataagatggcggaggcctacagtgagattgggatgaaaggcgagcgccggaggggcaaggggcacgatggcctttaccagggtctcagtacagccaccaaggacacctacgacgcccttcacatgcaggccctgccccctcgctaa

SEQ ID NO: 338 - DNA, 1467 bp, synthetic construct
  source 1..1467: mol_type = other DNA
atggctctgcccgtcaccgctctgctgctgcctctggctctgctgctgcacgctgctcgccctcaggtcaaactggaagaatctggcggaggcctggtgcaggcaggacggagcctgcgcctgagctgcgcagcatccgagcacaccttcagctcccacgtgatgggctggtttcggcaggccccaggcaaggagagagagagcgtggccgtgatcggctggagggacatctccacatcttacgccgattccgtgaagggccggttcaccatcagccgggacaacgccaagaagacactgtatctgcagatgaacagcctgaagcccgaggacaccgccgtgtactattgcgcagcaaggagaatcgacgcagcagactttgattcctggggccagggcacccaggtgacagtgtctagcggaggaggaggatctgaggtgcagctggtggagagcggaggcggcctggtgcaggccggaggctctctgaggctgagctgtgcagcatccggaagaaccttcacaatgggctggtttaggcaggcaccaggaaaggagagggagttcgtggcagcaatcagcctgtcccctaccctggcctactatgccgagagcgtgaagggcaggtttaccatctcccgcgataacgccaagaatacagtggtgctgcagatgaactccctgaaacctgaggacacagccctgtactattgtgccgccgatcggaagagcgtgatgagcattagaccagactattgggggcagggaacacaggtgaccgtgagcagcactagtaccacgacgccagcgccgcgaccaccaacaccggcgcccaccatcgcgtcgcagcccctgtccctgcgcccagaggcgtgccggccagcggcggggggcgcagtgcacacgagggggctggacttcgcctgtgatatctacatctgggcgcccttggccgggacttgtggggtccttctcctgtcactggttatcaccctttactgcaaacggggcagaaagaaactcctgtatatattcaaacaaccatttatgagaccagtacaaactactcaagaggaagatggctgtagctgccgatttccagaagaagaagaaggaggatgtgaactgagagtgaagttcagcaggagcgcagacgcccccgcgtaccagcagggccagaaccagctctataacgagctcaatctaggacgaagagaggagtacgatgttttggacaagagacgtggccgggaccctgagatggggggaaagccgagaaggaagaaccctcaggaaggcctgtacaatgaactgcagaaagataagatggcggaggcctacagtgagattgggatgaaaggcgagcgccggaggggcaaggggcacgatggcctttaccagggtctcagtacagccaccaaggacacctacgacgcccttcacatgcaggccctgccccctcgctaa

SEQ ID NO: 339 - DNA, 1497 bp, synthetic construct
  source 1..1497: mol_type = other DNA
atggctctgcctgtcaccgctctgctgctgcctctggctctgctgctgcacgctgctcgccctcaggtcaaactggaagaaagtgggggaggcctggtgcaggcaggacggagcctgcgcctgagctgcgcagcatccgagcacaccttcagctcccacgtgatgggctggtttcggcaggccccaggcaaggagagagagtccgtggccgtgatcggctggagggacatctccacatcttacgccgattctgtgaagggccggttcaccatcagcagagacaacgccaagaagacactgtatctgcagatgaatagcctgaagcccgaggacaccgccgtgtactattgcgcagcaaggagaatcgacgcagcagactttgattcctggggccagggcacccaggtgacagtgtctagcggaggaggaggatctggaggaggaggaagcggaggaggaggatccgaggtgcagctggtggagtctggaggcggcctggtgcaggccggaggctctctgaggctgagctgtgcagcatccggaagaaccttcacaatgggctggtttaggcaggcaccaggaaaggagagggagttcgtggcagcaatcagcctgtcccctaccctggcctactatgccgagtccgtgaagggcaggtttaccatctctcgcgataacgccaagaatacagtggtgctgcagatgaacagcctgaaacctgaggacacagccctgtactattgtgccgccgatcggaagagcgtgatgagcattagacccgattattggggacagggcacacaggtgacagtgagtagcactagtaccacgacgccagcgccgcgaccaccaacaccggcgcccaccatcgcgtcgcagcccctgtccctgcgcccagaggcgtgccggccagcggcggggggcgcagtgcacacgagggggctggacttcgcctgtgatatctacatctgggcgcccttggccgggacttgtggggtccttctcctgtcactggttatcaccctttactgcaaacggggcagaaagaaactcctgtatatattcaaacaaccatttatgagaccagtacaaactactcaagaggaagatggctgtagctgccgatttccagaagaagaagaaggaggatgtgaactgagagtgaagttcagcaggagcgcagacgcccccgcgtaccagcagggccagaaccagctctataacgagctcaatctaggacgaagagaggagtacgatgttttggacaagagacgtggccgggaccctgagatggggggaaagccgagaaggaagaaccctcaggaaggcctgtacaatgaactgcagaaagataagatggcggaggcctacagtgagattgggatgaaaggcgagcgccggaggggcaaggggcacgatggcctttaccagggtctcagtacagccaccaaggacacctacgacgcccttcacatgcaggccctgccccctcgctaa

SEQ ID NO: 340 - DNA, 1527 bp, synthetic construct
  source 1..1527: mol_type = other DNA
atggctctgcccgtcaccgcactgctgctgcctctggctctgctgctgcacgccgcaagaccacaggtcaaactggaagaatcaggaggaggcctggtgcaggcaggacggagcctgcgcctgagctgcgcagcatccgagcacaccttcagctcccacgtgatgggctggtttcggcaggccccaggcaaggagagagagtccgtggccgtgatcggctggagggacatctccacatcttacgccgattccgtgaagggccggttcaccatcagccgggacaacgccaagaagacactgtatctgcagatgaacagcctgaagcccgaggacaccgccgtgtactattgcgcagcaaggagaatcgacgcagcagactttgatagctggggccagggcacccaggtgacagtgtctagcggaggaggaggatctggaggaggaggaagcggaggaggaggaagcggcggcggcggctctggcggcggcggcagcgaggtgcagctggtggagagcggcggcggcctggtgcaggccggcggctctctgaggctgagctgtgcagcatccggaagaaccttcacaatgggctggtttaggcaggcaccaggaaaggagagggagttcgtggcagcaatcagcctgtcccctaccctggcctactatgccgagagcgtgaagggcaggtttaccatctcccgcgataacgccaagaatacagtggtgttacaaatgaacagcctgaaacctgaggacacagccctgtactattgtgccgccgatcggaagagcgtgatgagcattagacccgattattgggggcaggggacacaggtgaccgtgagcagcactagtaccacgacgccagcgccgcgaccaccaacaccggcgcccaccatcgcgtcgcagcccctgtccctgcgcccagaggcgtgccggccagcggcggggggcgcagtgcacacgagggggctggacttcgcctgtgatatctacatctgggcgcccttggccgggacttgtggggtccttctcctgtcactggttatcaccctttactgcaaacggggcagaaagaaactcctgtatatattcaaacaaccatttatgagaccagtacaaactactcaagaggaagatggctgtagctgccgatttccagaagaagaagaaggaggatgtgaactgagagtgaagttcagcaggagcgcagacgcccccgcgtaccagcagggccagaaccagctctataacgagctcaatctaggacgaagagaggagtacgatgttttggacaagagacgtggccgggaccctgagatggggggaaagccgagaaggaagaaccctcaggaaggcctgtacaatgaactgcagaaagataagatggcggaggcctacagtgagattgggatgaaaggcgagcgccggaggggcaaggggcacgatggcctttaccagggtctcagtacagccaccaaggacacctacgacgcccttcacatgcaggccctgccccctcgctaa

SEQ ID NO: 341 - DNA, 1482 bp, synthetic construct
  source 1..1482: mol_type = other DNA
atggctctgcctgtgaccgcactgctgctgcctctggctctgctgctgcacgccgcacgacctgaagtccagctggtggaatccgggggaggcctggtgcaggcaggaggctccctgaggctgtcttgcgcagcaagcggaagaaccttcacaatgggctggtttaggcaggcaccaggaaaggagagggagttcgtggccgccatctccctgtctcctaccctggcctactatgccgagagcgtgaagggcaggtttaccatctcccgcgacaacgccaagaatacagtggtgctgcagatgaacagcctgaagccagaggacacagccctgtactattgcgccgccgatcggaagtctgtgatgagcatcagacccgattactggggccagggcacccaggtgacagtgagctccggaggaggaggatccggcggaggaggctctcaggtgaagctggaggagtccggaggcggcctggtgcaggccggacggtccctgagactgtcttgtgccgccagcgagcacaccttctctagccacgtgatgggatggttcaggcaggcacctggaaaggagagggagtccgtggcagtgatcggatggagggacatcagcacatcctacgccgattctgtgaagggccggttcaccatcagcagagacaacgccaagaagacactgtatttacaaatgaacagcctgaagcccgaggataccgccgtgtactattgtgccgcccggcggattgacgccgcagactttgactcatgggggcagggaactcaggtgaccgtgtcctcaactagtaccacgacgccagcgccgcgaccaccaacaccggcgcccaccatcgcgtcgcagcccctgtccctgcgcccagaggcgtgccggccagcggcggggggcgcagtgcacacgagggggctggacttcgcctgtgatatctacatctgggcgcccttggccgggacttgtggggtccttctcctgtcactggttatcaccctttactgcaaacggggcagaaagaaactcctgtatatattcaaacaaccatttatgagaccagtacaaactactcaagaggaagatggctgtagctgccgatttccagaagaagaagaaggaggatgtgaactgagagtgaagttcagcaggagcgcagacgcccccgcgtaccagcagggccagaaccagctctataacgagctcaatctaggacgaagagaggagtacgatgttttggacaagagacgtggccgggaccctgagatggggggaaagccgagaaggaagaaccctcaggaaggcctgtacaatgaactgcagaaagataagatggcggaggcctacagtgagattgggatgaaaggcgagcgccggaggggcaaggggcacgatggcctttaccagggtctcagtacagccaccaaggacacctacgacgcccttcacatgcaggccctgccccctcgctaa

SEQ ID NO: 342 - DNA, 1497 bp, synthetic construct
  source 1..1497: mol_type = other DNA
atggccctgcctgtcaccgctctgctgctgcccctggccctgctgctgcacgccgcacgccctgaggtccagctggtcgagtccgggggaggcctggtgcaggcaggaggctccctgaggctgtcttgcgcagcaagcggaagaaccttcacaatgggctggtttaggcaggcaccaggaaaggagagggagttcgtggccgccatctccctgtctcctaccctggcctactatgccgagtccgtgaagggcaggtttaccatctctcgcgacaacgccaagaatacagtggtgctgcagatgaactccctgaagccagaggacacagccctgtactattgcgccgccgatcggaagtctgtgatgagcatcagacccgattactggggccagggcacccaggtgacagtgagctccggaggaggaggatccggcggaggaggctctggcggcggcggcagccaggtgaagctggaggagagcggaggcggcctggtgcaggccggacggtccctgagactgtcttgtgccgccagcgagcacaccttctctagccacgtgatgggatggttcaggcaggcacctggaaaggagagggagtctgtggccgtgatcggctggagggacatcagcacatcctacgccgatagcgtgaagggccggttcaccatctccagagacaacgccaagaagacactgtatctgcagatgaatagcctgaagcccgaggataccgccgtgtactattgtgccgcccggcggattgacgccgcagattttgattcttgggggcagggaactcaggtgaccgtgtcctcaactagtaccacgacgccagcgccgcgaccaccaacaccggcgcccaccatcgcgtcgcagcccctgtccctgcgcccagaggcgtgccggccagcggcggggggcgcagtgcacacgagggggctggacttcgcctgtgatatctacatctgggcgcccttggccgggacttgtggggtccttctcctgtcactggttatcaccctttactgcaaacggggcagaaagaaactcctgtatatattcaaacaaccatttatgagaccagtacaaactactcaagaggaagatggctgtagctgccgatttccagaagaagaagaaggaggatgtgaactgagagtgaagttcagcaggagcgcagacgcccccgcgtaccagcagggccagaaccagctctataacgagctcaatctaggacgaagagaggagtacgatgttttggacaagagacgtggccgggaccctgagatggggggaaagccgagaaggaagaaccctcaggaaggcctgtacaatgaactgcagaaagataagatggcggaggcctacagtgagattgggatgaaaggcgagcgccggaggggcaaggggcacgatggcctttaccagggtctcagtacagccaccaaggacacctacgacgcccttcacatgcaggccctgccccctcgctaa

SEQ ID NO: 343 - DNA, 1512 bp, synthetic construct
  source 1..1512: mol_type = other DNA
atggctctgcctgtgaccgccctgctgctgcccctggccctgctgctgcacgccgcacgacctgaagtccagctggtggaatctggcggaggcctggtgcaggcaggaggctccctgaggctgtcttgcgcagcaagcggaagaaccttcacaatgggctggtttaggcaggcaccaggaaaggagagggagttcgtggccgccatctccctgtctcctaccctggcctactatgccgagtctgtgaagggcaggtttaccatcagccgcgacaacgccaagaatacagtggtgctgcagatgaacagcctgaagccagaggacacagccctgtactattgcgccgccgatcggaagtctgtgatgagcatcagacccgattactggggccagggcacccaggtgacagtgagctccggaggaggaggatccggcggaggaggctctggcggcggcggctccggcggcggcggctcccaggtgaagctggaggagtccggaggcggcctggtgcaggccggacggtccctgagactgtcttgtgccgccagcgagcacaccttctctagccacgtgatgggatggttcaggcaggcacctggaaaggagagggagagcgtggcagtgatcggatggagggacatcagcacatcctacgccgattccgtgaagggccggttcaccatcagccgggacaacgccaagaagacactgtatttacaaatgaacagcctgaagcccgaggataccgccgtgtactattgtgccgcccggcggattgatgccgcagactttgatagttggggacaggggactcaggtcaccgtcagcagcactagtaccacgacgccagcgccgcgaccaccaacaccggcgcccaccatcgcgtcgcagcccctgtccctgcgcccagaggcgtgccggccagcggcggggggcgcagtgcacacgagggggctggacttcgcctgtgatatctacatctgggcgcccttggccgggacttgtggggtccttctcctgtcactggttatcaccctttactgcaaacggggcagaaagaaactcctgtatatattcaaacaaccatttatgagaccagtacaaactactcaagaggaagatggctgtagctgccgatttccagaagaagaagaaggaggatgtgaactgagagtgaagttcagcaggagcgcagacgcccccgcgtaccagcagggccagaaccagctctataacgagctcaatctaggacgaagagaggagtacgatgttttggacaagagacgtggccgggaccctgagatggggggaaagccgagaaggaagaaccctcaggaaggcctgtacaatgaactgcagaaagataagatggcggaggcctacagtgagattgggatgaaaggcgagcgccggaggggcaaggggcacgatggcctttaccagggtctcagtacagccaccaaggacacctacgacgcccttcacatgcaggccctgccccctcgctaa

SEQ ID NO: 344 - DNA, 1470 bp, synthetic construct
  source 1..1470: mol_type = other DNA
atggctctgcccgtcaccgcactgctgctgcctctggctctgctgctgcacgctgctcgccctcaggtcaaactggaagaatctggcggaggcctggtgcaggcaggcaggtccctgaggctgtcttgcgcagcaagcgagcacacctttagctcccacgtgatgggatggttcaggcaggcaccaggcaaggagagagagtccgtggccgtgatcggctggagggacatctccacatcttacgccgattctgtgaagggccggtttaccatcagcagagacaacgccaagaagacactgtatctgcagatgaatagcctgaagcctgaggacaccgccgtgtactattgcgcagcaaggagaatcgatgcagcagacttcgattcctggggacagggaacccaggtgacagtgtctagcggaggaggaggaagcgccgtgcagctggtggagtccggcggcggcctggtgcaggccggcgattctctgcggctgacctgtacagcctccggcagagccttctctacctactttatggcctggtttagacaggcccctggcaaggagagggagtttgtggcaggaatcgcatggagcggaggatccacagcatacgccgactccgtgaagggcaggttcaccatctctcgcgataacgccaagaatacagtgtatctgcagatgaactctctgaagagcgaggacacagccgtgtactattgtgccagccggggaatcgaggtggaggaatttggggcttgggggcagggaactcaggtgaccgtctcatcaactagtaccacgacgccagcgccgcgaccaccaacaccggcgcccaccatcgcgtcgcagcccctgtccctgcgcccagaggcgtgccggccagcggcggggggcgcagtgcacacgagggggctggacttcgcctgtgatatctacatctgggcgcccttggccgggacttgtggggtccttctcctgtcactggttatcaccctttactgcaaacggggcagaaagaaactcctgtatatattcaaacaaccatttatgagaccagtacaaactactcaagaggaagatggctgtagctgccgatttccagaagaagaagaaggaggatgtgaactgagagtgaagttcagcaggagcgcagacgcccccgcgtaccagcagggccagaaccagctctataacgagctcaatctaggacgaagagaggagtacgatgttttggacaagagacgtggccgggaccctgagatggggggaaagccgagaaggaagaaccctcaggaaggcctgtacaatgaactgcagaaagataagatggcggaggcctacagtgagattgggatgaaaggcgagcgccggaggggcaaggggcacgatggcctttaccagggtctcagtacagccaccaaggacacctacgacgcccttcacatgcaggccctgccccctcgctaa

SEQ ID NO: 345 - DNA, 1500 bp, synthetic construct
  source 1..1500: mol_type = other DNA
atggctctgcccgtcaccgctctgctgctgcctctggctctgctgctgcacgctgctcgccctcaggtcaaactggaagaatctggcggaggcctggtgcaggcaggcaggtccctgaggctgtcttgcgcagcaagcgagcacacctttagctcccacgtgatgggatggttcaggcaggcaccaggcaaggagagagagagcgtggccgtgatcggctggagggacatctccacatcttacgccgatagcgtgaagggccggtttaccatctccagagacaacgccaagaagacactgtatctgcagatgaatagcctgaagcctgaggacaccgccgtgtactattgcgcagcaaggagaatcgatgcagcagacttcgattcctggggacagggaacccaggtgacagtgtctagcggaggaggaggatccggaggaggaggatctggcggcggcggcagcgccgtgcagctggtggagtccggcggcggcctggtgcaggccggcgactctctgaggctgacctgtacagcctccggcagagccttctctacctactttatggcctggtttagacaggcccctggcaaggagagggagtttgtggcaggaatcgcatggagcggaggatccacagcatacgcagactctgtgaagggcaggttcaccatcagccgcgataacgccaagaatacagtgtatctgcagatgaactctctgaagagcgaggatacagccgtgtactattgtgcctcccgggggattgaagtcgaggaatttggggcttgggggcagggcactcaggtcaccgtctcatctactagtaccacgacgccagcgccgcgaccaccaacaccggcgcccaccatcgcgtcgcagcccctgtccctgcgcccagaggcgtgccggccagcggcggggggcgcagtgcacacgagggggctggacttcgcctgtgatatctacatctgggcgcccttggccgggacttgtggggtccttctcctgtcactggttatcaccctttactgcaaacggggcagaaagaaactcctgtatatattcaaacaaccatttatgagaccagtacaaactactcaagaggaagatggctgtagctgccgatttccagaagaagaagaaggaggatgtgaactgagagtgaagttcagcaggagcgcagacgcccccgcgtaccagcagggccagaaccagctctataacgagctcaatctaggacgaagagaggagtacgatgttttggacaagagacgtggccgggaccctgagatggggggaaagccgagaaggaagaaccctcaggaaggcctgtacaatgaactgcagaaagataagatggcggaggcctacagtgagattgggatgaaaggcgagcgccggaggggcaaggggcacgatggcctttaccagggtctcagtacagccaccaaggacacctacgacgcccttcacatgcaggccctgccccctcgctaa

SEQ ID NO: 346 - DNA, 1530 bp, synthetic construct
  source 1..1530: mol_type = other DNA
atggctctgcccgtcactgctctgctgctgcctctggctctgctgctgcacgctgctagaccacaggtcaaactggaggagtcagggggaggcctggtgcaggcaggcaggtccctgaggctgtcttgcgcagcaagcgagcacacctttagctcccacgtgatgggatggttcaggcaggcaccaggcaaggagagagagagcgtggccgtgatcggctggagggacatctccacatcttacgccgattctgtgaagggccggtttaccatcagcagagacaacgccaagaagacactgtatctgcagatgaacagcctgaagcctgaggacaccgccgtgtactattgcgcagcaaggagaatcgatgcagcagacttcgattcctggggacagggaacccaggtgacagtgtctagcggaggaggaggatccggaggaggaggatctggcggcggcggcagtggcggcggcggctccggcggcggcggctctgccgtgcagctggtggagtccggcggcggcctggtgcaggccggcgactccctgaggctgacctgtacagccagcggcagagccttctccacctactttatggcctggtttagacaggcccctggcaaggagagggagtttgtggcaggaatcgcatggagcggaggatccacagcatacgccgactccgtgaagggcaggttcaccatctctcgcgataacgccaagaatacagtgtatctgcagatgaactctctgaagagcgaggatacagccgtgtactattgtgcctcccggggcattgaagtggaagaatttggggcttggggacaggggactcaggtcaccgtcagcagcactagtaccacgacgccagcgccgcgaccaccaacaccggcgcccaccatcgcgtcgcagcccctgtccctgcgcccagaggcgtgccggccagcggcggggggcgcagtgcacacgagggggctggacttcgcctgtgatatctacatctgggcgcccttggccgggacttgtggggtccttctcctgtcactggttatcaccctttactgcaaacggggcagaaagaaactcctgtatatattcaaacaaccatttatgagaccagtacaaactactcaagaggaagatggctgtagctgccgatttccagaagaagaagaaggaggatgtgaactgagagtgaagttcagcaggagcgcagacgcccccgcgtaccagcagggccagaaccagctctataacgagctcaatctaggacgaagagaggagtacgatgttttggacaagagacgtggccgggaccctgagatggggggaaagccgagaaggaagaaccctcaggaaggcctgtacaatgaactgcagaaagataagatggcggaggcctacagtgagattgggatgaaaggcgagcgccggaggggcaaggggcacgatggcctttaccagggtctcagtacagccaccaaggacacctacgacgcccttcacatgcaggccctgccccctcgctaa

SEQ ID NO: 347 - DNA, 1485 bp, synthetic construct
  source 1..1485: mol_type = other DNA
atggctctgcccgtgaccgctctgctgctgcctctggctctgctgctgcatgctgctcgccctcaggtgaaactggaagaatctggcggaggcctggtgcaggcaggcaggtccctgaggctgtcttgcgcagcaagcgagcacacctttagctcccacgtgatgggatggttcaggcaggcaccaggcaaggagagagagtccgtggccgtgatcggctggagggacatctccacatcttacgccgattctgtgaagggccggtttaccatcagcagagacaacgccaagaagacactgtatctgcagatgaacagcctgaagcctgaggacaccgccgtgtactattgcgcagcaaggagaatcgatgcagcagacttcgatagctggggacagggaacccaggtgacagtgtctagcggaggaggaggatccggaggaggaggatctgccgtgcagctggtggagagcggcggcggcctggtgcaggccggcgattccctgaggctgacctgtacagccagcggcagagccttctccacctactttatggcctggtttagacaggcccctggcaaggagagggagtttgtggcaggaatcgcatggagcggaggatccacagcatacgccgactccgtgaagggcaggttcaccatctctcgcgataacgccaagaatacagtgtatctgcagatgaactctctgaagagcgaggacacagccgtgtactattgtgccagccgggggattgaagtggaagaatttggggcttgggggcaggggactcaggtcacagtgtcatctactagtaccacgacgccagcgccgcgaccaccaacaccggcgcccaccatcgcgtcgcagcccctgtccctgcgcccagaggcgtgccggccagcggcggggggcgcagtgcacacgagggggctggacttcgcctgtgatatctacatctgggcgcccttggccgggacttgtggggtccttctcctgtcactggttatcaccctttactgcaaacggggcagaaagaaactcctgtatatattcaaacaaccatttatgagaccagtacaaactactcaagaggaagatggctgtagctgccgatttccagaagaagaagaaggaggatgtgaactgagagtgaagttcagcaggagcgcagacgcccccgcgtaccagcagggccagaaccagctctataacgagctcaatctaggacgaagagaggagtacgatgttttggacaagagacgtggccgggaccctgagatggggggaaagccgagaaggaagaaccctcaggaaggcctgtacaatgaactgcagaaagataagatggcggaggcctacagtgagattgggatgaaaggcgagcgccggaggggcaaggggcacgatggcctttaccagggtctcagtacagccaccaaggacacctacgacgcccttcacatgcaggccctgccccctcgctaa

SEQ ID NO: 348 - DNA, 1500 bp, synthetic construct
  source 1..1500: mol_type = other DNA
atggctctgcccgtcaccgcactgctgctgcccctggctctgctgctgcacgctgctcgccctcaggtcaaactggaagaatctggaggaggcctggtgcaggcaggcaggtccctgaggctgtcttgcgcagcaagcgagcacacctttagctcccacgtgatgggatggttcaggcaggcaccaggcaaggagagagagagcgtggccgtgatcggctggagggacatctccacatcttacgccgatagcgtgaagggccggtttaccatctccagagacaacgccaagaagacactgtatctgcagatgaatagcctgaagcctgaggacaccgccgtgtactattgcgcagcaaggagaatcgatgcagcagacttcgattcctggggacagggaacccaggtgacagtgtctagcggaggaggaggatccggaggaggaggatctggcggcggcggcagcgccgtgcagctggtggagtccggcggcggcctggtgcaggccggcgactctctgaggctgacctgtacagcctccggcagagccttctctacctactttatggcctggtttagacaggcccctggcaaggagagggagtttgtggcaggaatcgcatggagcggaggatccacagcatacgcagactctgtgaagggcaggttcaccatcagccgcgataacgccaagaatacagtgtatctgcagatgaactctctgaagagcgaggatacagccgtgtactattgtgcctcccgggggattgaagtggaagaatttggggcttgggggcaggggactcaggtcaccgtcagcagcactagtaccacgacgccagcgccgcgaccaccaacaccggcgcccaccatcgcgtcgcagcccctgtccctgcgcccagaggcgtgccggccagcggcggggggcgcagtgcacacgagggggctggacttcgcctgtgatatctacatctgggcgcccttggccgggacttgtggggtccttctcctgtcactggttatcaccctttactgcaaacggggcagaaagaaactcctgtatatattcaaacaaccatttatgagaccagtacaaactactcaagaggaagatggctgtagctgccgatttccagaagaagaagaaggaggatgtgaactgagagtgaagttcagcaggagcgcagacgcccccgcgtaccagcagggccagaaccagctctataacgagctcaatctaggacgaagagaggagtacgatgttttggacaagagacgtggccgggaccctgagatggggggaaagccgagaaggaagaaccctcaggaaggcctgtacaatgaactgcagaaagataagatggcggaggcctacagtgagattgggatgaaaggcgagcgccggaggggcaaggggcacgatggcctttaccagggtctcagtacagccaccaaggacacctacgacgcccttcacatgcaggccctgccccctcgctaa

SEQ ID NO: 349 - DNA, 1515 bp, synthetic construct
  source 1..1515: mol_type = other DNA
atggctctgcctgtgaccgctctgctgctgcctctggctctgctgctgcacgccgctcgccctcaggtgaaactggaagaatctggaggaggcctggtgcaggcaggcaggtccctgaggctgtcttgcgcagcaagcgagcacacctttagctcccacgtgatgggatggttcaggcaggcaccaggcaaggagagagagtccgtggccgtgatcggctggagggacatctccacatcttacgccgattccgtgaagggccggtttaccatcagccgggacaacgccaagaagacactgtatctgcagatgaacagcctgaagcctgaggacaccgccgtgtactattgcgcagcaaggagaatcgatgcagcagacttcgattcttggggccagggcacccaggtgacagtgtctagcggaggaggaggatccggaggaggaggatctggcggcggcggctccggcggcggcggctccgccgtgcagctggtggagtctggcggcggcctggtgcaggccggcgacagcctgaggctgacctgtacagcctctggcagagccttcagcacctactttatggcctggtttagacaggcccctggcaaggagagggagtttgtggcaggaatcgcatggagcggaggatccacagcatacgccgacagcgtgaagggcaggttcaccatctcccgcgataacgccaagaatacagtgtatctgcagatgaactctctgaagagcgaggatacagccgtgtactattgtgccagccgggggattgaagtggaagaatttggggcatgggggcaggggactcaggtcaccgtcagtagcactagtaccacgacgccagcgccgcgaccaccaacaccggcgcccaccatcgcgtcgcagcccctgtccctgcgcccagaggcgtgccggccagcggcggggggcgcagtgcacacgagggggctggacttcgcctgtgatatctacatctgggcgcccttggccgggacttgtggggtccttctcctgtcactggttatcaccctttactgcaaacggggcagaaagaaactcctgtatatattcaaacaaccatttatgagaccagtacaaactactcaagaggaagatggctgtagctgccgatttccagaagaagaagaaggaggatgtgaactgagagtgaagttcagcaggagcgcagacgcccccgcgtaccagcagggccagaaccagctctataacgagctcaatctaggacgaagagaggagtacgatgttttggacaagagacgtggccgggaccctgagatggggggaaagccgagaaggaagaaccctcaggaaggcctgtacaatgaactgcagaaagataagatggcggaggcctacagtgagattgggatgaaaggcgagcgccggaggggcaaggggcacgatggcctttaccagggtctcagtacagccaccaaggacacctacgacgcccttcacatgcaggccctgccccctcgctaa

SEQ ID NO: 350 - DNA, 1470 bp, synthetic construct
  source 1..1470: mol_type = other DNA
atggctctgcccgtcaccgctctgctgctgcctctggctctgctgctgcacgctgctcgccctgaggtgcagctggtggagtctgggggaggaatggtgcaggctggggactctctgagactatcctgtgtgcagtctacttacaccgtcaatagcgatgtcatgggctggttccgccaggctccagggaaggagcgtgagtttgtaggagcgattatgtggaatgatggtattacatacttgcaagactccgtgaagggccgatttaccatcttcagagacaacgccaagaacacggtgtatctgcaaatgaacagcctgaaacttgaggatacggccgtttattactgtgcagcatccaagggtagatactcggaatatgagtactggggccaggggacccaggtcaccgtctcctcaggaggaggaggatctgcggtgcagctggtggagtctgggggaggattggtgcaggctggggactctctgagactcacctgtacagcctctggacgcgccttcagtacctatttcatggcctggttccgccaggctccagggaaggagcgtgagtttgtagcaggaattgcatggagtggtggtagcacggcgtatgcagactccgtgaagggccgattcaccatctccagagacaacgccaagaacacggtgtatctgcaaatgaacagcctgaaatctgaggacacggccgtttattactgtgccagcagggggattgaggtcgaagagtttggtgcctggggccaggggacccaggtcaccgtctcgtcgactagtaccacgacgccagcgccgcgaccaccaacaccggcgcccaccatcgcgtcgcagcccctgtccctgcgcccagaggcgtgccggccagcggcggggggcgcagtgcacacgagggggctggacttcgcctgtgatatctacatctgggcgcccttggccgggacttgtggggtccttctcctgtcactggttatcaccctttactgcaaacggggcagaaagaaactcctgtatatattcaaacaaccatttatgagaccagtacaaactactcaagaggaagatggctgtagctgccgatttccagaagaagaagaaggaggatgtgaactgagagtgaagttcagcaggagcgcagacgcccccgcgtaccagcagggccagaaccagctctataacgagctcaatctaggacgaagagaggagtacgatgttttggacaagagacgtggccgggaccctgagatggggggaaagccgagaaggaagaaccctcaggaaggcctgtacaatgaactgcagaaagataagatggcggaggcctacagtgagattgggatgaaaggcgagcgccggaggggcaaggggcacgatggcctttaccagggtctcagtacagccaccaaggacacctacgacgcccttcacatgcaggccctgccccctcgctaa

SEQ ID NO: 351 - DNA, 1500 bp, synthetic construct
  source 1..1500: mol_type = other DNA
atggctctgcccgtcaccgctctgctgctgcctctggctctgctgctgcacgctgctcgccctgaggtgcagctggtggagtctgggggaggaatggtgcaggctggggactctctgagactatcctgtgtgcagtctacttacaccgtcaatagcgatgtcatgggctggttccgccaggctccagggaaggagcgtgagtttgtaggagcgattatgtggaatgatggtattacatacttgcaagactccgtgaagggccgatttaccatcttcagagacaacgccaagaacacggtgtatctgcaaatgaacagcctgaaacttgaggatacggccgtttattactgtgcagcatccaagggtagatactcggaatatgagtactggggccaggggacccaggtcaccgtctcctcaggaggaggaggatctggaggaggaggaagcggaggaggaggatccgcggtgcagctggtggagtctgggggaggattggtgcaggctggggactctctgagactcacctgtacagcctctggacgcgccttcagtacctatttcatggcctggttccgccaggctccagggaaggagcgtgagtttgtagcaggaattgcatggagtggtggtagcacggcgtatgcagactccgtgaagggccgattcaccatctccagagacaacgccaagaacacggtgtatctgcaaatgaacagcctgaaatctgaggacacggccgtttattactgtgccagcagggggattgaggtcgaagagtttggtgcctggggccaggggacccaggtcaccgtctcgtcgactagtaccacgacgccagcgccgcgaccaccaacaccggcgcccaccatcgcgtcgcagcccctgtccctgcgcccagaggcgtgccggccagcggcggggggcgcagtgcacacgagggggctggacttcgcctgtgatatctacatctgggcgcccttggccgggacttgtggggtccttctcctgtcactggttatcaccctttactgcaaacggggcagaaagaaactcctgtatatattcaaacaaccatttatgagaccagtacaaactactcaagaggaagatggctgtagctgccgatttccagaagaagaagaaggaggatgtgaactgagagtgaagttcagcaggagcgcagacgcccccgcgtaccagcagggccagaaccagctctataacgagctcaatctaggacgaagagaggagtacgatgttttggacaagagacgtggccgggaccctgagatggggggaaagccgagaaggaagaaccctcaggaaggcctgtacaatgaactgcagaaagataagatggcggaggcctacagtgagattgggatgaaaggcgagcgccggaggggcaaggggcacgatggcctttaccagggtctcagtacagccaccaaggacacctacgacgcccttcacatgcaggccctgccccctcgctaa

SEQ ID NO: 352 - DNA, 1530 bp, synthetic construct
  source 1..1530: mol_type = other DNA
atggctctgcccgtcaccgctctgctgctgcctctggctctgctgctgcacgctgctcgccctgaggtgcagctggtggagtctgggggaggaatggtgcaggctggggactctctgagactatcctgtgtgcagtctacttacaccgtcaatagcgatgtcatgggctggttccgccaggctccagggaaggagcgtgagtttgtaggagcgattatgtggaatgatggtattacatacttgcaagactccgtgaagggccgatttaccatcttcagagacaacgccaagaacacggtgtatctgcaaatgaacagcctgaaacttgaggatacggccgtttattactgtgcagcatccaagggtagatactcggaatatgagtactggggccaggggacccaggtcaccgtctcctcaggaggaggaggatctggaggaggaggaagcggaggaggaggaagcggcggcggcggctctggcggcggcggcagcgcggtgcagctggtggagtctgggggaggattggtgcaggctggggactctctgagactcacctgtacagcctctggacgcgccttcagtacctatttcatggcctggttccgccaggctccagggaaggagcgtgagtttgtagcaggaattgcatggagtggtggtagcacggcgtatgcagactccgtgaagggccgattcaccatctccagagacaacgccaagaacacggtgtatctgcaaatgaacagcctgaaatctgaggacacggccgtttattactgtgccagcagggggattgaggtcgaagagtttggtgcctggggccaggggacccaggtcaccgtctcgtcgactagtaccacgacgccagcgccgcgaccaccaacaccggcgcccaccatcgcgtcgcagcccctgtccctgcgcccagaggcgtgccggccagcggcggggggcgcagtgcacacgagggggctggacttcgcctgtgatatctacatctgggcgcccttggccgggacttgtggggtccttctcctgtcactggttatcaccctttactgcaaacggggcagaaagaaactcctgtatatattcaaacaaccatttatgagaccagtacaaactactcaagaggaagatggctgtagctgccgatttccagaagaagaagaaggaggatgtgaactgagagtgaagttcagcaggagcgcagacgcccccgcgtaccagcagggccagaaccagctctataacgagctcaatctaggacgaagagaggagtacgatgttttggacaagagacgtggccgggaccctgagatggggggaaagccgagaaggaagaaccctcaggaaggcctgtacaatgaactgcagaaagataagatggcggaggcctacagtgagattgggatgaaaggcgagcgccggaggggcaaggggcacgatggcctttaccagggtctcagtacagccaccaaggacacctacgacgcccttcacatgcaggccctgccccctcgctaa

SEQ ID NO: 353 - DNA, 1485 bp, synthetic construct
  source 1..1485: mol_type = other DNA
atggctctgcccgtcaccgctctgctgctgcctctggctctgctgctgcacgctgctcgccctgaggtgcagctggtggagtctgggggaggaatggtgcaggctggggactctctgagactatcctgtgtgcagtctacttacaccgtcaatagcgatgtcatgggctggttccgccaggctccagggaaggagcgtgagtttgtaggagcgattatgtggaatgatggtattacatacttgcaagactccgtgaagggccgatttaccatcttcagagacaacgccaagaacacggtgtatctgcaaatgaacagcctgaaacttgaggatacggccgtttattactgtgcagcatccaagggtagatactcggaatatgagtactggggccaggggacccaggtcaccgtctcctcaggaggaggaggatccggcggaggaggctctgcggtgcagctggtggagtctgggggaggattggtgcaggctggggactctctgagactcacctgtacagcctctggacgcgccttcagtacctatttcatggcctggttccgccaggctccagggaaggagcgtgagtttgtagcaggaattgcatggagtggtggtagcacggcgtatgcagactccgtgaagggccgattcaccatctccagagacaacgccaagaacacggtgtatctgcaaatgaacagcctgaaatctgaggacacggccgtttattactgtgccagcagggggattgaggtcgaagagtttggtgcctggggccaggggacccaggtcaccgtctcgtcgactagtaccacgacgccagcgccgcgaccaccaacaccggcgcccaccatcgcgtcgcagcccctgtccctgcgcccagaggcgtgccggccagcggcggggggcgcagtgcacacgagggggctggacttcgcctgtgatatctacatctgggcgcccttggccgggacttgtggggtccttctcctgtcactggttatcaccctttactgcaaacggggcagaaagaaactcctgtatatattcaaacaaccatttatgagaccagtacaaactactcaagaggaagatggctgtagctgccgatttccagaagaagaagaaggaggatgtgaactgagagtgaagttcagcaggagcgcagacgcccccgcgtaccagcagggccagaaccagctctataacgagctcaatctaggacgaagagaggagtacgatgttttggacaagagacgtggccgggaccctgagatggggggaaagccgagaaggaagaaccctcaggaaggcctgtacaatgaactgcagaaagataagatggcggaggcctacagtgagattgggatgaaaggcgagcgccggaggggcaaggggcacgatggcctttaccagggtctcagtacagccaccaaggacacctacgacgcccttcacatgcaggccctgccccctcgctaa

SEQ ID NO: 354 - DNA, 1500 bp, synthetic construct
  source 1..1500: mol_type = other DNA
atggctctgcccgtcaccgctctgctgctgcctctggctctgctgctgcacgctgctcgccctgaggtgcagctggtggagtctgggggaggaatggtgcaggctggggactctctgagactatcctgtgtgcagtctacttacaccgtcaatagcgatgtcatgggctggttccgccaggctccagggaaggagcgtgagtttgtaggagcgattatgtggaatgatggtattacatacttgcaagactccgtgaagggccgatttaccatcttcagagacaacgccaagaacacggtgtatctgcaaatgaacagcctgaaacttgaggatacggccgtttattactgtgcagcatccaagggtagatactcggaatatgagtactggggccaggggacccaggtcaccgtctcctcaggaggaggaggatccggcggaggaggctctggcggcggcggcagcgcggtgcagctggtggagtctgggggaggattggtgcaggctggggactctctgagactcacctgtacagcctctggacgcgccttcagtacctatttcatggcctggttccgccaggctccagggaaggagcgtgagtttgtagcaggaattgcatggagtggtggtagcacggcgtatgcagactccgtgaagggccgattcaccatctccagagacaacgccaagaacacggtgtatctgcaaatgaacagcctgaaatctgaggacacggccgtttattactgtgccagcagggggattgaggtcgaagagtttggtgcctggggccaggggacccaggtcaccgtctcgtcgactagtaccacgacgccagcgccgcgaccaccaacaccggcgcccaccatcgcgtcgcagcccctgtccctgcgcccagaggcgtgccggccagcggcggggggcgcagtgcacacgagggggctggacttcgcctgtgatatctacatctgggcgcccttggccgggacttgtggggtccttctcctgtcactggttatcaccctttactgcaaacggggcagaaagaaactcctgtatatattcaaacaaccatttatgagaccagtacaaactactcaagaggaagatggctgtagctgccgatttccagaagaagaagaaggaggatgtgaactgagagtgaagttcagcaggagcgcagacgcccccgcgtaccagcagggccagaaccagctctataacgagctcaatctaggacgaagagaggagtacgatgttttggacaagagacgtggccgggaccctgagatggggggaaagccgagaaggaagaaccctcaggaaggcctgtacaatgaactgcagaaagataagatggcggaggcctacagtgagattgggatgaaaggcgagcgccggaggggcaaggggcacgatggcctttaccagggtctcagtacagccaccaaggacacctacgacgcccttcacatgcaggccctgccccctcgctaa

SEQ ID NO: 355 - DNA, 1515 bp, synthetic construct
  source 1..1515: mol_type = other DNA
atggctctgcccgtcaccgctctgctgctgcctctggctctgctgctgcacgctgctcgccctgaggtgcagctggtggagtctgggggaggaatggtgcaggctggggactctctgagactatcctgtgtgcagtctacttacaccgtcaatagcgatgtcatgggctggttccgccaggctccagggaaggagcgtgagtttgtaggagcgattatgtggaatgatggtattacatacttgcaagactccgtgaagggccgatttaccatcttcagagacaacgccaagaacacggtgtatctgcaaatgaacagcctgaaacttgaggatacggccgtttattactgtgcagcatccaagggtagatactcggaatatgagtactggggccaggggacccaggtcaccgtctcctcaggaggaggaggatccggcggaggaggctctggcggcggcggctccggcggcggcggctccgcggtgcagctggtggagtctgggggaggattggtgcaggctggggactctctgagactcacctgtacagcctctggacgcgccttcagtacctatttcatggcctggttccgccaggctccagggaaggagcgtgagtttgtagcaggaattgcatggagtggtggtagcacggcgtatgcagactccgtgaagggccgattcaccatctccagagacaacgccaagaacacggtgtatctgcaaatgaacagcctgaaatctgaggacacggccgtttattactgtgccagcagggggattgaggtcgaagagtttggtgcctggggccaggggacccaggtcaccgtctcgtcgactagtaccacgacgccagcgccgcgaccaccaacaccggcgcccaccatcgcgtcgcagcccctgtccctgcgcccagaggcgtgccggccagcggcggggggcgcagtgcacacgagggggctggacttcgcctgtgatatctacatctgggcgcccttggccgggacttgtggggtccttctcctgtcactggttatcaccctttactgcaaacggggcagaaagaaactcctgtatatattcaaacaaccatttatgagaccagtacaaactactcaagaggaagatggctgtagctgccgatttccagaagaagaagaaggaggatgtgaactgagagtgaagttcagcaggagcgcagacgcccccgcgtaccagcagggccagaaccagctctataacgagctcaatctaggacgaagagaggagtacgatgttttggacaagagacgtggccgggaccctgagatggggggaaagccgagaaggaagaaccctcaggaaggcctgtacaatgaactgcagaaagataagatggcggaggcctacagtgagattgggatgaaaggcgagcgccggaggggcaaggggcacgatggcctttaccagggtctcagtacagccaccaaggacacctacgacgcccttcacatgcaggccctgccccctcgctaa

SEQ ID NO: 356 - DNA, 1479 bp, synthetic construct
  source 1..1479: mol_type = other DNA
atggctctgcccgtcaccgctctgctgctgcctctggctctgctgctgcacgctgctcgccctcaggtaaagctggaggagtctgggggaggattggtgcaggctgggggctctctgagactctcctgtgcagcctctggaggcaccttaagtaagaataccgtggcttgggtccgccaggctccagggaaggagcgtgggtttgtaacgtctattacctgtgatggtcgtacgacatactatgcgaactccgtaaacggccgattccccatcaaccgaaacaacgccgagaatttggtggttttgcaaatgaacagcctgaaacctgacgacacggccctttattactgtgcagcataccggaagtcaataatgtctattcagcccgactactggggccaggggacccaggtcaccgtctcctcaggaggaggaggatctcaggtacagctggtggagtctgggggaggattggtgcaggctgggggctctctgagactctcctgtgcagcctctggaggcaccttaagtaaaaataccgtggcttggttccgccaggctccagggaaggagcgtgggtttgtagcgtctattacctgggatggtcgtacgacatactatgcagactccgtgaagggccgattcaccatctccagagacaacgccaagaacacagtgtatctgcaaatgaacagcctgaaacctgaggatacggccgtttatgtctgtgcagacttagggaaatggcctgcgggcccggcggactactggggccaggggacccaggtcaccgtctcctcaactagtaccacgacgccagcgccgcgaccaccaacaccggcgcccaccatcgcgtcgcagcccctgtccctgcgcccagaggcgtgccggccagcggcggggggcgcagtgcacacgagggggctggacttcgcctgtgatatctacatctgggcgcccttggccgggacttgtggggtccttctcctgtcactggttatcaccctttactgcaaacggggcagaaagaaactcctgtatatattcaaacaaccatttatgagaccagtacaaactactcaagaggaagatggctgtagctgccgatttccagaagaagaagaaggaggatgtgaactgagagtgaagttcagcaggagcgcagacgcccccgcgtaccagcagggccagaaccagctctataacgagctcaatctaggacgaagagaggagtacgatgttttggacaagagacgtggccgggaccctgagatggggggaaagccgagaaggaagaaccctcaggaaggcctgtacaatgaactgcagaaagataagatggcggaggcctacagtgagattgggatgaaaggcgagcgccggaggggcaaggggcacgatggcctttaccagggtctcagtacagccaccaaggacacctacgacgcccttcacatgcaggccctgccccctcgctaa

SEQ ID NO: 357 - DNA, 1509 bp, synthetic construct
  source 1..1509: mol_type = other DNA
atggctctgcccgtcaccgctctgctgctgcctctggctctgctgctgcacgctgctcgccctcaggtaaagctggaggagtctgggggaggattggtgcaggctgggggctctctgagactctcctgtgcagcctctggaggcaccttaagtaagaataccgtggcttgggtccgccaggctccagggaaggagcgtgggtttgtaacgtctattacctgtgatggtcgtacgacatactatgcgaactccgtaaacggccgattccccatcaaccgaaacaacgccgagaatttggtggttttgcaaatgaacagcctgaaacctgacgacacggccctttattactgtgcagcataccggaagtcaataatgtctattcagcccgactactggggccaggggacccaggtcaccgtctcctcaggaggaggaggatctggaggaggaggaagcggaggaggaggatcccaggtacagctggtggagtctgggggaggattggtgcaggctgggggctctctgagactctcctgtgcagcctctggaggcaccttaagtaaaaataccgtggcttggttccgccaggctccagggaaggagcgtgggtttgtagcgtctattacctgggatggtcgtacgacatactatgcagactccgtgaagggccgattcaccatctccagagacaacgccaagaacacagtgtatctgcaaatgaacagcctgaaacctgaggatacggccgtttatgtctgtgcagacttagggaaatggcctgcgggcccggcggactactggggccaggggacccaggtcaccgtctcctcaactagtaccacgacgccagcgccgcgaccaccaacaccggcgcccaccatcgcgtcgcagcccctgtccctgcgcccagaggcgtgccggccagcggcggggggcgcagtgcacacgagggggctggacttcgcctgtgatatctacatctgggcgcccttggccgggacttgtggggtccttctcctgtcactggttatcaccctttactgcaaacggggcagaaagaaactcctgtatatattcaaacaaccatttatgagaccagtacaaactactcaagaggaagatggctgtagctgccgatttccagaagaagaagaaggaggatgtgaactgagagtgaagttcagcaggagcgcagacgcccccgcgtaccagcagggccagaaccagctctataacgagctcaatctaggacgaagagaggagtacgatgttttggacaagagacgtggccgggaccctgagatggggggaaagccgagaaggaagaaccctcaggaaggcctgtacaatgaactgcagaaagataagatggcggaggcctacagtgagattgggatgaaaggcgagcgccggaggggcaaggggcacgatggcctttaccagggtctcagtacagccaccaaggacacctacgacgcccttcacatgcaggccctgccccctcgctaa

SEQ ID NO: 358 - DNA, 1539 bp, synthetic construct
  source 1..1539: mol_type = other DNA
atggctctgcccgtcaccgctctgctgctgcctctggctctgctgctgcacgctgctcgccctcaggtaaagctggaggagtctgggggaggattggtgcaggctgggggctctctgagactctcctgtgcagcctctggaggcaccttaagtaagaataccgtggcttgggtccgccaggctccagggaaggagcgtgggtttgtaacgtctattacctgtgatggtcgtacgacatactatgcgaactccgtaaacggccgattccccatcaaccgaaacaacgccgagaatttggtggttttgcaaatgaacagcctgaaacctgacgacacggccctttattactgtgcagcataccggaagtcaataatgtctattcagcccgactactggggccaggggacccaggtcaccgtctcctcaggaggaggaggatctggaggaggaggaagcggaggaggaggaagcggcggcggcggctctggcggcggcggcagccaggtacagctggtggagtctgggggaggattggtgcaggctgggggctctctgagactctcctgtgcagcctctggaggcaccttaagtaaaaataccgtggcttggttccgccaggctccagggaaggagcgtgggtttgtagcgtctattacctgggatggtcgtacgacatactatgcagactccgtgaagggccgattcaccatctccagagacaacgccaagaacacagtgtatctgcaaatgaacagcctgaaacctgaggatacggccgtttatgtctgtgcagacttagggaaatggcctgcgggcccggcggactactggggccaggggacccaggtcaccgtctcctcaactagtaccacgacgccagcgccgcgaccaccaacaccggcgcccaccatcgcgtcgcagcccctgtccctgcgcccagaggcgtgccggccagcggcggggggcgcagtgcacacgagggggctggacttcgcctgtgatatctacatctgggcgcccttggccgggacttgtggggtccttctcctgtcactggttatcaccctttactgcaaacggggcagaaagaaactcctgtatatattcaaacaaccatttatgagaccagtacaaactactcaagaggaagatggctgtagctgccgatttccagaagaagaagaaggaggatgtgaactgagagtgaagttcagcaggagcgcagacgcccccgcgtaccagcagggccagaaccagctctataacgagctcaatctaggacgaagagaggagtacgatgttttggacaagagacgtggccgggaccctgagatggggggaaagccgagaaggaagaaccctcaggaaggcctgtacaatgaactgcagaaagataagatggcggaggcctacagtgagattgggatgaaaggcgagcgccggaggggcaaggggcacgatggcctttaccagggtctcagtacagccaccaaggacacctacgacgcccttcacatgcaggccctgccccctcgctaa

SEQ ID NO: 359 - DNA, 1494 bp, synthetic construct
  source 1..1494: mol_type = other DNA
atggctctgcccgtcaccgctctgctgctgcctctggctctgctgctgcacgctgctcgccctcaggtaaagctggaggagtctgggggaggattggtgcaggctgggggctctctgagactctcctgtgcagcctctggaggcaccttaagtaagaataccgtggcttgggtccgccaggctccagggaaggagcgtgggtttgtaacgtctattacctgtgatggtcgtacgacatactatgcgaactccgtaaacggccgattccccatcaaccgaaacaacgccgagaatttggtggttttgcaaatgaacagcctgaaacctgacgacacggccctttattactgtgcagcataccggaagtcaataatgtctattcagcccgactactggggccaggggacccaggtcaccgtctcctcaggaggaggaggatccggcggaggaggctctcaggtacagctggtggagtctgggggaggattggtgcaggctgggggctctctgagactctcctgtgcagcctctggaggcaccttaagtaaaaataccgtggcttggttccgccaggctccagggaaggagcgtgggtttgtagcgtctattacctgggatggtcgtacgacatactatgcagactccgtgaagggccgattcaccatctccagagacaacgccaagaacacagtgtatctgcaaatgaacagcctgaaacctgaggatacggccgtttatgtctgtgcagacttagggaaatggcctgcgggcccggcggactactggggccaggggacccaggtcaccgtctcctcaactagtaccacgacgccagcgccgcgaccaccaacaccggcgcccaccatcgcgtcgcagcccctgtccctgcgcccagaggcgtgccggccagcggcggggggcgcagtgcacacgagggggctggacttcgcctgtgatatctacatctgggcgcccttggccgggacttgtggggtccttctcctgtcactggttatcaccctttactgcaaacggggcagaaagaaactcctgtatatattcaaacaaccatttatgagaccagtacaaactactcaagaggaagatggctgtagctgccgatttccagaagaagaagaaggaggatgtgaactgagagtgaagttcagcaggagcgcagacgcccccgcgtaccagcagggccagaaccagctctataacgagctcaatctaggacgaagagaggagtacgatgttttggacaagagacgtggccgggaccctgagatggggggaaagccgagaaggaagaaccctcaggaaggcctgtacaatgaactgcagaaagataagatggcggaggcctacagtgagattgggatgaaaggcgagcgccggaggggcaaggggcacgatggcctttaccagggtctcagtacagccaccaaggacacctacgacgcccttcacatgcaggccctgccccctcgctaa

SEQ ID NO: 360 - DNA, 1509 bp, synthetic construct
  source 1..1509: mol_type = other DNA
atggctctgcccgtcaccgctctgctgctgcctctggctctgctgctgcacgctgctcgccctcaggtaaagctggaggagtctgggggaggattggtgcaggctgggggctctctgagactctcctgtgcagcctctggaggcaccttaagtaagaataccgtggcttgggtccgccaggctccagggaaggagcgtgggtttgtaacgtctattacctgtgatggtcgtacgacatactatgcgaactccgtaaacggccgattccccatcaaccgaaacaacgccgagaatttggtggttttgcaaatgaacagcctgaaacctgacgacacggccctttattactgtgcagcataccggaagtcaataatgtctattcagcccgactactggggccaggggacccaggtcaccgtctcctcaggaggaggaggatccggcggaggaggctctggcggcggcggcagccaggtacagctggtggagtctgggggaggattggtgcaggctgggggctctctgagactctcctgtgcagcctctggaggcaccttaagtaaaaataccgtggcttggttccgccaggctccagggaaggagcgtgggtttgtagcgtctattacctgggatggtcgtacgacatactatgcagactccgtgaagggccgattcaccatctccagagacaacgccaagaacacagtgtatctgcaaatgaacagcctgaaacctgaggatacggccgtttatgtctgtgcagacttagggaaatggcctgcgggcccggcggactactggggccaggggacccaggtcaccgtctcctcaactagtaccacgacgccagcgccgcgaccaccaacaccggcgcccaccatcgcgtcgcagcccctgtccctgcgcccagaggcgtgccggccagcggcggggggcgcagtgcacacgagggggctggacttcgcctgtgatatctacatctgggcgcccttggccgggacttgtggggtccttctcctgtcactggttatcaccctttactgcaaacggggcagaaagaaactcctgtatatattcaaacaaccatttatgagaccagtacaaactactcaagaggaagatggctgtagctgccgatttccagaagaagaagaaggaggatgtgaactgagagtgaagttcagcaggagcgcagacgcccccgcgtaccagcagggccagaaccagctctataacgagctcaatctaggacgaagagaggagtacgatgttttggacaagagacgtggccgggaccctgagatggggggaaagccgagaaggaagaaccctcaggaaggcctgtacaatgaactgcagaaagataagatggcggaggcctacagtgagattgggatgaaaggcgagcgccggaggggcaaggggcacgatggcctttaccagggtctcagtacagccaccaaggacacctacgacgcccttcacatgcaggccctgccccctcgctaa

SEQ ID NO: 361 - DNA, 1524 bp, synthetic construct
  source 1..1524: mol_type = other DNA
atggctctgcccgtcaccgctctgctgctgcctctggctctgctgctgcacgctgctcgccctcaggtaaagctggaggagtctgggggaggattggtgcaggctgggggctctctgagactctcctgtgcagcctctggaggcaccttaagtaagaataccgtggcttgggtccgccaggctccagggaaggagcgtgggtttgtaacgtctattacctgtgatggtcgtacgacatactatgcgaactccgtaaacggccgattccccatcaaccgaaacaacgccgagaatttggtggttttgcaaatgaacagcctgaaacctgacgacacggccctttattactgtgcagcataccggaagtcaataatgtctattcagcccgactactggggccaggggacccaggtcaccgtctcctcaggaggaggaggatccggcggaggaggctctggcggcggcggctccggcggcggcggctcccaggtacagctggtggagtctgggggaggattggtgcaggctgggggctctctgagactctcctgtgcagcctctggaggcaccttaagtaaaaataccgtggcttggttccgccaggctccagggaaggagcgtgggtttgtagcgtctattacctgggatggtcgtacgacatactatgcagactccgtgaagggccgattcaccatctccagagacaacgccaagaacacagtgtatctgcaaatgaacagcctgaaacctgaggatacggccgtttatgtctgtgcagacttagggaaatggcctgcgggcccggcggactactggggccaggggacccaggtcaccgtctcctcaactagtaccacgacgccagcgccgcgaccaccaacaccggcgcccaccatcgcgtcgcagcccctgtccctgcgcccagaggcgtgccggccagcggcggggggcgcagtgcacacgagggggctggacttcgcctgtgatatctacatctgggcgcccttggccgggacttgtggggtccttctcctgtcactggttatcaccctttactgcaaacggggcagaaagaaactcctgtatatattcaaacaaccatttatgagaccagtacaaactactcaagaggaagatggctgtagctgccgatttccagaagaagaagaaggaggatgtgaactgagagtgaagttcagcaggagcgcagacgcccccgcgtaccagcagggccagaaccagctctataacgagctcaatctaggacgaagagaggagtacgatgttttggacaagagacgtggccgggaccctgagatggggggaaagccgagaaggaagaaccctcaggaaggcctgtacaatgaactgcagaaagataagatggcggaggcctacagtgagattgggatgaaaggcgagcgccggaggggcaaggggcacgatggcctttaccagggtctcagtacagccaccaaggacacctacgacgcccttcacatgcaggccctgccccctcgctaa

SEQ ID NO: 362 - DNA, 1476 bp, synthetic construct
  source 1..1476: mol_type = other DNA
atggctctgcccgtcaccgctctgctgctgcctctggctctgctgctgcacgctgctcgccctcaggtacagctggtggagtctgggggaggattggtgcaggctgggggctctctgagactctcctgtgcagcctctggaggcaccttaagtaaaaataccgtggcttggttccgccaggctccagggaaggagcgtgggtttgtagcgtctattacctgggatggtcgtacgacatactatgcagactccgtgaagggccgattcaccatctccagagacaacgccaagaacacagtgtatctgcaaatgaacagcctgaaacctgaggatacggccgtttatgtctgtgcagacttagggaaatggcctgcgggcccggcggactactggggccaggggacccaggtcaccgtctcctcaggaggaggaggatctgatgtgcagctggtggagtctgggggaggattggtgcaggctgggggctctctgagactctcctgtgcagcctctggaggcaccttaagtaagaataccgtggcttgggtccgccaggctccagggaaggagcgtgggtttgtaacgtctattacctgtgatggtcgtacgacatactatgcgaactccgtgaagggccgattccccatctccagagacaacgccgagaacacagtgtatctgcaaatgaacagcctgaaacctgaggatacggccggttatgtctgtgcagacttagggaagtggcctgcgggttcggcggactactggggccaggggacccacgtcaccgtctcctccactagtaccacgacgccagcgccgcgaccaccaacaccggcgcccaccatcgcgtcgcagcccctgtccctgcgcccagaggcgtgccggccagcggcggggggcgcagtgcacacgagggggctggacttcgcctgtgatatctacatctgggcgcccttggccgggacttgtggggtccttctcctgtcactggttatcaccctttactgcaaacggggcagaaagaaactcctgtatatattcaaacaaccatttatgagaccagtacaaactactcaagaggaagatggctgtagctgccgatttccagaagaagaagaaggaggatgtgaactgagagtgaagttcagcaggagcgcagacgcccccgcgtaccagcagggccagaaccagctctataacgagctcaatctaggacgaagagaggagtacgatgttttggacaagagacgtggccgggaccctgagatggggggaaagccgagaaggaagaaccctcaggaaggcctgtacaatgaactgcagaaagataagatggcggaggcctacagtgagattgggatgaaaggcgagcgccggaggggcaaggggcacgatggcctttaccagggtctcagtacagccaccaaggacacctacgacgcccttcacatgcaggccctgccccctcgctaa

SEQ ID NO: 363 - DNA, 1506 bp, synthetic construct
  source 1..1506: mol_type = other DNA
atggctctgcccgtcaccgctctgctgctgcctctggctctgctgctgcacgctgctcgccctcaggtacagctggtggagtctgggggaggattggtgcaggctgggggctctctgagactctcctgtgcagcctctggaggcaccttaagtaaaaataccgtggcttggttccgccaggctccagggaaggagcgtgggtttgtagcgtctattacctgggatggtcgtacgacatactatgcagactccgtgaagggccgattcaccatctccagagacaacgccaagaacacagtgtatctgcaaatgaacagcctgaaacctgaggatacggccgtttatgtctgtgcagacttagggaaatggcctgcgggcccggcggactactggggccaggggacccaggtcaccgtctcctcaggaggaggaggatctggaggaggaggaagcggaggaggaggatccgatgtgcagctggtggagtctgggggaggattggtgcaggctgggggctctctgagactctcctgtgcagcctctggaggcaccttaagtaagaataccgtggcttgggtccgccaggctccagggaaggagcgtgggtttgtaacgtctattacctgtgatggtcgtacgacatactatgcgaactccgtgaagggccgattccccatctccagagacaacgccgagaacacagtgtatctgcaaatgaacagcctgaaacctgaggatacggccggttatgtctgtgcagacttagggaagtggcctgcgggttcggcggactactggggccaggggacccacgtcaccgtctcctccactagtaccacgacgccagcgccgcgaccaccaacaccggcgcccaccatcgcgtcgcagcccctgtccctgcgcccagaggcgtgccggccagcggcggggggcgcagtgcacacgagggggctggacttcgcctgtgatatctacatctgggcgcccttggccgggacttgtggggtccttctcctgtcactggttatcaccctttactgcaaacggggcagaaagaaactcctgtatatattcaaacaaccatttatgagaccagtacaaactactcaagaggaagatggctgtagctgccgatttccagaagaagaagaaggaggatgtgaactgagagtgaagttcagcaggagcgcagacgcccccgcgtaccagcagggccagaaccagctctataacgagctcaatctaggacgaagagaggagtacgatgttttggacaagagacgtggccgggaccctgagatggggggaaagccgagaaggaagaaccctcaggaaggcctgtacaatgaactgcagaaagataagatggcggaggcctacagtgagattgggatgaaaggcgagcgccggaggggcaaggggcacgatggcctttaccagggtctcagtacagccaccaaggacacctacgacgcccttcacatgcaggccctgccccctcgctaa

SEQ ID NO: 364 - DNA, 1536 bp, synthetic construct
  source 1..1536: mol_type = other DNA
atggctctgcccgtcaccgctctgctgctgcctctggctctgctgctgcacgctgctcgccctcaggtacagctggtggagtctgggggaggattggtgcaggctgggggctctctgagactctcctgtgcagcctctggaggcaccttaagtaaaaataccgtggcttggttccgccaggctccagggaaggagcgtgggtttgtagcgtctattacctgggatggtcgtacgacatactatgcagactccgtgaagggccgattcaccatctccagagacaacgccaagaacacagtgtatctgcaaatgaacagcctgaaacctgaggatacggccgtttatgtctgtgcagacttagggaaatggcctgcgggcccggcggactactggggccaggggacccaggtcaccgtctcctcaggaggaggaggatctggaggaggaggaagcggaggaggaggaagcggcggcggcggctctggcggcggcggcagcgatgtgcagctggtggagtctgggggaggattggtgcaggctgggggctctctgagactctcctgtgcagcctctggaggcaccttaagtaagaataccgtggcttgggtccgccaggctccagggaaggagcgtgggtttgtaacgtctattacctgtgatggtcgtacgacatactatgcgaactccgtgaagggccgattccccatctccagagacaacgccgagaacacagtgtatctgcaaatgaacagcctgaaacctgaggatacggccggttatgtctgtgcagacttagggaagtggcctgcgggttcggcggactactggggccaggggacccacgtcaccgtctcctccactagtaccacgacgccagcgccgcgaccaccaacaccggcgcccaccatcgcgtcgcagcccctgtccctgcgcccagaggcgtgccggccagcggcggggggcgcagtgcacacgagggggctggacttcgcctgtgatatctacatctgggcgcccttggccgggacttgtggggtccttctcctgtcactggttatcaccctttactgcaaacggggcagaaagaaactcctgtatatattcaaacaaccatttatgagaccagtacaaactactcaagaggaagatggctgtagctgccgatttccagaagaagaagaaggaggatgtgaactgagagtgaagttcagcaggagcgcagacgcccccgcgtaccagcagggccagaaccagctctataacgagctcaatctaggacgaagagaggagtacgatgttttggacaagagacgtggccgggaccctgagatggggggaaagccgagaaggaagaaccctcaggaaggcctgtacaatgaactgcagaaagataagatggcggaggcctacagtgagattgggatgaaaggcgagcgccggaggggcaaggggcacgatggcctttaccagggtctcagtacagccaccaaggacacctacgacgcccttcacatgcaggccctgccccctcgctaa

SEQ ID NO: 365 - DNA, 1491 bp, synthetic construct
  source 1..1491: mol_type = other DNA
atggctctgcccgtcaccgctctgctgctgcctctggctctgctgctgcacgctgctcgccctcaggtacagctggtggagtctgggggaggattggtgcaggctgggggctctctgagactctcctgtgcagcctctggaggcaccttaagtaaaaataccgtggcttggttccgccaggctccagggaaggagcgtgggtttgtagcgtctattacctgggatggtcgtacgacatactatgcagactccgtgaagggccgattcaccatctccagagacaacgccaagaacacagtgtatctgcaaatgaacagcctgaaacctgaggatacggccgtttatgtctgtgcagacttagggaaatggcctgcgggcccggcggactactggggccaggggacccaggtcaccgtctcctcaggaggaggaggatccggcggaggaggctctgatgtgcagctggtggagtctgggggaggattggtgcaggctgggggctctctgagactctcctgtgcagcctctggaggcaccttaagtaagaataccgtggcttgggtccgccaggctccagggaaggagcgtgggtttgtaacgtctattacctgtgatggtcgtacgacatactatgcgaactccgtgaagggccgattccccatctccagagacaacgccgagaacacagtgtatctgcaaatgaacagcctgaaacctgaggatacggccggttatgtctgtgcagacttagggaagtggcctgcgggttcggcggactactggggccaggggacccacgtcaccgtctcctccactagtaccacgacgccagcgccgcgaccaccaacaccggcgcccaccatcgcgtcgcagcccctgtccctgcgcccagaggcgtgccggccagcggcggggggcgcagtgcacacgagggggctggacttcgcctgtgatatctacatctgggcgcccttggccgggacttgtggggtccttctcctgtcactggttatcaccctttactgcaaacggggcagaaagaaactcctgtatatattcaaacaaccatttatgagaccagtacaaactactcaagaggaagatggctgtagctgccgatttccagaagaagaagaaggaggatgtgaactgagagtgaagttcagcaggagcgcagacgcccccgcgtaccagcagggccagaaccagctctataacgagctcaatctaggacgaagagaggagtacgatgttttggacaagagacgtggccgggaccctgagatggggggaaagccgagaaggaagaaccctcaggaaggcctgtacaatgaactgcagaaagataagatggcggaggcctacagtgagattgggatgaaaggcgagcgccggaggggcaaggggcacgatggcctttaccagggtctcagtacagccaccaaggacacctacgacgcccttcacatgcaggccctgccccctcgctaa

SEQ ID NO: 366 - DNA, 1506 bp, synthetic construct
  source 1..1506: mol_type = other DNA
atggctctgcccgtcaccgctctgctgctgcctctggctctgctgctgcacgctgctcgccctcaggtacagctggtggagtctgggggaggattggtgcaggctgggggctctctgagactctcctgtgcagcctctggaggcaccttaagtaaaaataccgtggcttggttccgccaggctccagggaaggagcgtgggtttgtagcgtctattacctgggatggtcgtacgacatactatgcagactccgtgaagggccgattcaccatctccagagacaacgccaagaacacagtgtatctgcaaatgaacagcctgaaacctgaggatacggccgtttatgtctgtgcagacttagggaaatggcctgcgggcccggcggactactggggccaggggacccaggtcaccgtctcctcaggaggaggaggatccggcggaggaggctctggcggcggcggcagcgatgtgcagctggtggagtctgggggaggattggtgcaggctgggggctctctgagactctcctgtgcagcctctggaggcaccttaagtaagaataccgtggcttgggtccgccaggctccagggaaggagcgtgggtttgtaacgtctattacctgtgatggtcgtacgacatactatgcgaactccgtgaagggccgattccccatctccagagacaacgccgagaacacagtgtatctgcaaatgaacagcctgaaacctgaggatacggccggttatgtctgtgcagacttagggaagtggcctgcgggttcggcggactactggggccaggggacccacgtcaccgtctcctccactagtaccacgacgccagcgccgcgaccaccaacaccggcgcccaccatcgcgtcgcagcccctgtccctgcgcccagaggcgtgccggccagcggcggggggcgcagtgcacacgagggggctggacttcgcctgtgatatctacatctgggcgcccttggccgggacttgtggggtccttctcctgtcactggttatcaccctttactgcaaacggggcagaaagaaactcctgtatatattcaaacaaccatttatgagaccagtacaaactactcaagaggaagatggctgtagctgccgatttccagaagaagaagaaggaggatgtgaactgagagtgaagttcagcaggagcgcagacgcccccgcgtaccagcagggccagaaccagctctataacgagctcaatctaggacgaagagaggagtacgatgttttggacaagagacgtggccgggaccctgagatggggggaaagccgagaaggaagaaccctcaggaaggcctgtacaatgaactgcagaaagataagatggcggaggcctacagtgagattgggatgaaaggcgagcgccggaggggcaaggggcacgatggcctttaccagggtctcagtacagccaccaaggacacctacgacgcccttcacatgcaggccctgccccctcgctaa

SEQ ID NO: 367 - DNA, 1521 bp, synthetic construct
  source 1..1521: mol_type = other DNA
atggctctgcccgtcaccgctctgctgctgcctctggctctgctgctgcacgctgctcgccctcaggtacagctggtggagtctgggggaggattggtgcaggctgggggctctctgagactctcctgtgcagcctctggaggcaccttaagtaaaaataccgtggcttggttccgccaggctccagggaaggagcgtgggtttgtagcgtctattacctgggatggtcgtacgacatactatgcagactccgtgaagggccgattcaccatctccagagacaacgccaagaacacagtgtatctgcaaatgaacagcctgaaacctgaggatacggccgtttatgtctgtgcagacttagggaaatggcctgcgggcccggcggactactggggccaggggacccaggtcaccgtctcctcaggaggaggaggatccggcggaggaggctctggcggcggcggctccggcggcggcggctccgatgtgcagctggtggagtctgggggaggattggtgcaggctgggggctctctgagactctcctgtgcagcctctggaggcaccttaagtaagaataccgtggcttgggtccgccaggctccagggaaggagcgtgggtttgtaacgtctattacctgtgatggtcgtacgacatactatgcgaactccgtgaagggccgattccccatctccagagacaacgccgagaacacagtgtatctgcaaatgaacagcctgaaacctgaggatacggccggttatgtctgtgcagacttagggaagtggcctgcgggttcggcggactactggggccaggggacccacgtcaccgtctcctccactagtaccacgacgccagcgccgcgaccaccaacaccggcgcccaccatcgcgtcgcagcccctgtccctgcgcccagaggcgtgccggccagcggcggggggcgcagtgcacacgagggggctggacttcgcctgtgatatctacatctgggcgcccttggccgggacttgtggggtccttctcctgtcactggttatcaccctttactgcaaacggggcagaaagaaactcctgtatatattcaaacaaccatttatgagaccagtacaaactactcaagaggaagatggctgtagctgccgatttccagaagaagaagaaggaggatgtgaactgagagtgaagttcagcaggagcgcagacgcccccgcgtaccagcagggccagaaccagctctataacgagctcaatctaggacgaagagaggagtacgatgttttggacaagagacgtggccgggaccctgagatggggggaaagccgagaaggaagaaccctcaggaaggcctgtacaatgaactgcagaaagataagatggcggaggcctacagtgagattgggatgaaaggcgagcgccggaggggcaaggggcacgatggcctttaccagggtctcagtacagccaccaaggacacctacgacgcccttcacatgcaggccctgccccctcgctaa

SEQ ID NO: 368 - DNA, 1473 bp, synthetic construct
  source 1..1473: mol_type = other DNA
atggctctgcccgtcaccgctctgctgctgcctctggctctgctgctgcacgctgctcgccctgatgtgcagctggtggagtctgggggaggattggtgcaggctgggggctctctgagactctcctgtgcagcctctggaggcaccttaagtaagaataccgtggcttgggtccgccaggctccagggaaggagcgtgggtttgtaacgtctattacctgtgatggtcgtacgacatactatgcgaactccgtgaagggccgattccccatctccagagacaacgccgagaacacagtgtatctgcaaatgaacagcctgaaacctgaggatacggccggttatgtctgtgcagacttagggaagtggcctgcgggttcggcggactactggggccaggggacccacgtcaccgtctcctccggaggaggaggatctgatgtgcagctggtggagtctgggggaggcttggtgcagcctggggggtctctgagactctcctgtgcagcctctggacggaccttcagtagcattgtcatgggctggttccgccaggctccagggaaggagcgtgagtttgtaggagcgattatgtggaatgatggtattacatacttgcaagactccgtgaagggccgatttaccatcttcagagacaacgccaagaacacggtgtatctgcaaatgaacagcctgaaacttgaggatacggccgtttattactgtgcagcatccaagggtagatactcggaatatgagtactggggccaggggacccaggtcaccgtctcctcaactagtaccacgacgccagcgccgcgaccaccaacaccggcgcccaccatcgcgtcgcagcccctgtccctgcgcccagaggcgtgccggccagcggcggggggcgcagtgcacacgagggggctggacttcgcctgtgatatctacatctgggcgcccttggccgggacttgtggggtccttctcctgtcactggttatcaccctttactgcaaacggggcagaaagaaactcctgtatatattcaaacaaccatttatgagaccagtacaaactactcaagaggaagatggctgtagctgccgatttccagaagaagaagaaggaggatgtgaactgagagtgaagttcagcaggagcgcagacgcccccgcgtaccagcagggccagaaccagctctataacgagctcaatctaggacgaagagaggagtacgatgttttggacaagagacgtggccgggaccctgagatggggggaaagccgagaaggaagaaccctcaggaaggcctgtacaatgaactgcagaaagataagatggcggaggcctacagtgagattgggatgaaaggcgagcgccggaggggcaaggggcacgatggcctttaccagggtctcagtacagccaccaaggacacctacgacgcccttcacatgcaggccctgccccctcgctaa

SEQ ID NO: 369 - DNA, 1503 bp, synthetic construct
  source 1..1503: mol_type = other DNA
atggctctgcccgtcaccgctctgctgctgcctctggctctgctgctgcacgctgctcgccctgatgtgcagctggtggagtctgggggaggattggtgcaggctgggggctctctgagactctcctgtgcagcctctggaggcaccttaagtaagaataccgtggcttgggtccgccaggctccagggaaggagcgtgggtttgtaacgtctattacctgtgatggtcgtacgacatactatgcgaactccgtgaagggccgattccccatctccagagacaacgccgagaacacagtgtatctgcaaatgaacagcctgaaacctgaggatacggccggttatgtctgtgcagacttagggaagtggcctgcgggttcggcggactactggggccaggggacccacgtcaccgtctcctccggaggaggaggatctggaggaggaggaagcggaggaggaggatccgatgtgcagctggtggagtctgggggaggcttggtgcagcctggggggtctctgagactctcctgtgcagcctctggacggaccttcagtagcattgtcatgggctggttccgccaggctccagggaaggagcgtgagtttgtaggagcgattatgtggaatgatggtattacatacttgcaagactccgtgaagggccgatttaccatcttcagagacaacgccaagaacacggtgtatctgcaaatgaacagcctgaaacttgaggatacggccgtttattactgtgcagcatccaagggtagatactcggaatatgagtactggggccaggggacccaggtcaccgtctcctcaactagtaccacgacgccagcgccgcgaccaccaacaccggcgcccaccatcgcgtcgcagcccctgtccctgcgcccagaggcgtgccggccagcggcggggggcgcagtgcacacgagggggctggacttcgcctgtgatatctacatctgggcgcccttggccgggacttgtggggtccttctcctgtcactggttatcaccctttactgcaaacggggcagaaagaaactcctgtatatattcaaacaaccatttatgagaccagtacaaactactcaagaggaagatggctgtagctgccgatttccagaagaagaagaaggaggatgtgaactgagagtgaagttcagcaggagcgcagacgcccccgcgtaccagcagggccagaaccagctctataacgagctcaatctaggacgaagagaggagtacgatgttttggacaagagacgtggccgggaccctgagatggggggaaagccgagaaggaagaaccctcaggaaggcctgtacaatgaactgcagaaagataagatggcggaggcctacagtgagattgggatgaaaggcgagcgccggaggggcaaggggcacgatggcctttaccagggtctcagtacagccaccaaggacacctacgacgcccttcacatgcaggccctgccccctcgctaa

SEQ ID NO: 370 - DNA, 1533 bp, synthetic construct
  source 1..1533: mol_type = other DNA
atggctctgcccgtcaccgctctgctgctgcctctggctctgctgctgcacgctgctcgccctgatgtgcagctggtggagtctgggggaggattggtgcaggctgggggctctctgagactctcctgtgcagcctctggaggcaccttaagtaagaataccgtggcttgggtccgccaggctccagggaaggagcgtgggtttgtaacgtctattacctgtgatggtcgtacgacatactatgcgaactccgtgaagggccgattccccatctccagagacaacgccgagaacacagtgtatctgcaaatgaacagcctgaaacctgaggatacggccggttatgtctgtgcagacttagggaagtggcctgcgggttcggcggactactggggccaggggacccacgtcaccgtctcctccggaggaggaggatctggaggaggaggaagcggaggaggaggaagcggcggcggcggctctggcggcggcggcagcgatgtgcagctggtggagtctgggggaggcttggtgcagcctggggggtctctgagactctcctgtgcagcctctggacggaccttcagtagcattgtcatgggctggttccgccaggctccagggaaggagcgtgagtttgtaggagcgattatgtggaatgatggtattacatacttgcaagactccgtgaagggccgatttaccatcttcagagacaacgccaagaacacggtgtatctgcaaatgaacagcctgaaacttgaggatacggccgtttattactgtgcagcatccaagggtagatactcggaatatgagtactggggccaggggacccaggtcaccgtctcctcaactagtaccacgacgccagcgccgcgaccaccaacaccggcgcccaccatcgcgtcgcagcccctgtccctgcgcccagaggcgtgccggccagcggcggggggcgcagtgcacacgagggggctggacttcgcctgtgatatctacatctgggcgcccttggccgggacttgtggggtccttctcctgtcactggttatcaccctttactgcaaacggggcagaaagaaactcctgtatatattcaaacaaccatttatgagaccagtacaaactactcaagaggaagatggctgtagctgccgatttccagaagaagaagaaggaggatgtgaactgagagtgaagttcagcaggagcgcagacgcccccgcgtaccagcagggccagaaccagctctataacgagctcaatctaggacgaagagaggagtacgatgttttggacaagagacgtggccgggaccctgagatggggggaaagccgagaaggaagaaccctcaggaaggcctgtacaatgaactgcagaaagataagatggcggaggcctacagtgagattgggatgaaaggcgagcgccggaggggcaaggggcacgatggcctttaccagggtctcagtacagccaccaaggacacctacgacgcccttcacatgcaggccctgccccctcgctaa

SEQ ID NO: 371 - DNA, 1488 bp, synthetic construct
  source 1..1488: mol_type = other DNA
atggctctgcccgtcaccgctctgctgctgcctctggctctgctgctgcacgctgctcgccctgatgtgcagctggtggagtctgggggaggattggtgcaggctgggggctctctgagactctcctgtgcagcctctggaggcaccttaagtaagaataccgtggcttgggtccgccaggctccagggaaggagcgtgggtttgtaacgtctattacctgtgatggtcgtacgacatactatgcgaactccgtgaagggccgattccccatctccagagacaacgccgagaacacagtgtatctgcaaatgaacagcctgaaacctgaggatacggccggttatgtctgtgcagacttagggaagtggcctgcgggttcggcggactactggggccaggggacccacgtcaccgtctcctccggaggaggaggatccggcggaggaggctctgatgtgcagctggtggagtctgggggaggcttggtgcagcctggggggtctctgagactctcctgtgcagcctctggacggaccttcagtagcattgtcatgggctggttccgccaggctccagggaaggagcgtgagtttgtaggagcgattatgtggaatgatggtattacatacttgcaagactccgtgaagggccgatttaccatcttcagagacaacgccaagaacacggtgtatctgcaaatgaacagcctgaaacttgaggatacggccgtttattactgtgcagcatccaagggtagatactcggaatatgagtactggggccaggggacccaggtcaccgtctcctcaactagtaccacgacgccagcgccgcgaccaccaacaccggcgcccaccatcgcgtcgcagcccctgtccctgcgcccagaggcgtgccggccagcggcggggggcgcagtgcacacgagggggctggacttcgcctgtgatatctacatctgggcgcccttggccgggacttgtggggtccttctcctgtcactggttatcaccctttactgcaaacggggcagaaagaaactcctgtatatattcaaacaaccatttatgagaccagtacaaactactcaagaggaagatggctgtagctgccgatttccagaagaagaagaaggaggatgtgaactgagagtgaagttcagcaggagcgcagacgcccccgcgtaccagcagggccagaaccagctctataacgagctcaatctaggacgaagagaggagtacgatgttttggacaagagacgtggccgggaccctgagatggggggaaagccgagaaggaagaaccctcaggaaggcctgtacaatgaactgcagaaagataagatggcggaggcctacagtgagattgggatgaaaggcgagcgccggaggggcaaggggcacgatggcctttaccagggtctcagtacagccaccaaggacacctacgacgcccttcacatgcaggccctgccccctcgctaa

SEQ ID NO: 372 - DNA, 1503 bp, synthetic construct
  source 1..1503: mol_type = other DNA
atggctctgcccgtcaccgctctgctgctgcctctggctctgctgctgcacgctgctcgccctgatgtgcagctggtggagtctgggggaggattggtgcaggctgggggctctctgagactctcctgtgcagcctctggaggcaccttaagtaagaataccgtggcttgggtccgccaggctccagggaaggagcgtgggtttgtaacgtctattacctgtgatggtcgtacgacatactatgcgaactccgtgaagggccgattccccatctccagagacaacgccgagaacacagtgtatctgcaaatgaacagcctgaaacctgaggatacggccggttatgtctgtgcagacttagggaagtggcctgcgggttcggcggactactggggccaggggacccacgtcaccgtctcctccggaggaggaggatccggcggaggaggctctggcggcggcggcagcgatgtgcagctggtggagtctgggggaggcttggtgcagcctggggggtctctgagactctcctgtgcagcctctggacggaccttcagtagcattgtcatgggctggttccgccaggctccagggaaggagcgtgagtttgtaggagcgattatgtggaatgatggtattacatacttgcaagactccgtgaagggccgatttaccatcttcagagacaacgccaagaacacggtgtatctgcaaatgaacagcctgaaacttgaggatacggccgtttattactgtgcagcatccaagggtagatactcggaatatgagtactggggccaggggacccaggtcaccgtctcctcaactagtaccacgacgccagcgccgcgaccaccaacaccggcgcccaccatcgcgtcgcagcccctgtccctgcgcccagaggcgtgccggccagcggcggggggcgcagtgcacacgagggggctggacttcgcctgtgatatctacatctgggcgcccttggccgggacttgtggggtccttctcctgtcactggttatcaccctttactgcaaacggggcagaaagaaactcctgtatatattcaaacaaccatttatgagaccagtacaaactactcaagaggaagatggctgtagctgccgatttccagaagaagaagaaggaggatgtgaactgagagtgaagttcagcaggagcgcagacgcccccgcgtaccagcagggccagaaccagctctataacgagctcaatctaggacgaagagaggagtacgatgttttggacaagagacgtggccgggaccctgagatggggggaaagccgagaaggaagaaccctcaggaaggcctgtacaatgaactgcagaaagataagatggcggaggcctacagtgagattgggatgaaaggcgagcgccggaggggcaaggggcacgatggcctttaccagggtctcagtacagccaccaaggacacctacgacgcccttcacatgcaggccctgccccctcgctaa

SEQ ID NO: 373 - DNA, 1518 bp, synthetic construct
  source 1..1518: mol_type = other DNA
atggctctgcccgtcaccgctctgctgctgcctctggctctgctgctgcacgctgctcgccctgatgtgcagctggtggagtctgggggaggattggtgcaggctgggggctctctgagactctcctgtgcagcctctggaggcaccttaagtaagaataccgtggcttgggtccgccaggctccagggaaggagcgtgggtttgtaacgtctattacctgtgatggtcgtacgacatactatgcgaactccgtgaagggccgattccccatctccagagacaacgccgagaacacagtgtatctgcaaatgaacagcctgaaacctgaggatacggccggttatgtctgtgcagacttagggaagtggcctgcgggttcggcggactactggggccaggggacccacgtcaccgtctcctccggaggaggaggatccggcggaggaggctctggcggcggcggctccggcggcggcggctccgatgtgcagctggtggagtctgggggaggcttggtgcagcctggggggtctctgagactctcctgtgcagcctctggacggaccttcagtagcattgtcatgggctggttccgccaggctccagggaaggagcgtgagtttgtaggagcgattatgtggaatgatggtattacatacttgcaagactccgtgaagggccgatttaccatcttcagagacaacgccaagaacacggtgtatctgcaaatgaacagcctgaaacttgaggatacggccgtttattactgtgcagcatccaagggtagatactcggaatatgagtactggggccaggggacccaggtcaccgtctcctcaactagtaccacgacgccagcgccgcgaccaccaacaccggcgcccaccatcgcgtcgcagcccctgtccctgcgcccagaggcgtgccggccagcggcggggggcgcagtgcacacgagggggctggacttcgcctgtgatatctacatctgggcgcccttggccgggacttgtggggtccttctcctgtcactggttatcaccctttactgcaaacggggcagaaagaaactcctgtatatattcaaacaaccatttatgagaccagtacaaactactcaagaggaagatggctgtagctgccgatttccagaagaagaagaaggaggatgtgaactgagagtgaagttcagcaggagcgcagacgcccccgcgtaccagcagggccagaaccagctctataacgagctcaatctaggacgaagagaggagtacgatgttttggacaagagacgtggccgggaccctgagatggggggaaagccgagaaggaagaaccctcaggaaggcctgtacaatgaactgcagaaagataagatggcggaggcctacagtgagattgggatgaaaggcgagcgccggaggggcaaggggcacgatggcctttaccagggtctcagtacagccaccaaggacacctacgacgcccttcacatgcaggccctgccccctcgctaa

SEQ ID NO: 374 - DNA, 23 bp, synthetic construct
  source 1..23: mol_type = other DNA
gtcctggctgctcttctacaagg

SEQ ID NO: 375 - DNA, 23 bp, synthetic construct
  source 1..23: mol_type = other DNA
ggtacgtgctgttgaactgttcc

SEQ ID NO: 376 - DNA, 29 bp, synthetic construct
  source 1..29: mol_type = other DNA
gatgtgcagctgcaggagtctggaggagg

SEQ ID NO: 377 - DNA, 29 bp, synthetic construct
  source 1..29: mol_type = other DNA
gatgtgcagctgcaggagtctgggggagg

SEQ ID NO: 378 - DNA, 34 bp, synthetic construct
  source 1..34: mol_type = other DNA
ctagtgcggccgctgaggagacggtgacctgggt

SEQ ID NO: 379-384 - skipped (6 entries)

SEQ ID NO: 385 - protein, 21 aa, synthetic construct
GSGEGRGSLLTCGDVEENPGP

SEQ ID NO: 386 - protein, 18 aa, Homo sapiens
MKWVTFISLLFLFSSAYS

SEQ ID NO: 387 - protein, 9 aa, synthetic construct
GSGHHHHHH

SEQ ID NO: 388 - protein, 10 aa, synthetic construct
MLQMAGQCSQ

SEQ ID NO: 389 - protein, 14 aa, synthetic construct
CSQNEYFDSLLHAC

SEQ ID NO: 390 - protein, 13 aa, synthetic construct
NEYFDSLLHACIP

SEQ ID NO: 391 - protein, 11 aa, synthetic construct
ACIPCQLRCSS

SEQ ID NO: 392 - protein, 19 aa, synthetic construct
CQLRCSSNTPPLTCQRYCN

SEQ ID NO: 393 - protein, 10 aa, synthetic construct
LTCQRYCNAS

SEQ ID NO: 394 - protein, 12 aa, synthetic construct
ASVTNSVKGTNA

SEQ ID NO: 395 - protein, 54 aa, synthetic construct
MLQMAGQCSQNEYFDSLLHACIPCQLRCSSNTPPLTCQRYCNASVTNSVKGTNA

SEQ ID NO: 396 - protein, 23 aa, synthetic construct
ILWTCLGLSLIISLAVFVLMFLL

SEQ ID NO: 397 - protein, 107 aa, synthetic construct
RKINSEPLKDEFKNTGSGLLGMANIDLEKSRTGDEIILPRGLEYTVEECTCEDCIKSKPKVDSDHCFPLPAMEEGATILVTTKTNDYCKSLPAALSATEIEKSISAR

SEQ ID NO: 398 - DNA, 23 bp, synthetic construct
  source 1..23: mol_type = other DNA
gtccttctcctgtcactggttat

SEQ ID NO: 399 - DNA, 23 bp, synthetic construct
  source 1..23: mol_type = other DNA
tcttcttcttctggaaatcggca